European Patent Application EP 4 806 466 A1, published September 16, 2026. Title: FOLATE RECEPTOR ALPHA ANTIBODY DRUG CONJUGATES. Applicant: AbbVie Inc. Application EP. The sequence listing filed with the application follows.

SEQUENCE LISTING (352 sequences)

SEQ ID NO: 1 - protein, 5 aa, synthetic construct
GYFMN

SEQ ID NO: 2 - protein, 17 aa, synthetic construct
RIHPYDGDTFYNQKFQG

SEQ ID NO: 3 - protein, 9 aa, synthetic construct
YDGSRAMDY

SEQ ID NO: 4 - protein, 118 aa, synthetic construct
QVQLVQSGAEVVKPGASVKISCKASGYTFTGYFMNWVKQSPGQSLEWIGRIHPYDGDTFYNQKFQGKATLTVDKSSNTAHMELLSLTSEDFAVYYCTRYDGSRAMDYWGQGTTVTVSS

SEQ ID NO: 5 - protein, 448 aa, synthetic construct
QVQLVQSGAEVVKPGASVKISCKASGYTFTGYFMNWVKQSPGQSLEWIGRIHPYDGDTFYNQKFQGKATLTVDKSSNTAHMELLSLTSEDFAVYYCTRYDGSRAMDYWGQGTTVTVSSASTKGPSVFPLAPSSKSTSGGTAALGCLVKDYFPEPVTVSWNSGALTSGVHTFPAVLQSSGLYSLSSVVTVPSSSLGTQTYICNVNHKPSNTKVDKKVEPKSCDKTHTCPPCPAPELLGGPSVFLFPPKPKDTLMISRTPEVTCVVVDVSHEDPEVKFNWYVDGVEVHNAKTKPREEQYNSTYRVVSVLTVLHQDWLNGKEYKCKVSNKALPAPIEKTISKAKGQPREPQVYTLPPSRDELTKNQVSLTCLVKGFYPSDIAVEWESNGQPENNYKTTPPVLDSDGSFFLYSKLTVDKSRWQQGNVFSCSVMHEALHNHYTQKSLSLSPGK

SEQ ID NO: 6 - protein, 447 aa, synthetic construct
QVQLVQSGAEVVKPGASVKISCKASGYTFTGYFMNWVKQSPGQSLEWIGRIHPYDGDTFYNQKFQGKATLTVDKSSNTAHMELLSLTSEDFAVYYCTRYDGSRAMDYWGQGTTVTVSSASTKGPSVFPLAPSSKSTSGGTAALGCLVKDYFPEPVTVSWNSGALTSGVHTFPAVLQSSGLYSLSSVVTVPSSSLGTQTYICNVNHKPSNTKVDKKVEPKSCDKTHTCPPCPAPELLGGPSVFLFPPKPKDTLMISRTPEVTCVVVDVSHEDPEVKFNWYVDGVEVHNAKTKPREEQYNSTYRVVSVLTVLHQDWLNGKEYKCKVSNKALPAPIEKTISKAKGQPREPQVYTLPPSRDELTKNQVSLTCLVKGFYPSDIAVEWESNGQPENNYKTTPPVLDSDGSFFLYSKLTVDKSRWQQGNVFSCSVMHEALHNHYTQKSLSLSPG

SEQ ID NO: 7 - protein, 15 aa, synthetic construct
KASQSVSFAGTSLMH

SEQ ID NO: 8 - protein, 7 aa, synthetic construct
RASNLEA

SEQ ID NO: 9 - protein, 9 aa, synthetic construct
QQSREYPYT

SEQ ID NO: 10 - protein, 112 aa, synthetic construct
DIVLTQSPLSLAVSLGQPAIISCKASQSVSFAGTSLMHWYHQKPGQQPRLLIYRASNLEAGVPDRFSGSGSKTDFTLTISPVEAEDAATYYCQQSREYPYTFGGGTKLEIKR

SEQ ID NO: 11 - protein, 218 aa, synthetic construct
DIVLTQSPLSLAVSLGQPAIISCKASQSVSFAGTSLMHWYHQKPGQQPRLLIYRASNLEAGVPDRFSGSGSKTDFTLTISPVEAEDAATYYCQQSREYPYTFGGGTKLEIKRTVAAPSVFIFPPSDEQLKSGTASVVCLLNNFYPREAKVQWKVDNALQSGNSQESVTEQDSKDSTYSLSSTLTLSKADYEKHKVYACEVTHQGLSSPVTKSFNRGEC

SEQ ID NO: 12 - protein, 479 aa, synthetic construct
EIVLTQSPATLSVTPGDRVSLSCRASQNINNNLHWYQQKPGQSPRLLIKYVSQSVSGIPDRFSGSGSGTDFTLSISSVEPEDEGMYFCQQSNSWPHYTFGCGTKLEIKGGGGSGGGGSGGGGSGGGGSEVQLVQSGGGLVQPGGSRRLSCAASGFTFSSFGMHWVRQAPGKCLEWVAYISSGSSTISYADSVKGRFTISRDNSKKTLLLQMTSLRAEDTAMYYCAREAYGSSMEYWGQGTLVTVSSGSEPKSSDKTHTCPPCPAPELLGGPSVFLFPPKPKDTLMISRTPEVTCVVVDVSHEDPEVKFNWYVDGVEVHNAKTKPREEQYNSTYRVVSVLTVLHQDWLNGKEYKCKVSNKALPAPIEKTISKAKGQPREPQVYTLPPSREEMTKNQVSLWCLVKGFYPSDIAVEWESNGQPENNYKTTPPVLDSDGSFFLYSKLTVDKSRWQQGNVFSCSVMHEALHNHYTQKSLSLSPG

SEQ ID NO: 13 - protein, 447 aa, synthetic construct
QVQLVQSGAEVVKPGASVKISCKASGYTFTGYFMNWVKQSPGQSLEWIGRIHPYDGDTFYNQKFQGKATLTVDKSSNTAHMELLSLTSEDFAVYYCTRYDGSRAMDYWGQGTTVTVSSASTKGPSVFPLAPSSKSTSGGTAALGCLVKDYFPEPVTVSWNSGALTSGVHTFPAVLQSSGLYSLSSVVTVPSSSLGTQTYICNVNHKPSNTKVDKKVEPKSCDKTHTCPPCPAPELLGGPSVFLFPPKPKDTLMISRTPEVTCVVVDVSHEDPEVKFNWYVDGVEVHNAKTKPREEQYNSTYRVVSVLTVLHQDWLNGKEYKCKVSNKALPAPIEKTISKAKGQPREPQVYTLPPSREEMTKNQVSLSCAVKGFYPSDIAVEWESNGQPENNYKTTPPVLDSDGSFFLVSKLTVDKSRWQQGNVFSCSVMHEALHNHYTQKSLSLSPG

SEQ ID NO: 14 - protein, 118 aa, synthetic construct
EVQLVQSGGGLVQPGGSRRLSCAASGFTFSSFGMHWVRQAPGKCLEWVAYISSGSSTISYADSVKGRFTISRDNSKKTLLLQMTSLRAEDTAMYYCAREAYGSSMEYWGQGTLVTVSS

SEQ ID NO: 15 - protein, 108 aa, synthetic construct
EIVLTQSPATLSVTPGDRVSLSCRASQNINNNLHWYQQKPGQSPRLLIKYVSQSVSGIPDRFSGSGSGTDFTLSISSVEPEDEGMYFCQQSNSWPHYTFGCGTKLEIK

SEQ ID NO: 16 - protein, 11 aa, synthetic construct
RASQNINNNLH

SEQ ID NO: 17 - protein, 7 aa, synthetic construct
YVSQSVS

SEQ ID NO: 18 - protein, 10 aa, synthetic construct
QQSNSWPHYT

SEQ ID NO: 19 - protein, 5 aa, synthetic construct
SFGMH

SEQ ID NO: 20 - protein, 17 aa, synthetic construct
YISSGSSTISYADSVKG

SEQ ID NO: 21 - protein, 9 aa, synthetic construct
EAYGSSMEY

SEQ ID NO: 22 - protein, 111 aa, synthetic construct
DIVLTQSPLSLAVSLGQPAIISCKASQSVSFAGTSLMHWYHQKPGQQPRLLIYRASNLEAGVPDRFSGSGSKTDFTLTISPVEAEDAATYYCQQSREYPYTFGGGTKLEIK

SEQ ID NO: 23 - protein, 10 aa, synthetic construct
GYTFTGYFMN

SEQ ID NO: 24 - protein, 10 aa, synthetic construct
RIHPYDGDTF

SEQ ID NO: 25 - protein, 10 aa, synthetic construct
GFTFSSFGMH

SEQ ID NO: 26 - protein, 10 aa, synthetic construct
YISSGSSTIS

SEQ ID NO: 27 - protein, 330 aa, synthetic construct [sequence omitted]

SEQ ID NO: 28 - protein, 329 aa, synthetic construct
ASTKGPSVFPLAPSSKSTSGGTAALGCLVKDYFPEPVTVSWNSGALTSGVHTFPAVLQSSGLYSLSSVVTVPSSSLGTQTYICNVNHKPSNTKVDKKVEPKSCDKTHTCPPCPAPELLGGPSVFLFPPKPKDTLMISRTPEVTCVVVDVSHEDPEVKFNWYVDGVEVHNAKTKPREEQYNSTYRVVSVLTVLHQDWLNGKEYKCKVSNKALPAPIEKTISKAKGQPREPQVYTLPPSRDELTKNQVSLTCLVKGFYPSDIAVEWESNGQPENNYKTTPPVLDSDGSFFLYSKLTVDKSRWQQGNVFSCSVMHEALHNHYTQKSLSLSPG

SEQ ID NO: 29 - protein, 330 aa, synthetic construct
ASTKGPSVFPLAPSSKSTSGGTAALGCLVKDYFPEPVTVSWNSGALTSGVHTFPAVLQSSGLYSLSSVVTVPSSSLGTQTYICNVNHKPSNTKVDKKVEPKSCDKTHTCPPCPAPESTRGPSVFLFPPKPKDTLMISRTPEVTCVVVDVSHEDPEVKFNWYVDGVEVHNAKTKPREEQYNSTYRVVSVLTVLHQDWLNGKEYKCKVSNKALPAPIEKTISKAKGQPREPQVYTLPPSRDELTKNQVSLTCLVKGFYPSDIAVEWESNGQPENNYKTTPPVLDSDGSFFLYSKLTVDKSRWQQGNVFSCSVMHEALHNHYTQKSLSLSPGK

SEQ ID NO: 30 - protein, 329 aa, synthetic construct
ASTKGPSVFPLAPSSKSTSGGTAALGCLVKDYFPEPVTVSWNSGALTSGVHTFPAVLQSSGLYSLSSVVTVPSSSLGTQTYICNVNHKPSNTKVDKKVEPKSCDKTHTCPPCPAPESTRGPSVFLFPPKPKDTLMISRTPEVTCVVVDVSHEDPEVKFNWYVDGVEVHNAKTKPREEQYNSTYRVVSVLTVLHQDWLNGKEYKCKVSNKALPAPIEKTISKAKGQPREPQVYTLPPSRDELTKNQVSLTCLVKGFYPSDIAVEWESNGQPENNYKTTPPVLDSDGSFFLYSKLTVDKSRWQQGNVFSCSVMHEALHNHYTQKSLSLSPG

SEQ ID NO: 31 - protein, 330 aa, synthetic construct
ASTKGPSVFPLAPSSKSTSGGTAALGCLVKDYFPEPVTVSWNSGALTSGVHTFPAVLQSSGLYSLSSVVTVPSSSLGTQTYICNVNHKPSNTKVDKKVEPKSCDKTHTCPPCPAPEAAGGPSVFLFPPKPKDTLMISRTPEVTCVVVDVSHEDPEVKFNWYVDGVEVHNAKTKPREEQYNSTYRVVSVLTVLHQDWLNGKEYKCKVSNKALPAPIEKTISKAKGQPREPQVYTLPPSRDELTKNQVSLTCLVKGFYPSDIAVEWESNGQPENNYKTTPPVLDSDGSFFLYSKLTVDKSRWQQGNVFSCSVMHEALHNHYTQKSLSLSPGK

SEQ ID NO: 32 - protein, 329 aa, synthetic construct
ASTKGPSVFPLAPSSKSTSGGTAALGCLVKDYFPEPVTVSWNSGALTSGVHTFPAVLQSSGLYSLSSVVTVPSSSLGTQTYICNVNHKPSNTKVDKKVEPKSCDKTHTCPPCPAPEAAGGPSVFLFPPKPKDTLMISRTPEVTCVVVDVSHEDPEVKFNWYVDGVEVHNAKTKPREEQYNSTYRVVSVLTVLHQDWLNGKEYKCKVSNKALPAPIEKTISKAKGQPREPQVYTLPPSRDELTKNQVSLTCLVKGFYPSDIAVEWESNGQPENNYKTTPPVLDSDGSFFLYSKLTVDKSRWQQGNVFSCSVMHEALHNHYTQKSLSLSPG

SEQ ID NO: 33 - protein, 330 aa, synthetic construct
ASTKGPSVFPLAPSSKSTSGGTAALGCLVKDYFPEPVTVSWNSGALTSGVHTFPAVLQSSGLYSLSSVVTVPSSSLGTQTYICNVNHKPSNTKVDKKVEPKSCDKTHTCPPCPAPELLGGPSVFLFPPKPKDTLYITREPEVTCVVVDVSHEDPEVKFNWYVDGVEVHNAKTKPREEQYNSTYRVVSVLTVLHQDWLNGKEYKCKVSNKALPAPIEKTISKAKGQPREPQVYTLPPSRDELTKNQVSLTCLVKGFYPSDIAVEWESNGQPENNYKTTPPVLDSDGSFFLYSKLTVDKSRWQQGNVFSCSVMHEALHNHYTQKSLSLSPGK

SEQ ID NO: 34 - protein, 329 aa, synthetic construct
ASTKGPSVFPLAPSSKSTSGGTAALGCLVKDYFPEPVTVSWNSGALTSGVHTFPAVLQSSGLYSLSSVVTVPSSSLGTQTYICNVNHKPSNTKVDKKVEPKSCDKTHTCPPCPAPELLGGPSVFLFPPKPKDTLYITREPEVTCVVVDVSHEDPEVKFNWYVDGVEVHNAKTKPREEQYNSTYRVVSVLTVLHQDWLNGKEYKCKVSNKALPAPIEKTISKAKGQPREPQVYTLPPSRDELTKNQVSLTCLVKGFYPSDIAVEWESNGQPENNYKTTPPVLDSDGSFFLYSKLTVDKSRWQQGNVFSCSVMHEALHNHYTQKSLSLSPG

SEQ ID NO: 35 - protein, 330 aa, synthetic construct
ASTKGPSVFPLAPSSKSTSGGTAALGCLVKDYFPEPVTVSWNSGALTSGVHTFPAVLQSSGLYSLSSVVTVPSSSLGTQTYICNVNHKPSNTKVDKKVEPKSCDKTHTCPPCPAPESTRGPSVFLFPPKPKDTLYITREPEVTCVVVDVSHEDPEVKFNWYVDGVEVHNAKTKPREEQYNSTYRVVSVLTVLHQDWLNGKEYKCKVSNKALPAPIEKTISKAKGQPREPQVYTLPPSRDELTKNQVSLTCLVKGFYPSDIAVEWESNGQPENNYKTTPPVLDSDGSFFLYSKLTVDKSRWQQGNVFSCSVMHEALHNHYTQKSLSLSPGK

SEQ ID NO: 36 - protein, 329 aa, synthetic construct
ASTKGPSVFPLAPSSKSTSGGTAALGCLVKDYFPEPVTVSWNSGALTSGVHTFPAVLQSSGLYSLSSVVTVPSSSLGTQTYICNVNHKPSNTKVDKKVEPKSCDKTHTCPPCPAPESTRGPSVFLFPPKPKDTLYITREPEVTCVVVDVSHEDPEVKFNWYVDGVEVHNAKTKPREEQYNSTYRVVSVLTVLHQDWLNGKEYKCKVSNKALPAPIEKTISKAKGQPREPQVYTLPPSRDELTKNQVSLTCLVKGFYPSDIAVEWESNGQPENNYKTTPPVLDSDGSFFLYSKLTVDKSRWQQGNVFSCSVMHEALHNHYTQKSLSLSPG

SEQ ID NO: 37 - protein, 330 aa, synthetic construct
ASTKGPSVFPLAPSSKSTSGGTAALGCLVKDYFPEPVTVSWNSGALTSGVHTFPAVLQSSGLYSLSSVVTVPSSSLGTQTYICNVNHKPSNTKVDKKVEPKSCDKTHTCPPCPAPEAAGGPSVFLFPPKPKDTLYITREPEVTCVVVDVSHEDPEVKFNWYVDGVEVHNAKTKPREEQYNSTYRVVSVLTVLHQDWLNGKEYKCKVSNKALPAPIEKTISKAKGQPREPQVYTLPPSRDELTKNQVSLTCLVKGFYPSDIAVEWESNGQPENNYKTTPPVLDSDGSFFLYSKLTVDKSRWQQGNVFSCSVMHEALHNHYTQKSLSLSPGK

SEQ ID NO: 38 - protein, 329 aa, synthetic construct
ASTKGPSVFPLAPSSKSTSGGTAALGCLVKDYFPEPVTVSWNSGALTSGVHTFPAVLQSSGLYSLSSVVTVPSSSLGTQTYICNVNHKPSNTKVDKKVEPKSCDKTHTCPPCPAPEAAGGPSVFLFPPKPKDTLYITREPEVTCVVVDVSHEDPEVKFNWYVDGVEVHNAKTKPREEQYNSTYRVVSVLTVLHQDWLNGKEYKCKVSNKALPAPIEKTISKAKGQPREPQVYTLPPSRDELTKNQVSLTCLVKGFYPSDIAVEWESNGQPENNYKTTPPVLDSDGSFFLYSKLTVDKSRWQQGNVFSCSVMHEALHNHYTQKSLSLSPG

SEQ ID NO: 39 - protein, 330 aa, synthetic construct
ASTKGPSVFPLAPSSKSTSGGTAALGCLVKDYFPEPVTVSWNSGALTSGVHTFPAVLQSSGLYSLSSVVTVPSSSLGTQTYICNVNHKPSNTKVDKKVEPKSCDKTHTCPPCPAPELLGGPSVFLFPPKPKDTLMISRTPEVTCVVVDVSHEDPEVKFNWYVDGVEVHNAKTKPREEQYNSTYRVVSVLTVLHRDWLNGKEYKCKVSNKALPAPIEKTISKAKGQPREPQVYTLPPSRDELTKNQVSLTCLVKGFYPSDIAVEWESNGQPENNYKTTPPVLDSDGSFFLYSKLTVDKSRWQQGNVFSCSVEHEALHWHYTQKSLSLSPGK

SEQ ID NO: 40 - protein, 329 aa, synthetic construct
ASTKGPSVFPLAPSSKSTSGGTAALGCLVKDYFPEPVTVSWNSGALTSGVHTFPAVLQSSGLYSLSSVVTVPSSSLGTQTYICNVNHKPSNTKVDKKVEPKSCDKTHTCPPCPAPELLGGPSVFLFPPKPKDTLMISRTPEVTCVVVDVSHEDPEVKFNWYVDGVEVHNAKTKPREEQYNSTYRVVSVLTVLHRDWLNGKEYKCKVSNKALPAPIEKTISKAKGQPREPQVYTLPPSRDELTKNQVSLTCLVKGFYPSDIAVEWESNGQPENNYKTTPPVLDSDGSFFLYSKLTVDKSRWQQGNVFSCSVEHEALHWHYTQKSLSLSPG

SEQ ID NO: 41 - protein, 330 aa, synthetic construct
ASTKGPSVFPLAPSSKSTSGGTAALGCLVKDYFPEPVTVSWNSGALTSGVHTFPAVLQSSGLYSLSSVVTVPSSSLGTQTYICNVNHKPSNTKVDKKVEPKSCDKTHTCPPCPAPESTRGPSVFLFPPKPKDTLMISRTPEVTCVVVDVSHEDPEVKFNWYVDGVEVHNAKTKPREEQYNSTYRVVSVLTVLHRDWLNGKEYKCKVSNKALPAPIEKTISKAKGQPREPQVYTLPPSRDELTKNQVSLTCLVKGFYPSDIAVEWESNGQPENNYKTTPPVLDSDGSFFLYSKLTVDKSRWQQGNVFSCSVEHEALHWHYTQKSLSLSPGK

SEQ ID NO: 42 - protein, 329 aa, synthetic construct
ASTKGPSVFPLAPSSKSTSGGTAALGCLVKDYFPEPVTVSWNSGALTSGVHTFPAVLQSSGLYSLSSVVTVPSSSLGTQTYICNVNHKPSNTKVDKKVEPKSCDKTHTCPPCPAPESTRGPSVFLFPPKPKDTLMISRTPEVTCVVVDVSHEDPEVKFNWYVDGVEVHNAKTKPREEQYNSTYRVVSVLTVLHRDWLNGKEYKCKVSNKALPAPIEKTISKAKGQPREPQVYTLPPSRDELTKNQVSLTCLVKGFYPSDIAVEWESNGQPENNYKTTPPVLDSDGSFFLYSKLTVDKSRWQQGNVFSCSVEHEALHWHYTQKSLSLSPG

SEQ ID NO: 43 - protein, 330 aa, synthetic construct
ASTKGPSVFPLAPSSKSTSGGTAALGCLVKDYFPEPVTVSWNSGALTSGVHTFPAVLQSSGLYSLSSVVTVPSSSLGTQTYICNVNHKPSNTKVDKKVEPKSCDKTHTCPPCPAPEAAGGPSVFLFPPKPKDTLMISRTPEVTCVVVDVSHEDPEVKFNWYVDGVEVHNAKTKPREEQYNSTYRVVSVLTVLHRDWLNGKEYKCKVSNKALPAPIEKTISKAKGQPREPQVYTLPPSRDELTKNQVSLTCLVKGFYPSDIAVEWESNGQPENNYKTTPPVLDSDGSFFLYSKLTVDKSRWQQGNVFSCSVEHEALHWHYTQKSLSLSPGK

SEQ ID NO: 44 - protein, 329 aa, synthetic construct
ASTKGPSVFPLAPSSKSTSGGTAALGCLVKDYFPEPVTVSWNSGALTSGVHTFPAVLQSSGLYSLSSVVTVPSSSLGTQTYICNVNHKPSNTKVDKKVEPKSCDKTHTCPPCPAPEAAGGPSVFLFPPKPKDTLMISRTPEVTCVVVDVSHEDPEVKFNWYVDGVEVHNAKTKPREEQYNSTYRVVSVLTVLHRDWLNGKEYKCKVSNKALPAPIEKTISKAKGQPREPQVYTLPPSRDELTKNQVSLTCLVKGFYPSDIAVEWESNGQPENNYKTTPPVLDSDGSFFLYSKLTVDKSRWQQGNVFSCSVEHEALHWHYTQKSLSLSPG

SEQ ID NO: 45 - protein, 330 aa, synthetic construct
ASTKGPSVFPLAPSSKSTSGGTAALGCLVKDYFPEPVTVSWNSGALTSGVHTFPAVLQSSGLYSLSSVVTVPSSSLGTQTYICNVNHKPSNTKVDKKVEPKSCDKTHTCPPCPAPELLGGPSVFLFPPKPKDTLMISRTPEVTCVVVDVSHEDPEVKFNWYVDGVEVHNAKTKPREEQYNSTYRVVSVLTVLHQDWLNGKEYKCKVSNKALPAPIEKTISKAKGQPREPQVYTLPPSRDELTKNQVSLTCLVKGFYPSDIAVEWESNGQPENNYKTTPPVLDSDGSFFLYSKLTVDKSRWQQGNVFSCSVLHEALHSHYTQKSLSLSPGK

SEQ ID NO: 46 - protein, 329 aa, synthetic construct
ASTKGPSVFPLAPSSKSTSGGTAALGCLVKDYFPEPVTVSWNSGALTSGVHTFPAVLQSSGLYSLSSVVTVPSSSLGTQTYICNVNHKPSNTKVDKKVEPKSCDKTHTCPPCPAPELLGGPSVFLFPPKPKDTLMISRTPEVTCVVVDVSHEDPEVKFNWYVDGVEVHNAKTKPREEQYNSTYRVVSVLTVLHQDWLNGKEYKCKVSNKALPAPIEKTISKAKGQPREPQVYTLPPSRDELTKNQVSLTCLVKGFYPSDIAVEWESNGQPENNYKTTPPVLDSDGSFFLYSKLTVDKSRWQQGNVFSCSVLHEALHSHYTQKSLSLSPG

SEQ ID NO: 47 - protein, 330 aa, synthetic construct
ASTKGPSVFPLAPSSKSTSGGTAALGCLVKDYFPEPVTVSWNSGALTSGVHTFPAVLQSSGLYSLSSVVTVPSSSLGTQTYICNVNHKPSNTKVDKKVEPKSCDKTHTCPPCPAPESTRGPSVFLFPPKPKDTLMISRTPEVTCVVVDVSHEDPEVKFNWYVDGVEVHNAKTKPREEQYNSTYRVVSVLTVLHQDWLNGKEYKCKVSNKALPAPIEKTISKAKGQPREPQVYTLPPSRDELTKNQVSLTCLVKGFYPSDIAVEWESNGQPENNYKTTPPVLDSDGSFFLYSKLTVDKSRWQQGNVFSCSVLHEALHSHYTQKSLSLSPGK

SEQ ID NO: 48 - protein, 329 aa, synthetic construct
ASTKGPSVFPLAPSSKSTSGGTAALGCLVKDYFPEPVTVSWNSGALTSGVHTFPAVLQSSGLYSLSSVVTVPSSSLGTQTYICNVNHKPSNTKVDKKVEPKSCDKTHTCPPCPAPESTRGPSVFLFPPKPKDTLMISRTPEVTCVVVDVSHEDPEVKFNWYVDGVEVHNAKTKPREEQYNSTYRVVSVLTVLHQDWLNGKEYKCKVSNKALPAPIEKTISKAKGQPREPQVYTLPPSRDELTKNQVSLTCLVKGFYPSDIAVEWESNGQPENNYKTTPPVLDSDGSFFLYSKLTVDKSRWQQGNVFSCSVLHEALHSHYTQKSLSLSPG

SEQ ID NO: 49 - protein, 330 aa, synthetic construct
ASTKGPSVFPLAPSSKSTSGGTAALGCLVKDYFPEPVTVSWNSGALTSGVHTFPAVLQSSGLYSLSSVVTVPSSSLGTQTYICNVNHKPSNTKVDKKVEPKSCDKTHTCPPCPAPEAAGGPSVFLFPPKPKDTLMISRTPEVTCVVVDVSHEDPEVKFNWYVDGVEVHNAKTKPREEQYNSTYRVVSVLTVLHQDWLNGKEYKCKVSNKALPAPIEKTISKAKGQPREPQVYTLPPSRDELTKNQVSLTCLVKGFYPSDIAVEWESNGQPENNYKTTPPVLDSDGSFFLYSKLTVDKSRWQQGNVFSCSVLHEALHSHYTQKSLSLSPGK

SEQ ID NO: 50 - protein, 329 aa, synthetic construct
ASTKGPSVFPLAPSSKSTSGGTAALGCLVKDYFPEPVTVSWNSGALTSGVHTFPAVLQSSGLYSLSSVVTVPSSSLGTQTYICNVNHKPSNTKVDKKVEPKSCDKTHTCPPCPAPEAAGGPSVFLFPPKPKDTLMISRTPEVTCVVVDVSHEDPEVKFNWYVDGVEVHNAKTKPREEQYNSTYRVVSVLTVLHQDWLNGKEYKCKVSNKALPAPIEKTISKAKGQPREPQVYTLPPSRDELTKNQVSLTCLVKGFYPSDIAVEWESNGQPENNYKTTPPVLDSDGSFFLYSKLTVDKSRWQQGNVFSCSVLHEALHSHYTQKSLSLSPG

SEQ ID NO: 51 - protein, 330 aa, synthetic construct
ASTKGPSVFPLAPSSKSTSGGTAALGCLVKDYFPEPVTVSWNSGALTSGVHTFPAVLQSSGLYSLSSVVTVPSSSLGTQTYICNVNHKPSNTKVDKKVEPKSCDKTHTCPPCPAPELLGGPSVFLFPPKPKDQLMISRTPEVTCVVVDVSHEDPEVKFNWYVDGVEVHNAKTKPREEQYNSTYRVVSVLTVLHQDWLNGKEYKCKVSNKALPAPIEKTISKAKGQPREPQVYTLPPSRDELTKNQVSLTCLVKGFYPSDIAVEWESNGQPENNYKTTPPVLDSDGSFFLYSKLTVDKSRWQQGNVFSCSVLHEALHNHYTQKSLSLSPGK

SEQ ID NO: 52 - protein, 329 aa, synthetic construct
ASTKGPSVFPLAPSSKSTSGGTAALGCLVKDYFPEPVTVSWNSGALTSGVHTFPAVLQSSGLYSLSSVVTVPSSSLGTQTYICNVNHKPSNTKVDKKVEPKSCDKTHTCPPCPAPELLGGPSVFLFPPKPKDQLMISRTPEVTCVVVDVSHEDPEVKFNWYVDGVEVHNAKTKPREEQYNSTYRVVSVLTVLHQDWLNGKEYKCKVSNKALPAPIEKTISKAKGQPREPQVYTLPPSRDELTKNQVSLTCLVKGFYPSDIAVEWESNGQPENNYKTTPPVLDSDGSFFLYSKLTVDKSRWQQGNVFSCSVLHEALHNHYTQKSLSLSPG

SEQ ID NO: 53 - protein, 330 aa, synthetic construct
ASTKGPSVFPLAPSSKSTSGGTAALGCLVKDYFPEPVTVSWNSGALTSGVHTFPAVLQSSGLYSLSSVVTVPSSSLGTQTYICNVNHKPSNTKVDKKVEPKSCDKTHTCPPCPAPESTRGPSVFLFPPKPKDQLMISRTPEVTCVVVDVSHEDPEVKFNWYVDGVEVHNAKTKPREEQYNSTYRVVSVLTVLHQDWLNGKEYKCKVSNKALPAPIEKTISKAKGQPREPQVYTLPPSRDELTKNQVSLTCLVKGFYPSDIAVEWESNGQPENNYKTTPPVLDSDGSFFLYSKLTVDKSRWQQGNVFSCSVLHEALHNHYTQKSLSLSPGK

SEQ ID NO: 54 - protein, 329 aa, synthetic construct
ASTKGPSVFPLAPSSKSTSGGTAALGCLVKDYFPEPVTVSWNSGALTSGVHTFPAVLQSSGLYSLSSVVTVPSSSLGTQTYICNVNHKPSNTKVDKKVEPKSCDKTHTCPPCPAPESTRGPSVFLFPPKPKDQLMISRTPEVTCVVVDVSHEDPEVKFNWYVDGVEVHNAKTKPREEQYNSTYRVVSVLTVLHQDWLNGKEYKCKVSNKALPAPIEKTISKAKGQPREPQVYTLPPSRDELTKNQVSLTCLVKGFYPSDIAVEWESNGQPENNYKTTPPVLDSDGSFFLYSKLTVDKSRWQQGNVFSCSVLHEALHNHYTQKSLSLSPG

SEQ ID NO: 55 - protein, 330 aa, synthetic construct
ASTKGPSVFPLAPSSKSTSGGTAALGCLVKDYFPEPVTVSWNSGALTSGVHTFPAVLQSSGLYSLSSVVTVPSSSLGTQTYICNVNHKPSNTKVDKKVEPKSCDKTHTCPPCPAPEAAGGPSVFLFPPKPKDQLMISRTPEVTCVVVDVSHEDPEVKFNWYVDGVEVHNAKTKPREEQYNSTYRVVSVLTVLHQDWLNGKEYKCKVSNKALPAPIEKTISKAKGQPREPQVYTLPPSRDELTKNQVSLTCLVKGFYPSDIAVEWESNGQPENNYKTTPPVLDSDGSFFLYSKLTVDKSRWQQGNVFSCSVLHEALHNHYTQKSLSLSPGK

SEQ ID NO: 56 - protein, 329 aa, synthetic construct
ASTKGPSVFPLAPSSKSTSGGTAALGCLVKDYFPEPVTVSWNSGALTSGVHTFPAVLQSSGLYSLSSVVTVPSSSLGTQTYICNVNHKPSNTKVDKKVEPKSCDKTHTCPPCPAPEAAGGPSVFLFPPKPKDQLMISRTPEVTCVVVDVSHEDPEVKFNWYVDGVEVHNAKTKPREEQYNSTYRVVSVLTVLHQDWLNGKEYKCKVSNKALPAPIEKTISKAKGQPREPQVYTLPPSRDELTKNQVSLTCLVKGFYPSDIAVEWESNGQPENNYKTTPPVLDSDGSFFLYSKLTVDKSRWQQGNVFSCSVLHEALHNHYTQKSLSLSPG

SEQ ID NO: 57 - protein, 330 aa, synthetic construct
ASTKGPSVFPLAPSSKSTSGGTAALGCLVKDYFPEPVTVSWNSGALTSGVHTFPAVLQSSGLYSLSSVVTVPSSSLGTQTYICNVNHKPSNTKVDKKVEPKSCDKTHTCPPCPAPELLGGPSVFLFPPKPKDTLMISRTPEVTCVVVDVSHEDPEVKFNWYVDGVEVHNAKTKPREEQYNSTYRVVSVLTVDHHDWLNGKEYKCKVSNKALPAPIEKTISKAKGQPREPQVYTLPPSRDELTKNQVSLTCLVKGFYPSDIAVEWESNGQPENNYKTTPPVLDSDGSFFLYSKLTVDKSRWQQGNVFSCSVMHEALHSHYTQKSLSLSPGK

SEQ ID NO: 58 - protein, 329 aa, synthetic construct
ASTKGPSVFPLAPSSKSTSGGTAALGCLVKDYFPEPVTVSWNSGALTSGVHTFPAVLQSSGLYSLSSVVTVPSSSLGTQTYICNVNHKPSNTKVDKKVEPKSCDKTHTCPPCPAPELLGGPSVFLFPPKPKDTLMISRTPEVTCVVVDVSHEDPEVKFNWYVDGVEVHNAKTKPREEQYNSTYRVVSVLTVDHHDWLNGKEYKCKVSNKALPAPIEKTISKAKGQPREPQVYTLPPSRDELTKNQVSLTCLVKGFYPSDIAVEWESNGQPENNYKTTPPVLDSDGSFFLYSKLTVDKSRWQQGNVFSCSVMHEALHSHYTQKSLSLSPG

SEQ ID NO: 59 - protein, 330 aa, synthetic construct
ASTKGPSVFPLAPSSKSTSGGTAALGCLVKDYFPEPVTVSWNSGALTSGVHTFPAVLQSSGLYSLSSVVTVPSSSLGTQTYICNVNHKPSNTKVDKKVEPKSCDKTHTCPPCPAPESTRGPSVFLFPPKPKDTLMISRTPEVTCVVVDVSHEDPEVKFNWYVDGVEVHNAKTKPREEQYNSTYRVVSVLTVDHHDWLNGKEYKCKVSNKALPAPIEKTISKAKGQPREPQVYTLPPSRDELTKNQVSLTCLVKGFYPSDIAVEWESNGQPENNYKTTPPVLDSDGSFFLYSKLTVDKSRWQQGNVFSCSVMHEALHSHYTQKSLSLSPGK

SEQ ID NO: 60 - protein, 329 aa, synthetic construct
ASTKGPSVFPLAPSSKSTSGGTAALGCLVKDYFPEPVTVSWNSGALTSGVHTFPAVLQSSGLYSLSSVVTVPSSSLGTQTYICNVNHKPSNTKVDKKVEPKSCDKTHTCPPCPAPESTRGPSVFLFPPKPKDTLMISRTPEVTCVVVDVSHEDPEVKFNWYVDGVEVHNAKTKPREEQYNSTYRVVSVLTVDHHDWLNGKEYKCKVSNKALPAPIEKTISKAKGQPREPQVYTLPPSRDELTKNQVSLTCLVKGFYPSDIAVEWESNGQPENNYKTTPPVLDSDGSFFLYSKLTVDKSRWQQGNVFSCSVMHEALHSHYTQKSLSLSPG

SEQ ID NO: 61 - protein, 330 aa, synthetic construct
ASTKGPSVFPLAPSSKSTSGGTAALGCLVKDYFPEPVTVSWNSGALTSGVHTFPAVLQSSGLYSLSSVVTVPSSSLGTQTYICNVNHKPSNTKVDKKVEPKSCDKTHTCPPCPAPEAAGGPSVFLFPPKPKDTLMISRTPEVTCVVVDVSHEDPEVKFNWYVDGVEVHNAKTKPREEQYNSTYRVVSVLTVDHHDWLNGKEYKCKVSNKALPAPIEKTISKAKGQPREPQVYTLPPSRDELTKNQVSLTCLVKGFYPSDIAVEWESNGQPENNYKTTPPVLDSDGSFFLYSKLTVDKSRWQQGNVFSCSVMHEALHSHYTQKSLSLSPGK

SEQ ID NO: 62 - protein, 329 aa, synthetic construct
ASTKGPSVFPLAPSSKSTSGGTAALGCLVKDYFPEPVTVSWNSGALTSGVHTFPAVLQSSGLYSLSSVVTVPSSSLGTQTYICNVNHKPSNTKVDKKVEPKSCDKTHTCPPCPAPEAAGGPSVFLFPPKPKDTLMISRTPEVTCVVVDVSHEDPEVKFNWYVDGVEVHNAKTKPREEQYNSTYRVVSVLTVDHHDWLNGKEYKCKVSNKALPAPIEKTISKAKGQPREPQVYTLPPSRDELTKNQVSLTCLVKGFYPSDIAVEWESNGQPENNYKTTPPVLDSDGSFFLYSKLTVDKSRWQQGNVFSCSVMHEALHSHYTQKSLSLSPG

SEQ ID NO: 63 - protein, 327 aa, synthetic construct
ASTKGPSVFPLAPCSRSTSESTAALGCLVKDYFPEPVTVSWNSGALTSGVHTFPAVLQSSGLYSLSSVVTVPSSSLGTKTYTCNVDHKPSNTKVDKRVESKYGPPCPPCPAPEFLGGPSVFLFPPKPKDTLMISRTPEVTCVVVDVSQEDPEVQFNWYVDGVEVHNAKTKPREEQFNSTYRVVSVLTVLHQDWLNGKEYKCKVSNKGLPSSIEKTISKAKGQPREPQVYTLPPSQEEMTKNQVSLTCLVKGFYPSDIAVEWESNGQPENNYKTTPPVLDSDGSFFLYSRLTVDKSRWQEGNVFSCSVMHEALHNHYTQKSLSLSLGK

SEQ ID NO: 64 - protein, 326 aa, synthetic construct
ASTKGPSVFPLAPCSRSTSESTAALGCLVKDYFPEPVTVSWNSGALTSGVHTFPAVLQSSGLYSLSSVVTVPSSSLGTKTYTCNVDHKPSNTKVDKRVESKYGPPCPPCPAPEFLGGPSVFLFPPKPKDTLMISRTPEVTCVVVDVSQEDPEVQFNWYVDGVEVHNAKTKPREEQFNSTYRVVSVLTVLHQDWLNGKEYKCKVSNKGLPSSIEKTISKAKGQPREPQVYTLPPSQEEMTKNQVSLTCLVKGFYPSDIAVEWESNGQPENNYKTTPPVLDSDGSFFLYSRLTVDKSRWQEGNVFSCSVMHEALHNHYTQKSLSLSLG

SEQ ID NO: 65 - protein, 327 aa, synthetic construct
ASTKGPSVFPLAPCSRSTSESTAALGCLVKDYFPEPVTVSWNSGALTSGVHTFPAVLQSSGLYSLSSVVTVPSSSLGTKTYTCNVDHKPSNTKVDKRVESKYGPPCPPCPAPESTRGPSVFLFPPKPKDTLMISRTPEVTCVVVDVSQEDPEVQFNWYVDGVEVHNAKTKPREEQFNSTYRVVSVLTVLHQDWLNGKEYKCKVSNKGLPSSIEKTISKAKGQPREPQVYTLPPSQEEMTKNQVSLTCLVKGFYPSDIAVEWESNGQPENNYKTTPPVLDSDGSFFLYSRLTVDKSRWQEGNVFSCSVMHEALHNHYTQKSLSLSLGK

SEQ ID NO: 66 - protein, 326 aa, synthetic construct
ASTKGPSVFPLAPCSRSTSESTAALGCLVKDYFPEPVTVSWNSGALTSGVHTFPAVLQSSGLYSLSSVVTVPSSSLGTKTYTCNVDHKPSNTKVDKRVESKYGPPCPPCPAPESTRGPSVFLFPPKPKDTLMISRTPEVTCVVVDVSQEDPEVQFNWYVDGVEVHNAKTKPREEQFNSTYRVVSVLTVLHQDWLNGKEYKCKVSNKGLPSSIEKTISKAKGQPREPQVYTLPPSQEEMTKNQVSLTCLVKGFYPSDIAVEWESNGQPENNYKTTPPVLDSDGSFFLYSRLTVDKSRWQEGNVFSCSVMHEALHNHYTQKSLSLSLG

SEQ ID NO: 67 - protein, 327 aa, synthetic construct
ASTKGPSVFPLAPCSRSTSESTAALGCLVKDYFPEPVTVSWNSGALTSGVHTFPAVLQSSGLYSLSSVVTVPSSSLGTKTYTCNVDHKPSNTKVDKRVESKYGPPCPPCPAPEAAGGPSVFLFPPKPKDTLMISRTPEVTCVVVDVSQEDPEVQFNWYVDGVEVHNAKTKPREEQFNSTYRVVSVLTVLHQDWLNGKEYKCKVSNKGLPSSIEKTISKAKGQPREPQVYTLPPSQEEMTKNQVSLTCLVKGFYPSDIAVEWESNGQPENNYKTTPPVLDSDGSFFLYSRLTVDKSRWQEGNVFSCSVMHEALHNHYTQKSLSLSLGK

SEQ ID NO: 68 - protein, 326 aa, synthetic construct
ASTKGPSVFPLAPCSRSTSESTAALGCLVKDYFPEPVTVSWNSGALTSGVHTFPAVLQSSGLYSLSSVVTVPSSSLGTKTYTCNVDHKPSNTKVDKRVESKYGPPCPPCPAPEAAGGPSVFLFPPKPKDTLMISRTPEVTCVVVDVSQEDPEVQFNWYVDGVEVHNAKTKPREEQFNSTYRVVSVLTVLHQDWLNGKEYKCKVSNKGLPSSIEKTISKAKGQPREPQVYTLPPSQEEMTKNQVSLTCLVKGFYPSDIAVEWESNGQPENNYKTTPPVLDSDGSFFLYSRLTVDKSRWQEGNVFSCSVMHEALHNHYTQKSLSLSLG

SEQ ID NO: 69 - protein, 327 aa, synthetic construct
ASTKGPSVFPLAPCSRSTSESTAALGCLVKDYFPEPVTVSWNSGALTSGVHTFPAVLQSSGLYSLSSVVTVPSSSLGTKTYTCNVDHKPSNTKVDKRVESKYGPPCPPCPAPEFLGGPSVFLFPPKPKDTLYITREPEVTCVVVDVSQEDPEVQFNWYVDGVEVHNAKTKPREEQFNSTYRVVSVLTVLHQDWLNGKEYKCKVSNKGLPSSIEKTISKAKGQPREPQVYTLPPSQEEMTKNQVSLTCLVKGFYPSDIAVEWESNGQPENNYKTTPPVLDSDGSFFLYSRLTVDKSRWQEGNVFSCSVMHEALHNHYTQKSLSLSLGK

SEQ ID NO: 70 - protein, 326 aa, synthetic construct
ASTKGPSVFPLAPCSRSTSESTAALGCLVKDYFPEPVTVSWNSGALTSGVHTFPAVLQSSGLYSLSSVVTVPSSSLGTKTYTCNVDHKPSNTKVDKRVESKYGPPCPPCPAPEFLGGPSVFLFPPKPKDTLYITREPEVTCVVVDVSQEDPEVQFNWYVDGVEVHNAKTKPREEQFNSTYRVVSVLTVLHQDWLNGKEYKCKVSNKGLPSSIEKTISKAKGQPREPQVYTLPPSQEEMTKNQVSLTCLVKGFYPSDIAVEWESNGQPENNYKTTPPVLDSDGSFFLYSRLTVDKSRWQEGNVFSCSVMHEALHNHYTQKSLSLSLG

SEQ ID NO: 71 - protein, 327 aa, synthetic construct
ASTKGPSVFPLAPCSRSTSESTAALGCLVKDYFPEPVTVSWNSGALTSGVHTFPAVLQSSGLYSLSSVVTVPSSSLGTKTYTCNVDHKPSNTKVDKRVESKYGPPCPPCPAPESTRGPSVFLFPPKPKDTLYITREPEVTCVVVDVSQEDPEVQFNWYVDGVEVHNAKTKPREEQFNSTYRVVSVLTVLHQDWLNGKEYKCKVSNKGLPSSIEKTISKAKGQPREPQVYTLPPSQEEMTKNQVSLTCLVKGFYPSDIAVEWESNGQPENNYKTTPPVLDSDGSFFLYSRLTVDKSRWQEGNVFSCSVMHEALHNHYTQKSLSLSLGK

SEQ ID NO: 72 - protein, 326 aa, synthetic construct
ASTKGPSVFPLAPCSRSTSESTAALGCLVKDYFPEPVTVSWNSGALTSGVHTFPAVLQSSGLYSLSSVVTVPSSSLGTKTYTCNVDHKPSNTKVDKRVESKYGPPCPPCPAPESTRGPSVFLFPPKPKDTLYITREPEVTCVVVDVSQEDPEVQFNWYVDGVEVHNAKTKPREEQFNSTYRVVSVLTVLHQDWLNGKEYKCKVSNKGLPSSIEKTISKAKGQPREPQVYTLPPSQEEMTKNQVSLTCLVKGFYPSDIAVEWESNGQPENNYKTTPPVLDSDGSFFLYSRLTVDKSRWQEGNVFSCSVMHEALHNHYTQKSLSLSLG

SEQ ID NO: 73 - protein, 327 aa, synthetic construct
ASTKGPSVFPLAPCSRSTSESTAALGCLVKDYFPEPVTVSWNSGALTSGVHTFPAVLQSSGLYSLSSVVTVPSSSLGTKTYTCNVDHKPSNTKVDKRVESKYGPPCPPCPAPEAAGGPSVFLFPPKPKDTLYITREPEVTCVVVDVSQEDPEVQFNWYVDGVEVHNAKTKPREEQFNSTYRVVSVLTVLHQDWLNGKEYKCKVSNKGLPSSIEKTISKAKGQPREPQVYTLPPSQEEMTKNQVSLTCLVKGFYPSDIAVEWESNGQPENNYKTTPPVLDSDGSFFLYSRLTVDKSRWQEGNVFSCSVMHEALHNHYTQKSLSLSLGK

SEQ ID NO: 74 - protein, 326 aa, synthetic construct
ASTKGPSVFPLAPCSRSTSESTAALGCLVKDYFPEPVTVSWNSGALTSGVHTFPAVLQSSGLYSLSSVVTVPSSSLGTKTYTCNVDHKPSNTKVDKRVESKYGPPCPPCPAPEAAGGPSVFLFPPKPKDTLYITREPEVTCVVVDVSQEDPEVQFNWYVDGVEVHNAKTKPREEQFNSTYRVVSVLTVLHQDWLNGKEYKCKVSNKGLPSSIEKTISKAKGQPREPQVYTLPPSQEEMTKNQVSLTCLVKGFYPSDIAVEWESNGQPENNYKTTPPVLDSDGSFFLYSRLTVDKSRWQEGNVFSCSVMHEALHNHYTQKSLSLSLG

SEQ ID NO: 75 - protein, 327 aa, synthetic construct
ASTKGPSVFPLAPCSRSTSESTAALGCLVKDYFPEPVTVSWNSGALTSGVHTFPAVLQSSGLYSLSSVVTVPSSSLGTKTYTCNVDHKPSNTKVDKRVESKYGPPCPPCPAPEFLGGPSVFLFPPKPKDTLMISRTPEVTCVVVDVSQEDPEVQFNWYVDGVEVHNAKTKPREEQFNSTYRVVSVLTVLHRDWLNGKEYKCKVSNKGLPSSIEKTISKAKGQPREPQVYTLPPSQEEMTKNQVSLTCLVKGFYPSDIAVEWESNGQPENNYKTTPPVLDSDGSFFLYSRLTVDKSRWQEGNVFSCSVEHEALHWHYTQKSLSLSLGK

SEQ ID NO: 76 - protein, 326 aa, synthetic construct
ASTKGPSVFPLAPCSRSTSESTAALGCLVKDYFPEPVTVSWNSGALTSGVHTFPAVLQSSGLYSLSSVVTVPSSSLGTKTYTCNVDHKPSNTKVDKRVESKYGPPCPPCPAPEFLGGPSVFLFPPKPKDTLMISRTPEVTCVVVDVSQEDPEVQFNWYVDGVEVHNAKTKPREEQFNSTYRVVSVLTVLHRDWLNGKEYKCKVSNKGLPSSIEKTISKAKGQPREPQVYTLPPSQEEMTKNQVSLTCLVKGFYPSDIAVEWESNGQPENNYKTTPPVLDSDGSFFLYSRLTVDKSRWQEGNVFSCSVEHEALHWHYTQKSLSLSLG

SEQ ID NO: 77 - protein, 327 aa, synthetic construct
ASTKGPSVFPLAPCSRSTSESTAALGCLVKDYFPEPVTVSWNSGALTSGVHTFPAVLQSSGLYSLSSVVTVPSSSLGTKTYTCNVDHKPSNTKVDKRVESKYGPPCPPCPAPESTRGPSVFLFPPKPKDTLMISRTPEVTCVVVDVSQEDPEVQFNWYVDGVEVHNAKTKPREEQFNSTYRVVSVLTVLHRDWLNGKEYKCKVSNKGLPSSIEKTISKAKGQPREPQVYTLPPSQEEMTKNQVSLTCLVKGFYPSDIAVEWESNGQPENNYKTTPPVLDSDGSFFLYSRLTVDKSRWQEGNVFSCSVEHEALHWHYTQKSLSLSLGK

SEQ ID NO: 78 - protein, 326 aa, synthetic construct
ASTKGPSVFPLAPCSRSTSESTAALGCLVKDYFPEPVTVSWNSGALTSGVHTFPAVLQSSGLYSLSSVVTVPSSSLGTKTYTCNVDHKPSNTKVDKRVESKYGPPCPPCPAPESTRGPSVFLFPPKPKDTLMISRTPEVTCVVVDVSQEDPEVQFNWYVDGVEVHNAKTKPREEQFNSTYRVVSVLTVLHRDWLNGKEYKCKVSNKGLPSSIEKTISKAKGQPREPQVYTLPPSQEEMTKNQVSLTCLVKGFYPSDIAVEWESNGQPENNYKTTPPVLDSDGSFFLYSRLTVDKSRWQEGNVFSCSVEHEALHWHYTQKSLSLSLG

SEQ ID NO: 79 - protein, 327 aa, synthetic construct
ASTKGPSVFPLAPCSRSTSESTAALGCLVKDYFPEPVTVSWNSGALTSGVHTFPAVLQSSGLYSLSSVVTVPSSSLGTKTYTCNVDHKPSNTKVDKRVESKYGPPCPPCPAPEAAGGPSVFLFPPKPKDTLMISRTPEVTCVVVDVSQEDPEVQFNWYVDGVEVHNAKTKPREEQFNSTYRVVSVLTVLHRDWLNGKEYKCKVSNKGLPSSIEKTISKAKGQPREPQVYTLPPSQEEMTKNQVSLTCLVKGFYPSDIAVEWESNGQPENNYKTTPPVLDSDGSFFLYSRLTVDKSRWQEGNVFSCSVEHEALHWHYTQKSLSLSLGK

SEQ ID NO: 80 - protein, 326 aa, synthetic construct
ASTKGPSVFPLAPCSRSTSESTAALGCLVKDYFPEPVTVSWNSGALTSGVHTFPAVLQSSGLYSLSSVVTVPSSSLGTKTYTCNVDHKPSNTKVDKRVESKYGPPCPPCPAPEAAGGPSVFLFPPKPKDTLMISRTPEVTCVVVDVSQEDPEVQFNWYVDGVEVHNAKTKPREEQFNSTYRVVSVLTVLHRDWLNGKEYKCKVSNKGLPSSIEKTISKAKGQPREPQVYTLPPSQEEMTKNQVSLTCLVKGFYPSDIAVEWESNGQPENNYKTTPPVLDSDGSFFLYSRLTVDKSRWQEGNVFSCSVEHEALHWHYTQKSLSLSLG

SEQ ID NO: 81 - protein, 327 aa, synthetic construct
ASTKGPSVFPLAPCSRSTSESTAALGCLVKDYFPEPVTVSWNSGALTSGVHTFPAVLQSSGLYSLSSVVTVPSSSLGTKTYTCNVDHKPSNTKVDKRVESKYGPPCPPCPAPEFLGGPSVFLFPPKPKDTLMISRTPEVTCVVVDVSQEDPEVQFNWYVDGVEVHNAKTKPREEQFNSTYRVVSVLTVLHQDWLNGKEYKCKVSNKGLPSSIEKTISKAKGQPREPQVYTLPPSQEEMTKNQVSLTCLVKGFYPSDIAVEWESNGQPENNYKTTPPVLDSDGSFFLYSRLTVDKSRWQEGNVFSCSVLHEALHSHYTQKSLSLSLGK

SEQ ID NO: 82 - protein, 326 aa, synthetic construct
ASTKGPSVFPLAPCSRSTSESTAALGCLVKDYFPEPVTVSWNSGALTSGVHTFPAVLQSSGLYSLSSVVTVPSSSLGTKTYTCNVDHKPSNTKVDKRVESKYGPPCPPCPAPEFLGGPSVFLFPPKPKDTLMISRTPEVTCVVVDVSQEDPEVQFNWYVDGVEVHNAKTKPREEQFNSTYRVVSVLTVLHQDWLNGKEYKCKVSNKGLPSSIEKTISKAKGQPREPQVYTLPPSQEEMTKNQVSLTCLVKGFYPSDIAVEWESNGQPENNYKTTPPVLDSDGSFFLYSRLTVDKSRWQEGNVFSCSVLHEALHSHYTQKSLSLSLG

SEQ ID NO: 83 - protein, 327 aa, synthetic construct
ASTKGPSVFPLAPCSRSTSESTAALGCLVKDYFPEPVTVSWNSGALTSGVHTFPAVLQSSGLYSLSSVVTVPSSSLGTKTYTCNVDHKPSNTKVDKRVESKYGPPCPPCPAPESTRGPSVFLFPPKPKDTLMISRTPEVTCVVVDVSQEDPEVQFNWYVDGVEVHNAKTKPREEQFNSTYRVVSVLTVLHQDWLNGKEYKCKVSNKGLPSSIEKTISKAKGQPREPQVYTLPPSQEEMTKNQVSLTCLVKGFYPSDIAVEWESNGQPENNYKTTPPVLDSDGSFFLYSRLTVDKSRWQEGNVFSCSVLHEALHSHYTQKSLSLSLGK

SEQ ID NO: 84 - protein, 326 aa, synthetic construct
ASTKGPSVFPLAPCSRSTSESTAALGCLVKDYFPEPVTVSWNSGALTSGVHTFPAVLQSSGLYSLSSVVTVPSSSLGTKTYTCNVDHKPSNTKVDKRVESKYGPPCPPCPAPESTRGPSVFLFPPKPKDTLMISRTPEVTCVVVDVSQEDPEVQFNWYVDGVEVHNAKTKPREEQFNSTYRVVSVLTVLHQDWLNGKEYKCKVSNKGLPSSIEKTISKAKGQPREPQVYTLPPSQEEMTKNQVSLTCLVKGFYPSDIAVEWESNGQPENNYKTTPPVLDSDGSFFLYSRLTVDKSRWQEGNVFSCSVLHEALHSHYTQKSLSLSLG

SEQ ID NO: 85 - protein, 327 aa, synthetic construct
ASTKGPSVFPLAPCSRSTSESTAALGCLVKDYFPEPVTVSWNSGALTSGVHTFPAVLQSSGLYSLSSVVTVPSSSLGTKTYTCNVDHKPSNTKVDKRVESKYGPPCPPCPAPEAAGGPSVFLFPPKPKDTLMISRTPEVTCVVVDVSQEDPEVQFNWYVDGVEVHNAKTKPREEQFNSTYRVVSVLTVLHQDWLNGKEYKCKVSNKGLPSSIEKTISKAKGQPREPQVYTLPPSQEEMTKNQVSLTCLVKGFYPSDIAVEWESNGQPENNYKTTPPVLDSDGSFFLYSRLTVDKSRWQEGNVFSCSVLHEALHSHYTQKSLSLSLGK

SEQ ID NO: 86 - protein, 326 aa, synthetic construct
ASTKGPSVFPLAPCSRSTSESTAALGCLVKDYFPEPVTVSWNSGALTSGVHTFPAVLQSSGLYSLSSVVTVPSSSLGTKTYTCNVDHKPSNTKVDKRVESKYGPPCPPCPAPEAAGGPSVFLFPPKPKDTLMISRTPEVTCVVVDVSQEDPEVQFNWYVDGVEVHNAKTKPREEQFNSTYRVVSVLTVLHQDWLNGKEYKCKVSNKGLPSSIEKTISKAKGQPREPQVYTLPPSQEEMTKNQVSLTCLVKGFYPSDIAVEWESNGQPENNYKTTPPVLDSDGSFFLYSRLTVDKSRWQEGNVFSCSVLHEALHSHYTQKSLSLSLG

SEQ ID NO: 87 - protein, 327 aa, synthetic construct
ASTKGPSVFPLAPCSRSTSESTAALGCLVKDYFPEPVTVSWNSGALTSGVHTFPAVLQSSGLYSLSSVVTVPSSSLGTKTYTCNVDHKPSNTKVDKRVESKYGPPCPPCPAPEFLGGPSVFLFPPKPKDQLMISRTPEVTCVVVDVSQEDPEVQFNWYVDGVEVHNAKTKPREEQFNSTYRVVSVLTVLHQDWLNGKEYKCKVSNKGLPSSIEKTISKAKGQPREPQVYTLPPSQEEMTKNQVSLTCLVKGFYPSDIAVEWESNGQPENNYKTTPPVLDSDGSFFLYSRLTVDKSRWQEGNVFSCSVLHEALHNHYTQKSLSLSLGK

SEQ ID NO: 88 - protein, 326 aa, synthetic construct
ASTKGPSVFPLAPCSRSTSESTAALGCLVKDYFPEPVTVSWNSGALTSGVHTFPAVLQSSGLYSLSSVVTVPSSSLGTKTYTCNVDHKPSNTKVDKRVESKYGPPCPPCPAPEFLGGPSVFLFPPKPKDQLMISRTPEVTCVVVDVSQEDPEVQFNWYVDGVEVHNAKTKPREEQFNSTYRVVSVLTVLHQDWLNGKEYKCKVSNKGLPSSIEKTISKAKGQPREPQVYTLPPSQEEMTKNQVSLTCLVKGFYPSDIAVEWESNGQPENNYKTTPPVLDSDGSFFLYSRLTVDKSRWQEGNVFSCSVLHEALHNHYTQKSLSLSLG

SEQ ID NO: 89 - protein, 327 aa, synthetic construct
ASTKGPSVFPLAPCSRSTSESTAALGCLVKDYFPEPVTVSWNSGALTSGVHTFPAVLQSSGLYSLSSVVTVPSSSLGTKTYTCNVDHKPSNTKVDKRVESKYGPPCPPCPAPESTRGPSVFLFPPKPKDQLMISRTPEVTCVVVDVSQEDPEVQFNWYVDGVEVHNAKTKPREEQFNSTYRVVSVLTVLHQDWLNGKEYKCKVSNKGLPSSIEKTISKAKGQPREPQVYTLPPSQEEMTKNQVSLTCLVKGFYPSDIAVEWESNGQPENNYKTTPPVLDSDGSFFLYSRLTVDKSRWQEGNVFSCSVLHEALHNHYTQKSLSLSLGK

SEQ ID NO: 90 - protein, 326 aa, synthetic construct
ASTKGPSVFPLAPCSRSTSESTAALGCLVKDYFPEPVTVSWNSGALTSGVHTFPAVLQSSGLYSLSSVVTVPSSSLGTKTYTCNVDHKPSNTKVDKRVESKYGPPCPPCPAPESTRGPSVFLFPPKPKDQLMISRTPEVTCVVVDVSQEDPEVQFNWYVDGVEVHNAKTKPREEQFNSTYRVVSVLTVLHQDWLNGKEYKCKVSNKGLPSSIEKTISKAKGQPREPQVYTLPPSQEEMTKNQVSLTCLVKGFYPSDIAVEWESNGQPENNYKTTPPVLDSDGSFFLYSRLTVDKSRWQEGNVFSCSVLHEALHNHYTQKSLSLSLG

SEQ ID NO: 91 - protein, 327 aa, synthetic construct
ASTKGPSVFPLAPCSRSTSESTAALGCLVKDYFPEPVTVSWNSGALTSGVHTFPAVLQSSGLYSLSSVVTVPSSSLGTKTYTCNVDHKPSNTKVDKRVESKYGPPCPPCPAPEAAGGPSVFLFPPKPKDQLMISRTPEVTCVVVDVSQEDPEVQFNWYVDGVEVHNAKTKPREEQFNSTYRVVSVLTVLHQDWLNGKEYKCKVSNKGLPSSIEKTISKAKGQPREPQVYTLPPSQEEMTKNQVSLTCLVKGFYPSDIAVEWESNGQPENNYKTTPPVLDSDGSFFLYSRLTVDKSRWQEGNVFSCSVLHEALHNHYTQKSLSLSLGK

SEQ ID NO: 92 - protein, 326 aa, synthetic construct
ASTKGPSVFPLAPCSRSTSESTAALGCLVKDYFPEPVTVSWNSGALTSGVHTFPAVLQSSGLYSLSSVVTVPSSSLGTKTYTCNVDHKPSNTKVDKRVESKYGPPCPPCPAPEAAGGPSVFLFPPKPKDQLMISRTPEVTCVVVDVSQEDPEVQFNWYVDGVEVHNAKTKPREEQFNSTYRVVSVLTVLHQDWLNGKEYKCKVSNKGLPSSIEKTISKAKGQPREPQVYTLPPSQEEMTKNQVSLTCLVKGFYPSDIAVEWESNGQPENNYKTTPPVLDSDGSFFLYSRLTVDKSRWQEGNVFSCSVLHEALHNHYTQKSLSLSLG

SEQ ID NO: 93 - protein, 327 aa, synthetic construct
ASTKGPSVFPLAPCSRSTSESTAALGCLVKDYFPEPVTVSWNSGALTSGVHTFPAVLQSSGLYSLSSVVTVPSSSLGTKTYTCNVDHKPSNTKVDKRVESKYGPPCPPCPAPEFLGGPSVFLFPPKPKDTLMISRTPEVTCVVVDVSQEDPEVQFNWYVDGVEVHNAKTKPREEQFNSTYRVVSVLTVDHHDWLNGKEYKCKVSNKGLPSSIEKTISKAKGQPREPQVYTLPPSQEEMTKNQVSLTCLVKGFYPSDIAVEWESNGQPENNYKTTPPVLDSDGSFFLYSRLTVDKSRWQEGNVFSCSVMHEALHSHYTQKSLSLSLGK

SEQ ID NO: 94 - protein, 326 aa, synthetic construct
ASTKGPSVFPLAPCSRSTSESTAALGCLVKDYFPEPVTVSWNSGALTSGVHTFPAVLQSSGLYSLSSVVTVPSSSLGTKTYTCNVDHKPSNTKVDKRVESKYGPPCPPCPAPEFLGGPSVFLFPPKPKDTLMISRTPEVTCVVVDVSQEDPEVQFNWYVDGVEVHNAKTKPREEQFNSTYRVVSVLTVDHHDWLNGKEYKCKVSNKGLPSSIEKTISKAKGQPREPQVYTLPPSQEEMTKNQVSLTCLVKGFYPSDIAVEWESNGQPENNYKTTPPVLDSDGSFFLYSRLTVDKSRWQEGNVFSCSVMHEALHSHYTQKSLSLSLG

SEQ ID NO: 95 - protein, 327 aa, synthetic construct
ASTKGPSVFPLAPCSRSTSESTAALGCLVKDYFPEPVTVSWNSGALTSGVHTFPAVLQSSGLYSLSSVVTVPSSSLGTKTYTCNVDHKPSNTKVDKRVESKYGPPCPPCPAPESTRGPSVFLFPPKPKDTLMISRTPEVTCVVVDVSQEDPEVQFNWYVDGVEVHNAKTKPREEQFNSTYRVVSVLTVDHHDWLNGKEYKCKVSNKGLPSSIEKTISKAKGQPREPQVYTLPPSQEEMTKNQVSLTCLVKGFYPSDIAVEWESNGQPENNYKTTPPVLDSDGSFFLYSRLTVDKSRWQEGNVFSCSVMHEALHSHYTQKSLSLSLGK

SEQ ID NO: 96 - protein, 326 aa, synthetic construct
ASTKGPSVFPLAPCSRSTSESTAALGCLVKDYFPEPVTVSWNSGALTSGVHTFPAVLQSSGLYSLSSVVTVPSSSLGTKTYTCNVDHKPSNTKVDKRVESKYGPPCPPCPAPESTRGPSVFLFPPKPKDTLMISRTPEVTCVVVDVSQEDPEVQFNWYVDGVEVHNAKTKPREEQFNSTYRVVSVLTVDHHDWLNGKEYKCKVSNKGLPSSIEKTISKAKGQPREPQVYTLPPSQEEMTKNQVSLTCLVKGFYPSDIAVEWESNGQPENNYKTTPPVLDSDGSFFLYSRLTVDKSRWQEGNVFSCSVMHEALHSHYTQKSLSLSLG

SEQ ID NO: 97 - protein, 327 aa, synthetic construct
ASTKGPSVFPLAPCSRSTSESTAALGCLVKDYFPEPVTVSWNSGALTSGVHTFPAVLQSSGLYSLSSVVTVPSSSLGTKTYTCNVDHKPSNTKVDKRVESKYGPPCPPCPAPEAAGGPSVFLFPPKPKDTLMISRTPEVTCVVVDVSQEDPEVQFNWYVDGVEVHNAKTKPREEQFNSTYRVVSVLTVDHHDWLNGKEYKCKVSNKGLPSSIEKTISKAKGQPREPQVYTLPPSQEEMTKNQVSLTCLVKGFYPSDIAVEWESNGQPENNYKTTPPVLDSDGSFFLYSRLTVDKSRWQEGNVFSCSVMHEALHSHYTQKSLSLSLGK

SEQ ID NO: 98 - protein, 326 aa, synthetic construct
ASTKGPSVFPLAPCSRSTSESTAALGCLVKDYFPEPVTVSWNSGALTSGVHTFPAVLQSSGLYSLSSVVTVPSSSLGTKTYTCNVDHKPSNTKVDKRVESKYGPPCPPCPAPEAAGGPSVFLFPPKPKDTLMISRTPEVTCVVVDVSQEDPEVQFNWYVDGVEVHNAKTKPREEQFNSTYRVVSVLTVDHHDWLNGKEYKCKVSNKGLPSSIEKTISKAKGQPREPQVYTLPPSQEEMTKNQVSLTCLVKGFYPSDIAVEWESNGQPENNYKTTPPVLDSDGSFFLYSRLTVDKSRWQEGNVFSCSVMHEALHSHYTQKSLSLSLG

SEQ ID NO: 99 - protein, 327 aa, synthetic construct
ASTKGPSVFPLAPCSRSTSESTAALGCLVKDYFPEPVTVSWNSGALTSGVHTFPAVLQSSGLYSLSSVVTVPSSSLGTKTYTCNVDHKPSNTKVDKRVESKYGPPCPSCPAPEFLGGPSVFLFPPKPKDTLMISRTPEVTCVVVDVSQEDPEVQFNWYVDGVEVHNAKTKPREEQFNSTYRVVSVLTVLHQDWLNGKEYKCKVSNKGLPSSIEKTISKAKGQPREPQVYTLPPSQEEMTKNQVSLTCLVKGFYPSDIAVEWESNGQPENNYKTTPPVLDSDGSFFLYSRLTVDKSRWQEGNVFSCSVMHEALHNHYTQKSLSLSLGK

SEQ ID NO: 100 - protein, 326 aa, synthetic construct
ASTKGPSVFPLAPCSRSTSESTAALGCLVKDYFPEPVTVSWNSGALTSGVHTFPAVLQSSGLYSLSSVVTVPSSSLGTKTYTCNVDHKPSNTKVDKRVESKYGPPCPSCPAPEFLGGPSVFLFPPKPKDTLMISRTPEVTCVVVDVSQEDPEVQFNWYVDGVEVHNAKTKPREEQFNSTYRVVSVLTVLHQDWLNGKEYKCKVSNKGLPSSIEKTISKAKGQPREPQVYTLPPSQEEMTKNQVSLTCLVKGFYPSDIAVEWESNGQPENNYKTTPPVLDSDGSFFLYSRLTVDKSRWQEGNVFSCSVMHEALHNHYTQKSLSLSLG

SEQ ID NO: 101 - protein, 327 aa, synthetic construct
ASTKGPSVFPLAPCSRSTSESTAALGCLVKDYFPEPVTVSWNSGALTSGVHTFPAVLQSSGLYSLSSVVTVPSSSLGTKTYTCNVDHKPSNTKVDKRVESKYGPPCPSCPAPESTRGPSVFLFPPKPKDTLMISRTPEVTCVVVDVSQEDPEVQFNWYVDGVEVHNAKTKPREEQFNSTYRVVSVLTVLHQDWLNGKEYKCKVSNKGLPSSIEKTISKAKGQPREPQVYTLPPSQEEMTKNQVSLTCLVKGFYPSDIAVEWESNGQPENNYKTTPPVLDSDGSFFLYSRLTVDKSRWQEGNVFSCSVMHEALHNHYTQKSLSLSLGK

SEQ ID NO: 102 - protein, 326 aa, synthetic construct
ASTKGPSVFPLAPCSRSTSESTAALGCLVKDYFPEPVTVSWNSGALTSGVHTFPAVLQSSGLYSLSSVVTVPSSSLGTKTYTCNVDHKPSNTKVDKRVESKYGPPCPSCPAPESTRGPSVFLFPPKPKDTLMISRTPEVTCVVVDVSQEDPEVQFNWYVDGVEVHNAKTKPREEQFNSTYRVVSVLTVLHQDWLNGKEYKCKVSNKGLPSSIEKTISKAKGQPREPQVYTLPPSQEEMTKNQVSLTCLVKGFYPSDIAVEWESNGQPENNYKTTPPVLDSDGSFFLYSRLTVDKSRWQEGNVFSCSVMHEALHNHYTQKSLSLSLG

SEQ ID NO: 103 - protein, 327 aa, synthetic construct
ASTKGPSVFPLAPCSRSTSESTAALGCLVKDYFPEPVTVSWNSGALTSGVHTFPAVLQSSGLYSLSSVVTVPSSSLGTKTYTCNVDHKPSNTKVDKRVESKYGPPCPSCPAPEAAGGPSVFLFPPKPKDTLMISRTPEVTCVVVDVSQEDPEVQFNWYVDGVEVHNAKTKPREEQFNSTYRVVSVLTVLHQDWLNGKEYKCKVSNKGLPSSIEKTISKAKGQPREPQVYTLPPSQEEMTKNQVSLTCLVKGFYPSDIAVEWESNGQPENNYKTTPPVLDSDGSFFLYSRLTVDKSRWQEGNVFSCSVMHEALHNHYTQKSLSLSLGK

SEQ ID NO: 104 - protein, 326 aa, synthetic construct
ASTKGPSVFPLAPCSRSTSESTAALGCLVKDYFPEPVTVSWNSGALTSGVHTFPAVLQSSGLYSLSSVVTVPSSSLGTKTYTCNVDHKPSNTKVDKRVESKYGPPCPSCPAPEAAGGPSVFLFPPKPKDTLMISRTPEVTCVVVDVSQEDPEVQFNWYVDGVEVHNAKTKPREEQFNSTYRVVSVLTVLHQDWLNGKEYKCKVSNKGLPSSIEKTISKAKGQPREPQVYTLPPSQEEMTKNQVSLTCLVKGFYPSDIAVEWESNGQPENNYKTTPPVLDSDGSFFLYSRLTVDKSRWQEGNVFSCSVMHEALHNHYTQKSLSLSLG

SEQ ID NO: 105 - protein, 327 aa, synthetic construct
ASTKGPSVFPLAPCSRSTSESTAALGCLVKDYFPEPVTVSWNSGALTSGVHTFPAVLQSSGLYSLSSVVTVPSSSLGTKTYTCNVDHKPSNTKVDKRVESKYGPPCPSCPAPEFLGGPSVFLFPPKPKDTLYITREPEVTCVVVDVSQEDPEVQFNWYVDGVEVHNAKTKPREEQFNSTYRVVSVLTVLHQDWLNGKEYKCKVSNKGLPSSIEKTISKAKGQPREPQVYTLPPSQEEMTKNQVSLTCLVKGFYPSDIAVEWESNGQPENNYKTTPPVLDSDGSFFLYSRLTVDKSRWQEGNVFSCSVMHEALHNHYTQKSLSLSLGK

SEQ ID NO: 106 - protein, 326 aa, synthetic construct
ASTKGPSVFPLAPCSRSTSESTAALGCLVKDYFPEPVTVSWNSGALTSGVHTFPAVLQSSGLYSLSSVVTVPSSSLGTKTYTCNVDHKPSNTKVDKRVESKYGPPCPSCPAPEFLGGPSVFLFPPKPKDTLYITREPEVTCVVVDVSQEDPEVQFNWYVDGVEVHNAKTKPREEQFNSTYRVVSVLTVLHQDWLNGKEYKCKVSNKGLPSSIEKTISKAKGQPREPQVYTLPPSQEEMTKNQVSLTCLVKGFYPSDIAVEWESNGQPENNYKTTPPVLDSDGSFFLYSRLTVDKSRWQEGNVFSCSVMHEALHNHYTQKSLSLSLG

SEQ ID NO: 107 - protein, 327 aa, synthetic construct
ASTKGPSVFPLAPCSRSTSESTAALGCLVKDYFPEPVTVSWNSGALTSGVHTFPAVLQSSGLYSLSSVVTVPSSSLGTKTYTCNVDHKPSNTKVDKRVESKYGPPCPSCPAPESTRGPSVFLFPPKPKDTLYITREPEVTCVVVDVSQEDPEVQFNWYVDGVEVHNAKTKPREEQFNSTYRVVSVLTVLHQDWLNGKEYKCKVSNKGLPSSIEKTISKAKGQPREPQVYTLPPSQEEMTKNQVSLTCLVKGFYPSDIAVEWESNGQPENNYKTTPPVLDSDGSFFLYSRLTVDKSRWQEGNVFSCSVMHEALHNHYTQKSLSLSLGK

SEQ ID NO: 108 - protein, 326 aa, synthetic construct
ASTKGPSVFPLAPCSRSTSESTAALGCLVKDYFPEPVTVSWNSGALTSGVHTFPAVLQSSGLYSLSSVVTVPSSSLGTKTYTCNVDHKPSNTKVDKRVESKYGPPCPSCPAPESTRGPSVFLFPPKPKDTLYITREPEVTCVVVDVSQEDPEVQFNWYVDGVEVHNAKTKPREEQFNSTYRVVSVLTVLHQDWLNGKEYKCKVSNKGLPSSIEKTISKAKGQPREPQVYTLPPSQEEMTKNQVSLTCLVKGFYPSDIAVEWESNGQPENNYKTTPPVLDSDGSFFLYSRLTVDKSRWQEGNVFSCSVMHEALHNHYTQKSLSLSLG

SEQ ID NO: 109 - protein, 327 aa, synthetic construct
ASTKGPSVFPLAPCSRSTSESTAALGCLVKDYFPEPVTVSWNSGALTSGVHTFPAVLQSSGLYSLSSVVTVPSSSLGTKTYTCNVDHKPSNTKVDKRVESKYGPPCPSCPAPEAAGGPSVFLFPPKPKDTLYITREPEVTCVVVDVSQEDPEVQFNWYVDGVEVHNAKTKPREEQFNSTYRVVSVLTVLHQDWLNGKEYKCKVSNKGLPSSIEKTISKAKGQPREPQVYTLPPSQEEMTKNQVSLTCLVKGFYPSDIAVEWESNGQPENNYKTTPPVLDSDGSFFLYSRLTVDKSRWQEGNVFSCSVMHEALHNHYTQKSLSLSLGK

SEQ ID NO: 110 - protein, 326 aa, synthetic construct
ASTKGPSVFPLAPCSRSTSESTAALGCLVKDYFPEPVTVSWNSGALTSGVHTFPAVLQSSGLYSLSSVVTVPSSSLGTKTYTCNVDHKPSNTKVDKRVESKYGPPCPSCPAPEAAGGPSVFLFPPKPKDTLYITREPEVTCVVVDVSQEDPEVQFNWYVDGVEVHNAKTKPREEQFNSTYRVVSVLTVLHQDWLNGKEYKCKVSNKGLPSSIEKTISKAKGQPREPQVYTLPPSQEEMTKNQVSLTCLVKGFYPSDIAVEWESNGQPENNYKTTPPVLDSDGSFFLYSRLTVDKSRWQEGNVFSCSVMHEALHNHYTQKSLSLSLG

SEQ ID NO: 111 - protein, 327 aa, synthetic construct
ASTKGPSVFPLAPCSRSTSESTAALGCLVKDYFPEPVTVSWNSGALTSGVHTFPAVLQSSGLYSLSSVVTVPSSSLGTKTYTCNVDHKPSNTKVDKRVESKYGPPCPSCPAPEFLGGPSVFLFPPKPKDTLMISRTPEVTCVVVDVSQEDPEVQFNWYVDGVEVHNAKTKPREEQFNSTYRVVSVLTVLHRDWLNGKEYKCKVSNKGLPSSIEKTISKAKGQPREPQVYTLPPSQEEMTKNQVSLTCLVKGFYPSDIAVEWESNGQPENNYKTTPPVLDSDGSFFLYSRLTVDKSRWQEGNVFSCSVEHEALHWHYTQKSLSLSLGK

SEQ ID NO: 112 - protein, 326 aa, synthetic construct
ASTKGPSVFPLAPCSRSTSESTAALGCLVKDYFPEPVTVSWNSGALTSGVHTFPAVLQSSGLYSLSSVVTVPSSSLGTKTYTCNVDHKPSNTKVDKRVESKYGPPCPSCPAPEFLGGPSVFLFPPKPKDTLMISRTPEVTCVVVDVSQEDPEVQFNWYVDGVEVHNAKTKPREEQFNSTYRVVSVLTVLHRDWLNGKEYKCKVSNKGLPSSIEKTISKAKGQPREPQVYTLPPSQEEMTKNQVSLTCLVKGFYPSDIAVEWESNGQPENNYKTTPPVLDSDGSFFLYSRLTVDKSRWQEGNVFSCSVEHEALHWHYTQKSLSLSLG

SEQ ID NO: 113 - protein, 327 aa, synthetic construct
ASTKGPSVFPLAPCSRSTSESTAALGCLVKDYFPEPVTVSWNSGALTSGVHTFPAVLQSSGLYSLSSVVTVPSSSLGTKTYTCNVDHKPSNTKVDKRVESKYGPPCPSCPAPESTRGPSVFLFPPKPKDTLMISRTPEVTCVVVDVSQEDPEVQFNWYVDGVEVHNAKTKPREEQFNSTYRVVSVLTVLHRDWLNGKEYKCKVSNKGLPSSIEKTISKAKGQPREPQVYTLPPSQEEMTKNQVSLTCLVKGFYPSDIAVEWESNGQPENNYKTTPPVLDSDGSFFLYSRLTVDKSRWQEGNVFSCSVEHEALHWHYTQKSLSLSLGK

SEQ ID NO: 114 - protein, 326 aa, synthetic construct
ASTKGPSVFPLAPCSRSTSESTAALGCLVKDYFPEPVTVSWNSGALTSGVHTFPAVLQSSGLYSLSSVVTVPSSSLGTKTYTCNVDHKPSNTKVDKRVESKYGPPCPSCPAPESTRGPSVFLFPPKPKDTLMISRTPEVTCVVVDVSQEDPEVQFNWYVDGVEVHNAKTKPREEQFNSTYRVVSVLTVLHRDWLNGKEYKCKVSNKGLPSSIEKTISKAKGQPREPQVYTLPPSQEEMTKNQVSLTCLVKGFYPSDIAVEWESNGQPENNYKTTPPVLDSDGSFFLYSRLTVDKSRWQEGNVFSCSVEHEALHWHYTQKSLSLSLG

SEQ ID NO: 115 - protein, 327 aa, synthetic construct
ASTKGPSVFPLAPCSRSTSESTAALGCLVKDYFPEPVTVSWNSGALTSGVHTFPAVLQSSGLYSLSSVVTVPSSSLGTKTYTCNVDHKPSNTKVDKRVESKYGPPCPSCPAPEAAGGPSVFLFPPKPKDTLMISRTPEVTCVVVDVSQEDPEVQFNWYVDGVEVHNAKTKPREEQFNSTYRVVSVLTVLHRDWLNGKEYKCKVSNKGLPSSIEKTISKAKGQPREPQVYTLPPSQEEMTKNQVSLTCLVKGFYPSDIAVEWESNGQPENNYKTTPPVLDSDGSFFLYSRLTVDKSRWQEGNVFSCSVEHEALHWHYTQKSLSLSLGK

SEQ ID NO: 116 - protein, 326 aa, synthetic construct
ASTKGPSVFPLAPCSRSTSESTAALGCLVKDYFPEPVTVSWNSGALTSGVHTFPAVLQSSGLYSLSSVVTVPSSSLGTKTYTCNVDHKPSNTKVDKRVESKYGPPCPSCPAPEAAGGPSVFLFPPKPKDTLMISRTPEVTCVVVDVSQEDPEVQFNWYVDGVEVHNAKTKPREEQFNSTYRVVSVLTVLHRDWLNGKEYKCKVSNKGLPSSIEKTISKAKGQPREPQVYTLPPSQEEMTKNQVSLTCLVKGFYPSDIAVEWESNGQPENNYKTTPPVLDSDGSFFLYSRLTVDKSRWQEGNVFSCSVEHEALHWHYTQKSLSLSLG

SEQ ID NO: 117 - protein, 327 aa, synthetic construct
ASTKGPSVFPLAPCSRSTSESTAALGCLVKDYFPEPVTVSWNSGALTSGVHTFPAVLQSSGLYSLSSVVTVPSSSLGTKTYTCNVDHKPSNTKVDKRVESKYGPPCPSCPAPEFLGGPSVFLFPPKPKDTLMISRTPEVTCVVVDVSQEDPEVQFNWYVDGVEVHNAKTKPREEQFNSTYRVVSVLTVLHQDWLNGKEYKCKVSNKGLPSSIEKTISKAKGQPREPQVYTLPPSQEEMTKNQVSLTCLVKGFYPSDIAVEWESNGQPENNYKTTPPVLDSDGSFFLYSRLTVDKSRWQEGNVFSCSVLHEALHSHYTQKSLSLSLGK

SEQ ID NO: 118 - protein, 326 aa, synthetic construct
ASTKGPSVFPLAPCSRSTSESTAALGCLVKDYFPEPVTVSWNSGALTSGVHTFPAVLQSSGLYSLSSVVTVPSSSLGTKTYTCNVDHKPSNTKVDKRVESKYGPPCPSCPAPEFLGGPSVFLFPPKPKDTLMISRTPEVTCVVVDVSQEDPEVQFNWYVDGVEVHNAKTKPREEQFNSTYRVVSVLTVLHQDWLNGKEYKCKVSNKGLPSSIEKTISKAKGQPREPQVYTLPPSQEEMTKNQVSLTCLVKGFYPSDIAVEWESNGQPENNYKTTPPVLDSDGSFFLYSRLTVDKSRWQEGNVFSCSVLHEALHSHYTQKSLSLSLG

SEQ ID NO: 119 - protein, 327 aa, synthetic construct
ASTKGPSVFPLAPCSRSTSESTAALGCLVKDYFPEPVTVSWNSGALTSGVHTFPAVLQSSGLYSLSSVVTVPSSSLGTKTYTCNVDHKPSNTKVDKRVESKYGPPCPSCPAPESTRGPSVFLFPPKPKDTLMISRTPEVTCVVVDVSQEDPEVQFNWYVDGVEVHNAKTKPREEQFNSTYRVVSVLTVLHQDWLNGKEYKCKVSNKGLPSSIEKTISKAKGQPREPQVYTLPPSQEEMTKNQVSLTCLVKGFYPSDIAVEWESNGQPENNYKTTPPVLDSDGSFFLYSRLTVDKSRWQEGNVFSCSVLHEALHSHYTQKSLSLSLGK

SEQ ID NO: 120 - protein, 326 aa, synthetic construct
ASTKGPSVFPLAPCSRSTSESTAALGCLVKDYFPEPVTVSWNSGALTSGVHTFPAVLQSSGLYSLSSVVTVPSSSLGTKTYTCNVDHKPSNTKVDKRVESKYGPPCPSCPAPESTRGPSVFLFPPKPKDTLMISRTPEVTCVVVDVSQEDPEVQFNWYVDGVEVHNAKTKPREEQFNSTYRVVSVLTVLHQDWLNGKEYKCKVSNKGLPSSIEKTISKAKGQPREPQVYTLPPSQEEMTKNQVSLTCLVKGFYPSDIAVEWESNGQPENNYKTTPPVLDSDGSFFLYSRLTVDKSRWQEGNVFSCSVLHEALHSHYTQKSLSLSLG

SEQ ID NO: 121 - protein, 327 aa, synthetic construct
ASTKGPSVFPLAPCSRSTSESTAALGCLVKDYFPEPVTVSWNSGALTSGVHTFPAVLQSSGLYSLSSVVTVPSSSLGTKTYTCNVDHKPSNTKVDKRVESKYGPPCPSCPAPEAAGGPSVFLFPPKPKDTLMISRTPEVTCVVVDVSQEDPEVQFNWYVDGVEVHNAKTKPREEQFNSTYRVVSVLTVLHQDWLNGKEYKCKVSNKGLPSSIEKTISKAKGQPREPQVYTLPPSQEEMTKNQVSLTCLVKGFYPSDIAVEWESNGQPENNYKTTPPVLDSDGSFFLYSRLTVDKSRWQEGNVFSCSVLHEALHSHYTQKSLSLSLGK

SEQ ID NO: 122 - protein, 326 aa, synthetic construct
ASTKGPSVFPLAPCSRSTSESTAALGCLVKDYFPEPVTVSWNSGALTSGVHTFPAVLQSSGLYSLSSVVTVPSSSLGTKTYTCNVDHKPSNTKVDKRVESKYGPPCPSCPAPEAAGGPSVFLFPPKPKDTLMISRTPEVTCVVVDVSQEDPEVQFNWYVDGVEVHNAKTKPREEQFNSTYRVVSVLTVLHQDWLNGKEYKCKVSNKGLPSSIEKTISKAKGQPREPQVYTLPPSQEEMTKNQVSLTCLVKGFYPSDIAVEWESNGQPENNYKTTPPVLDSDGSFFLYSRLTVDKSRWQEGNVFSCSVLHEALHSHYTQKSLSLSLG

SEQ ID NO: 123 - protein, 327 aa, synthetic construct
ASTKGPSVFPLAPCSRSTSESTAALGCLVKDYFPEPVTVSWNSGALTSGVHTFPAVLQSSGLYSLSSVVTVPSSSLGTKTYTCNVDHKPSNTKVDKRVESKYGPPCPSCPAPEFLGGPSVFLFPPKPKDQLMISRTPEVTCVVVDVSQEDPEVQFNWYVDGVEVHNAKTKPREEQFNSTYRVVSVLTVLHQDWLNGKEYKCKVSNKGLPSSIEKTISKAKGQPREPQVYTLPPSQEEMTKNQVSLTCLVKGFYPSDIAVEWESNGQPENNYKTTPPVLDSDGSFFLYSRLTVDKSRWQEGNVFSCSVLHEALHNHYTQKSLSLSLGK

SEQ ID NO: 124 - protein, 326 aa, synthetic construct
ASTKGPSVFPLAPCSRSTSESTAALGCLVKDYFPEPVTVSWNSGALTSGVHTFPAVLQSSGLYSLSSVVTVPSSSLGTKTYTCNVDHKPSNTKVDKRVESKYGPPCPSCPAPEFLGGPSVFLFPPKPKDQLMISRTPEVTCVVVDVSQEDPEVQFNWYVDGVEVHNAKTKPREEQFNSTYRVVSVLTVLHQDWLNGKEYKCKVSNKGLPSSIEKTISKAKGQPREPQVYTLPPSQEEMTKNQVSLTCLVKGFYPSDIAVEWESNGQPENNYKTTPPVLDSDGSFFLYSRLTVDKSRWQEGNVFSCSVLHEALHNHYTQKSLSLSLG

SEQ ID NO: 125 - protein, 327 aa, synthetic construct
ASTKGPSVFPLAPCSRSTSESTAALGCLVKDYFPEPVTVSWNSGALTSGVHTFPAVLQSSGLYSLSSVVTVPSSSLGTKTYTCNVDHKPSNTKVDKRVESKYGPPCPSCPAPESTRGPSVFLFPPKPKDQLMISRTPEVTCVVVDVSQEDPEVQFNWYVDGVEVHNAKTKPREEQFNSTYRVVSVLTVLHQDWLNGKEYKCKVSNKGLPSSIEKTISKAKGQPREPQVYTLPPSQEEMTKNQVSLTCLVKGFYPSDIAVEWESNGQPENNYKTTPPVLDSDGSFFLYSRLTVDKSRWQEGNVFSCSVLHEALHNHYTQKSLSLSLGK

SEQ ID NO: 126 - protein, 326 aa, synthetic construct
ASTKGPSVFPLAPCSRSTSESTAALGCLVKDYFPEPVTVSWNSGALTSGVHTFPAVLQSSGLYSLSSVVTVPSSSLGTKTYTCNVDHKPSNTKVDKRVESKYGPPCPSCPAPESTRGPSVFLFPPKPKDQLMISRTPEVTCVVVDVSQEDPEVQFNWYVDGVEVHNAKTKPREEQFNSTYRVVSVLTVLHQDWLNGKEYKCKVSNKGLPSSIEKTISKAKGQPREPQVYTLPPSQEEMTKNQVSLTCLVKGFYPSDIAVEWESNGQPENNYKTTPPVLDSDGSFFLYSRLTVDKSRWQEGNVFSCSVLHEALHNHYTQKSLSLSLG

SEQ ID NO: 127 - protein, 327 aa, synthetic construct
ASTKGPSVFPLAPCSRSTSESTAALGCLVKDYFPEPVTVSWNSGALTSGVHTFPAVLQSSGLYSLSSVVTVPSSSLGTKTYTCNVDHKPSNTKVDKRVESKYGPPCPSCPAPEAAGGPSVFLFPPKPKDQLMISRTPEVTCVVVDVSQEDPEVQFNWYVDGVEVHNAKTKPREEQFNSTYRVVSVLTVLHQDWLNGKEYKCKVSNKGLPSSIEKTISKAKGQPREPQVYTLPPSQEEMTKNQVSLTCLVKGFYPSDIAVEWESNGQPENNYKTTPPVLDSDGSFFLYSRLTVDKSRWQEGNVFSCSVLHEALHNHYTQKSLSLSLGK

SEQ ID NO: 128 - protein, 326 aa, synthetic construct
ASTKGPSVFPLAPCSRSTSESTAALGCLVKDYFPEPVTVSWNSGALTSGVHTFPAVLQSSGLYSLSSVVTVPSSSLGTKTYTCNVDHKPSNTKVDKRVESKYGPPCPSCPAPEAAGGPSVFLFPPKPKDQLMISRTPEVTCVVVDVSQEDPEVQFNWYVDGVEVHNAKTKPREEQFNSTYRVVSVLTVLHQDWLNGKEYKCKVSNKGLPSSIEKTISKAKGQPREPQVYTLPPSQEEMTKNQVSLTCLVKGFYPSDIAVEWESNGQPENNYKTTPPVLDSDGSFFLYSRLTVDKSRWQEGNVFSCSVLHEALHNHYTQKSLSLSLG

SEQ ID NO: 129 - protein, 327 aa, synthetic construct
ASTKGPSVFPLAPCSRSTSESTAALGCLVKDYFPEPVTVSWNSGALTSGVHTFPAVLQSSGLYSLSSVVTVPSSSLGTKTYTCNVDHKPSNTKVDKRVESKYGPPCPSCPAPEFLGGPSVFLFPPKPKDTLMISRTPEVTCVVVDVSQEDPEVQFNWYVDGVEVHNAKTKPREEQFNSTYRVVSVLTVDHHDWLNGKEYKCKVSNKGLPSSIEKTISKAKGQPREPQVYTLPPSQEEMTKNQVSLTCLVKGFYPSDIAVEWESNGQPENNYKTTPPVLDSDGSFFLYSRLTVDKSRWQEGNVFSCSVMHEALHSHYTQKSLSLSLGK

SEQ ID NO: 130 - protein, 326 aa, synthetic construct
ASTKGPSVFPLAPCSRSTSESTAALGCLVKDYFPEPVTVSWNSGALTSGVHTFPAVLQSSGLYSLSSVVTVPSSSLGTKTYTCNVDHKPSNTKVDKRVESKYGPPCPSCPAPEFLGGPSVFLFPPKPKDTLMISRTPEVTCVVVDVSQEDPEVQFNWYVDGVEVHNAKTKPREEQFNSTYRVVSVLTVDHHDWLNGKEYKCKVSNKGLPSSIEKTISKAKGQPREPQVYTLPPSQEEMTKNQVSLTCLVKGFYPSDIAVEWESNGQPENNYKTTPPVLDSDGSFFLYSRLTVDKSRWQEGNVFSCSVMHEALHSHYTQKSLSLSLG

SEQ ID NO: 131 - protein, 327 aa, synthetic construct
ASTKGPSVFPLAPCSRSTSESTAALGCLVKDYFPEPVTVSWNSGALTSGVHTFPAVLQSSGLYSLSSVVTVPSSSLGTKTYTCNVDHKPSNTKVDKRVESKYGPPCPSCPAPESTRGPSVFLFPPKPKDTLMISRTPEVTCVVVDVSQEDPEVQFNWYVDGVEVHNAKTKPREEQFNSTYRVVSVLTVDHHDWLNGKEYKCKVSNKGLPSSIEKTISKAKGQPREPQVYTLPPSQEEMTKNQVSLTCLVKGFYPSDIAVEWESNGQPENNYKTTPPVLDSDGSFFLYSRLTVDKSRWQEGNVFSCSVMHEALHSHYTQKSLSLSLGK

SEQ ID NO: 132 - protein, 326 aa, synthetic construct
ASTKGPSVFPLAPCSRSTSESTAALGCLVKDYFPEPVTVSWNSGALTSGVHTFPAVLQSSGLYSLSSVVTVPSSSLGTKTYTCNVDHKPSNTKVDKRVESKYGPPCPSCPAPESTRGPSVFLFPPKPKDTLMISRTPEVTCVVVDVSQEDPEVQFNWYVDGVEVHNAKTKPREEQFNSTYRVVSVLTVDHHDWLNGKEYKCKVSNKGLPSSIEKTISKAKGQPREPQVYTLPPSQEEMTKNQVSLTCLVKGFYPSDIAVEWESNGQPENNYKTTPPVLDSDGSFFLYSRLTVDKSRWQEGNVFSCSVMHEALHSHYTQKSLSLSLG

SEQ ID NO: 133 - protein, 327 aa, synthetic construct
ASTKGPSVFPLAPCSRSTSESTAALGCLVKDYFPEPVTVSWNSGALTSGVHTFPAVLQSSGLYSLSSVVTVPSSSLGTKTYTCNVDHKPSNTKVDKRVESKYGPPCPSCPAPEAAGGPSVFLFPPKPKDTLMISRTPEVTCVVVDVSQEDPEVQFNWYVDGVEVHNAKTKPREEQFNSTYRVVSVLTVDHHDWLNGKEYKCKVSNKGLPSSIEKTISKAKGQPREPQVYTLPPSQEEMTKNQVSLTCLVKGFYPSDIAVEWESNGQPENNYKTTPPVLDSDGSFFLYSRLTVDKSRWQEGNVFSCSVMHEALHSHYTQKSLSLSLGK

SEQ ID NO: 134 - protein, 326 aa, synthetic construct
ASTKGPSVFPLAPCSRSTSESTAALGCLVKDYFPEPVTVSWNSGALTSGVHTFPAVLQSSGLYSLSSVVTVPSSSLGTKTYTCNVDHKPSNTKVDKRVESKYGPPCPSCPAPEAAGGPSVFLFPPKPKDTLMISRTPEVTCVVVDVSQEDPEVQFNWYVDGVEVHNAKTKPREEQFNSTYRVVSVLTVDHHDWLNGKEYKCKVSNKGLPSSIEKTISKAKGQPREPQVYTLPPSQEEMTKNQVSLTCLVKGFYPSDIAVEWESNGQPENNYKTTPPVLDSDGSFFLYSRLTVDKSRWQEGNVFSCSVMHEALHSHYTQKSLSLSLG

SEQ ID NO: 135 - protein, 227 aa, synthetic construct
DKTHTCPPCPAPELLGGPSVFLFPPKPKDTLMISRTPEVTCVVVDVSHEDPEVKFNWYVDGVEVHNAKTKPREEQYNSTYRVVSVLTVLHQDWLNGKEYKCKVSNKALPAPIEKTISKAKGQPREPQVYTLPPSREEMTKNQVSLWCLVKGFYPSDIAVEWESNGQPENNYKTTPPVLDSDGSFFLYSKLTVDKSRWQQGNVFSCSVMHEALHNHYTQKSLSLSPGK

SEQ ID NO: 136 - protein, 226 aa, synthetic construct
DKTHTCPPCPAPELLGGPSVFLFPPKPKDTLMISRTPEVTCVVVDVSHEDPEVKFNWYVDGVEVHNAKTKPREEQYNSTYRVVSVLTVLHQDWLNGKEYKCKVSNKALPAPIEKTISKAKGQPREPQVYTLPPSREEMTKNQVSLWCLVKGFYPSDIAVEWESNGQPENNYKTTPPVLDSDGSFFLYSKLTVDKSRWQQGNVFSCSVMHEALHNHYTQKSLSLSPG

SEQ ID NO: 137 - protein, 227 aa, synthetic construct
DKTHTCPPCPAPESTRGPSVFLFPPKPKDTLMISRTPEVTCVVVDVSHEDPEVKFNWYVDGVEVHNAKTKPREEQYNSTYRVVSVLTVLHQDWLNGKEYKCKVSNKALPAPIEKTISKAKGQPREPQVYTLPPSREEMTKNQVSLWCLVKGFYPSDIAVEWESNGQPENNYKTTPPVLDSDGSFFLYSKLTVDKSRWQQGNVFSCSVMHEALHNHYTQKSLSLSPGK

SEQ ID NO: 138 - protein, 226 aa, synthetic construct
DKTHTCPPCPAPESTRGPSVFLFPPKPKDTLMISRTPEVTCVVVDVSHEDPEVKFNWYVDGVEVHNAKTKPREEQYNSTYRVVSVLTVLHQDWLNGKEYKCKVSNKALPAPIEKTISKAKGQPREPQVYTLPPSREEMTKNQVSLWCLVKGFYPSDIAVEWESNGQPENNYKTTPPVLDSDGSFFLYSKLTVDKSRWQQGNVFSCSVMHEALHNHYTQKSLSLSPG

SEQ ID NO: 139 - protein, 227 aa, synthetic construct
DKTHTCPPCPAPEAAGGPSVFLFPPKPKDTLMISRTPEVTCVVVDVSHEDPEVKFNWYVDGVEVHNAKTKPREEQYNSTYRVVSVLTVLHQDWLNGKEYKCKVSNKALPAPIEKTISKAKGQPREPQVYTLPPSREEMTKNQVSLWCLVKGFYPSDIAVEWESNGQPENNYKTTPPVLDSDGSFFLYSKLTVDKSRWQQGNVFSCSVMHEALHNHYTQKSLSLSPGK

SEQ ID NO: 140 - protein, 226 aa, synthetic construct
DKTHTCPPCPAPEAAGGPSVFLFPPKPKDTLMISRTPEVTCVVVDVSHEDPEVKFNWYVDGVEVHNAKTKPREEQYNSTYRVVSVLTVLHQDWLNGKEYKCKVSNKALPAPIEKTISKAKGQPREPQVYTLPPSREEMTKNQVSLWCLVKGFYPSDIAVEWESNGQPENNYKTTPPVLDSDGSFFLYSKLTVDKSRWQQGNVFSCSVMHEALHNHYTQKSLSLSPG

SEQ ID NO: 141 - protein, 227 aa, synthetic construct
DKTHTCPPCPAPELLGGPSVFLFPPKPKDTLYITREPEVTCVVVDVSHEDPEVKFNWYVDGVEVHNAKTKPREEQYNSTYRVVSVLTVLHQDWLNGKEYKCKVSNKALPAPIEKTISKAKGQPREPQVYTLPPSREEMTKNQVSLWCLVKGFYPSDIAVEWESNGQPENNYKTTPPVLDSDGSFFLYSKLTVDKSRWQQGNVFSCSVMHEALHNHYTQKSLSLSPGK

SEQ ID NO: 142 - protein, 226 aa, synthetic construct
DKTHTCPPCPAPELLGGPSVFLFPPKPKDTLYITREPEVTCVVVDVSHEDPEVKFNWYVDGVEVHNAKTKPREEQYNSTYRVVSVLTVLHQDWLNGKEYKCKVSNKALPAPIEKTISKAKGQPREPQVYTLPPSREEMTKNQVSLWCLVKGFYPSDIAVEWESNGQPENNYKTTPPVLDSDGSFFLYSKLTVDKSRWQQGNVFSCSVMHEALHNHYTQKSLSLSPG

SEQ ID NO: 143 - protein, 227 aa, synthetic construct
DKTHTCPPCPAPESTRGPSVFLFPPKPKDTLYITREPEVTCVVVDVSHEDPEVKFNWYVDGVEVHNAKTKPREEQYNSTYRVVSVLTVLHQDWLNGKEYKCKVSNKALPAPIEKTISKAKGQPREPQVYTLPPSREEMTKNQVSLWCLVKGFYPSDIAVEWESNGQPENNYKTTPPVLDSDGSFFLYSKLTVDKSRWQQGNVFSCSVMHEALHNHYTQKSLSLSPGK

SEQ ID NO: 144 - protein, 226 aa, synthetic construct
DKTHTCPPCPAPESTRGPSVFLFPPKPKDTLYITREPEVTCVVVDVSHEDPEVKFNWYVDGVEVHNAKTKPREEQYNSTYRVVSVLTVLHQDWLNGKEYKCKVSNKALPAPIEKTISKAKGQPREPQVYTLPPSREEMTKNQVSLWCLVKGFYPSDIAVEWESNGQPENNYKTTPPVLDSDGSFFLYSKLTVDKSRWQQGNVFSCSVMHEALHNHYTQKSLSLSPG

SEQ ID NO: 145 - protein, 227 aa, synthetic construct
DKTHTCPPCPAPEAAGGPSVFLFPPKPKDTLYITREPEVTCVVVDVSHEDPEVKFNWYVDGVEVHNAKTKPREEQYNSTYRVVSVLTVLHQDWLNGKEYKCKVSNKALPAPIEKTISKAKGQPREPQVYTLPPSREEMTKNQVSLWCLVKGFYPSDIAVEWESNGQPENNYKTTPPVLDSDGSFFLYSKLTVDKSRWQQGNVFSCSVMHEALHNHYTQKSLSLSPGK

SEQ ID NO: 146 - protein, 226 aa, synthetic construct
DKTHTCPPCPAPEAAGGPSVFLFPPKPKDTLYITREPEVTCVVVDVSHEDPEVKFNWYVDGVEVHNAKTKPREEQYNSTYRVVSVLTVLHQDWLNGKEYKCKVSNKALPAPIEKTISKAKGQPREPQVYTLPPSREEMTKNQVSLWCLVKGFYPSDIAVEWESNGQPENNYKTTPPVLDSDGSFFLYSKLTVDKSRWQQGNVFSCSVMHEALHNHYTQKSLSLSPG

SEQ ID NO: 147 - protein, 227 aa, synthetic construct
DKTHTCPPCPAPELLGGPSVFLFPPKPKDTLMISRTPEVTCVVVDVSHEDPEVKFNWYVDGVEVHNAKTKPREEQYNSTYRVVSVLTVLHRDWLNGKEYKCKVSNKALPAPIEKTISKAKGQPREPQVYTLPPSREEMTKNQVSLWCLVKGFYPSDIAVEWESNGQPENNYKTTPPVLDSDGSFFLYSKLTVDKSRWQQGNVFSCSVEHEALHWHYTQKSLSLSPGK

SEQ ID NO: 148 - protein, 226 aa, synthetic construct
DKTHTCPPCPAPELLGGPSVFLFPPKPKDTLMISRTPEVTCVVVDVSHEDPEVKFNWYVDGVEVHNAKTKPREEQYNSTYRVVSVLTVLHRDWLNGKEYKCKVSNKALPAPIEKTISKAKGQPREPQVYTLPPSREEMTKNQVSLWCLVKGFYPSDIAVEWESNGQPENNYKTTPPVLDSDGSFFLYSKLTVDKSRWQQGNVFSCSVEHEALHWHYTQKSLSLSPG

SEQ ID NO: 149 - protein, 227 aa, synthetic construct
DKTHTCPPCPAPESTRGPSVFLFPPKPKDTLMISRTPEVTCVVVDVSHEDPEVKFNWYVDGVEVHNAKTKPREEQYNSTYRVVSVLTVLHRDWLNGKEYKCKVSNKALPAPIEKTISKAKGQPREPQVYTLPPSREEMTKNQVSLWCLVKGFYPSDIAVEWESNGQPENNYKTTPPVLDSDGSFFLYSKLTVDKSRWQQGNVFSCSVEHEALHWHYTQKSLSLSPGK

SEQ ID NO: 150 - protein, 226 aa, synthetic construct
DKTHTCPPCPAPESTRGPSVFLFPPKPKDTLMISRTPEVTCVVVDVSHEDPEVKFNWYVDGVEVHNAKTKPREEQYNSTYRVVSVLTVLHRDWLNGKEYKCKVSNKALPAPIEKTISKAKGQPREPQVYTLPPSREEMTKNQVSLWCLVKGFYPSDIAVEWESNGQPENNYKTTPPVLDSDGSFFLYSKLTVDKSRWQQGNVFSCSVEHEALHWHYTQKSLSLSPG

SEQ ID NO: 151 - protein, 227 aa, synthetic construct
DKTHTCPPCPAPEAAGGPSVFLFPPKPKDTLMISRTPEVTCVVVDVSHEDPEVKFNWYVDGVEVHNAKTKPREEQYNSTYRVVSVLTVLHRDWLNGKEYKCKVSNKALPAPIEKTISKAKGQPREPQVYTLPPSREEMTKNQVSLWCLVKGFYPSDIAVEWESNGQPENNYKTTPPVLDSDGSFFLYSKLTVDKSRWQQGNVFSCSVEHEALHWHYTQKSLSLSPGK

SEQ ID NO: 152 - protein, 226 aa, synthetic construct
DKTHTCPPCPAPEAAGGPSVFLFPPKPKDTLMISRTPEVTCVVVDVSHEDPEVKFNWYVDGVEVHNAKTKPREEQYNSTYRVVSVLTVLHRDWLNGKEYKCKVSNKALPAPIEKTISKAKGQPREPQVYTLPPSREEMTKNQVSLWCLVKGFYPSDIAVEWESNGQPENNYKTTPPVLDSDGSFFLYSKLTVDKSRWQQGNVFSCSVEHEALHWHYTQKSLSLSPG

SEQ ID NO: 153 - protein, 227 aa, synthetic construct
DKTHTCPPCPAPELLGGPSVFLFPPKPKDTLMISRTPEVTCVVVDVSHEDPEVKFNWYVDGVEVHNAKTKPREEQYNSTYRVVSVLTVLHQDWLNGKEYKCKVSNKALPAPIEKTISKAKGQPREPQVYTLPPSREEMTKNQVSLWCLVKGFYPSDIAVEWESNGQPENNYKTTPPVLDSDGSFFLYSKLTVDKSRWQQGNVFSCSVLHEALHSHYTQKSLSLSPGK

SEQ ID NO: 154 - protein, 226 aa, synthetic construct
DKTHTCPPCPAPELLGGPSVFLFPPKPKDTLMISRTPEVTCVVVDVSHEDPEVKFNWYVDGVEVHNAKTKPREEQYNSTYRVVSVLTVLHQDWLNGKEYKCKVSNKALPAPIEKTISKAKGQPREPQVYTLPPSREEMTKNQVSLWCLVKGFYPSDIAVEWESNGQPENNYKTTPPVLDSDGSFFLYSKLTVDKSRWQQGNVFSCSVLHEALHSHYTQKSLSLSPG

SEQ ID NO: 155 - protein, 227 aa, synthetic construct
DKTHTCPPCPAPESTRGPSVFLFPPKPKDTLMISRTPEVTCVVVDVSHEDPEVKFNWYVDGVEVHNAKTKPREEQYNSTYRVVSVLTVLHQDWLNGKEYKCKVSNKALPAPIEKTISKAKGQPREPQVYTLPPSREEMTKNQVSLWCLVKGFYPSDIAVEWESNGQPENNYKTTPPVLDSDGSFFLYSKLTVDKSRWQQGNVFSCSVLHEALHSHYTQKSLSLSPGK

SEQ ID NO: 156 - protein, 226 aa, synthetic construct
DKTHTCPPCPAPESTRGPSVFLFPPKPKDTLMISRTPEVTCVVVDVSHEDPEVKFNWYVDGVEVHNAKTKPREEQYNSTYRVVSVLTVLHQDWLNGKEYKCKVSNKALPAPIEKTISKAKGQPREPQVYTLPPSREEMTKNQVSLWCLVKGFYPSDIAVEWESNGQPENNYKTTPPVLDSDGSFFLYSKLTVDKSRWQQGNVFSCSVLHEALHSHYTQKSLSLSPG

SEQ ID NO: 157 - protein, 227 aa, synthetic construct
DKTHTCPPCPAPEAAGGPSVFLFPPKPKDTLMISRTPEVTCVVVDVSHEDPEVKFNWYVDGVEVHNAKTKPREEQYNSTYRVVSVLTVLHQDWLNGKEYKCKVSNKALPAPIEKTISKAKGQPREPQVYTLPPSREEMTKNQVSLWCLVKGFYPSDIAVEWESNGQPENNYKTTPPVLDSDGSFFLYSKLTVDKSRWQQGNVFSCSVLHEALHSHYTQKSLSLSPGK

SEQ ID NO: 158 - protein, 226 aa, synthetic construct
DKTHTCPPCPAPEAAGGPSVFLFPPKPKDTLMISRTPEVTCVVVDVSHEDPEVKFNWYVDGVEVHNAKTKPREEQYNSTYRVVSVLTVLHQDWLNGKEYKCKVSNKALPAPIEKTISKAKGQPREPQVYTLPPSREEMTKNQVSLWCLVKGFYPSDIAVEWESNGQPENNYKTTPPVLDSDGSFFLYSKLTVDKSRWQQGNVFSCSVLHEALHSHYTQKSLSLSPG

SEQ ID NO: 159 - protein, 227 aa, synthetic construct
DKTHTCPPCPAPELLGGPSVFLFPPKPKDQLMISRTPEVTCVVVDVSHEDPEVKFNWYVDGVEVHNAKTKPREEQYNSTYRVVSVLTVLHQDWLNGKEYKCKVSNKALPAPIEKTISKAKGQPREPQVYTLPPSREEMTKNQVSLWCLVKGFYPSDIAVEWESNGQPENNYKTTPPVLDSDGSFFLYSKLTVDKSRWQQGNVFSCSVLHEALHNHYTQKSLSLSPGK

SEQ ID NO: 160 - protein, 226 aa, synthetic construct
DKTHTCPPCPAPELLGGPSVFLFPPKPKDQLMISRTPEVTCVVVDVSHEDPEVKFNWYVDGVEVHNAKTKPREEQYNSTYRVVSVLTVLHQDWLNGKEYKCKVSNKALPAPIEKTISKAKGQPREPQVYTLPPSREEMTKNQVSLWCLVKGFYPSDIAVEWESNGQPENNYKTTPPVLDSDGSFFLYSKLTVDKSRWQQGNVFSCSVLHEALHNHYTQKSLSLSPG

SEQ ID NO: 161 - protein, 227 aa, synthetic construct
DKTHTCPPCPAPESTRGPSVFLFPPKPKDQLMISRTPEVTCVVVDVSHEDPEVKFNWYVDGVEVHNAKTKPREEQYNSTYRVVSVLTVLHQDWLNGKEYKCKVSNKALPAPIEKTISKAKGQPREPQVYTLPPSREEMTKNQVSLWCLVKGFYPSDIAVEWESNGQPENNYKTTPPVLDSDGSFFLYSKLTVDKSRWQQGNVFSCSVLHEALHNHYTQKSLSLSPGK

SEQ ID NO: 162 - protein, 226 aa, synthetic construct
DKTHTCPPCPAPESTRGPSVFLFPPKPKDQLMISRTPEVTCVVVDVSHEDPEVKFNWYVDGVEVHNAKTKPREEQYNSTYRVVSVLTVLHQDWLNGKEYKCKVSNKALPAPIEKTISKAKGQPREPQVYTLPPSREEMTKNQVSLWCLVKGFYPSDIAVEWESNGQPENNYKTTPPVLDSDGSFFLYSKLTVDKSRWQQGNVFSCSVLHEALHNHYTQKSLSLSPG

SEQ ID NO: 163 - protein, 227 aa, synthetic construct
DKTHTCPPCPAPEAAGGPSVFLFPPKPKDQLMISRTPEVTCVVVDVSHEDPEVKFNWYVDGVEVHNAKTKPREEQYNSTYRVVSVLTVLHQDWLNGKEYKCKVSNKALPAPIEKTISKAKGQPREPQVYTLPPSREEMTKNQVSLWCLVKGFYPSDIAVEWESNGQPENNYKTTPPVLDSDGSFFLYSKLTVDKSRWQQGNVFSCSVLHEALHNHYTQKSLSLSPGK

SEQ ID NO: 164 - protein, 226 aa, synthetic construct
DKTHTCPPCPAPEAAGGPSVFLFPPKPKDQLMISRTPEVTCVVVDVSHEDPEVKFNWYVDGVEVHNAKTKPREEQYNSTYRVVSVLTVLHQDWLNGKEYKCKVSNKALPAPIEKTISKAKGQPREPQVYTLPPSREEMTKNQVSLWCLVKGFYPSDIAVEWESNGQPENNYKTTPPVLDSDGSFFLYSKLTVDKSRWQQGNVFSCSVLHEALHNHYTQKSLSLSPG

SEQ ID NO: 165 - protein, 227 aa, synthetic construct
DKTHTCPPCPAPELLGGPSVFLFPPKPKDTLMISRTPEVTCVVVDVSHEDPEVKFNWYVDGVEVHNAKTKPREEQYNSTYRVVSVLTVDHHDWLNGKEYKCKVSNKALPAPIEKTISKAKGQPREPQVYTLPPSREEMTKNQVSLWCLVKGFYPSDIAVEWESNGQPENNYKTTPPVLDSDGSFFLYSKLTVDKSRWQQGNVFSCSVMHEALHSHYTQKSLSLSPGK

SEQ ID NO: 166 - protein, 226 aa, synthetic construct
DKTHTCPPCPAPELLGGPSVFLFPPKPKDTLMISRTPEVTCVVVDVSHEDPEVKFNWYVDGVEVHNAKTKPREEQYNSTYRVVSVLTVDHHDWLNGKEYKCKVSNKALPAPIEKTISKAKGQPREPQVYTLPPSREEMTKNQVSLWCLVKGFYPSDIAVEWESNGQPENNYKTTPPVLDSDGSFFLYSKLTVDKSRWQQGNVFSCSVMHEALHSHYTQKSLSLSPG

SEQ ID NO: 167 - protein, 227 aa, synthetic construct
DKTHTCPPCPAPESTRGPSVFLFPPKPKDTLMISRTPEVTCVVVDVSHEDPEVKFNWYVDGVEVHNAKTKPREEQYNSTYRVVSVLTVDHHDWLNGKEYKCKVSNKALPAPIEKTISKAKGQPREPQVYTLPPSREEMTKNQVSLWCLVKGFYPSDIAVEWESNGQPENNYKTTPPVLDSDGSFFLYSKLTVDKSRWQQGNVFSCSVMHEALHSHYTQKSLSLSPGK

SEQ ID NO: 168 - protein, 226 aa, synthetic construct
DKTHTCPPCPAPESTRGPSVFLFPPKPKDTLMISRTPEVTCVVVDVSHEDPEVKFNWYVDGVEVHNAKTKPREEQYNSTYRVVSVLTVDHHDWLNGKEYKCKVSNKALPAPIEKTISKAKGQPREPQVYTLPPSREEMTKNQVSLWCLVKGFYPSDIAVEWESNGQPENNYKTTPPVLDSDGSFFLYSKLTVDKSRWQQGNVFSCSVMHEALHSHYTQKSLSLSPG

SEQ ID NO: 169 - protein, 227 aa, synthetic construct
DKTHTCPPCPAPEAAGGPSVFLFPPKPKDTLMISRTPEVTCVVVDVSHEDPEVKFNWYVDGVEVHNAKTKPREEQYNSTYRVVSVLTVDHHDWLNGKEYKCKVSNKALPAPIEKTISKAKGQPREPQVYTLPPSREEMTKNQVSLWCLVKGFYPSDIAVEWESNGQPENNYKTTPPVLDSDGSFFLYSKLTVDKSRWQQGNVFSCSVMHEALHSHYTQKSLSLSPGK

SEQ ID NO: 170 - protein, 226 aa, synthetic construct
DKTHTCPPCPAPEAAGGPSVFLFPPKPKDTLMISRTPEVTCVVVDVSHEDPEVKFNWYVDGVEVHNAKTKPREEQYNSTYRVVSVLTVDHHDWLNGKEYKCKVSNKALPAPIEKTISKAKGQPREPQVYTLPPSREEMTKNQVSLWCLVKGFYPSDIAVEWESNGQPENNYKTTPPVLDSDGSFFLYSKLTVDKSRWQQGNVFSCSVMHEALHSHYTQKSLSLSPG

SEQ ID NO: 171 - protein, 227 aa, synthetic construct
KYGPPCPPCPAPEFLGGPSVFLFPPKPKDTLMISRTPEVTCVVVDVSQEDPEVQFNWYVDGVEVHNAKTKPREEQFNSTYRVVSVLTVLHQDWLNGKEYKCKVSNKGLPSSIEKTISKAKGQPREPQVYTLPPSQEEMTKNQVSLWCLVKGFYPSDIAVEWESNGQPENNYKTTPPVLDSDGSFFLYSRLTVDKSRWQEGNVFSCSVMHEALHNHYTQKSLSLSLGK

SEQ ID NO: 172 - protein, 226 aa, synthetic construct
KYGPPCPPCPAPEFLGGPSVFLFPPKPKDTLMISRTPEVTCVVVDVSQEDPEVQFNWYVDGVEVHNAKTKPREEQFNSTYRVVSVLTVLHQDWLNGKEYKCKVSNKGLPSSIEKTISKAKGQPREPQVYTLPPSQEEMTKNQVSLWCLVKGFYPSDIAVEWESNGQPENNYKTTPPVLDSDGSFFLYSRLTVDKSRWQEGNVFSCSVMHEALHNHYTQKSLSLSLG

SEQ ID NO: 173 - protein, 227 aa, synthetic construct
KYGPPCPPCPAPESTRGPSVFLFPPKPKDTLMISRTPEVTCVVVDVSQEDPEVQFNWYVDGVEVHNAKTKPREEQFNSTYRVVSVLTVLHQDWLNGKEYKCKVSNKGLPSSIEKTISKAKGQPREPQVYTLPPSQEEMTKNQVSLWCLVKGFYPSDIAVEWESNGQPENNYKTTPPVLDSDGSFFLYSRLTVDKSRWQEGNVFSCSVMHEALHNHYTQKSLSLSLGK

SEQ ID NO: 174 - protein, 226 aa, synthetic construct
KYGPPCPPCPAPESTRGPSVFLFPPKPKDTLMISRTPEVTCVVVDVSQEDPEVQFNWYVDGVEVHNAKTKPREEQFNSTYRVVSVLTVLHQDWLNGKEYKCKVSNKGLPSSIEKTISKAKGQPREPQVYTLPPSQEEMTKNQVSLWCLVKGFYPSDIAVEWESNGQPENNYKTTPPVLDSDGSFFLYSRLTVDKSRWQEGNVFSCSVMHEALHNHYTQKSLSLSLG

SEQ ID NO: 175 - protein, 227 aa, synthetic construct
KYGPPCPPCPAPEAAGGPSVFLFPPKPKDTLMISRTPEVTCVVVDVSQEDPEVQFNWYVDGVEVHNAKTKPREEQFNSTYRVVSVLTVLHQDWLNGKEYKCKVSNKGLPSSIEKTISKAKGQPREPQVYTLPPSQEEMTKNQVSLWCLVKGFYPSDIAVEWESNGQPENNYKTTPPVLDSDGSFFLYSRLTVDKSRWQEGNVFSCSVMHEALHNHYTQKSLSLSLGK

SEQ ID NO: 176 - protein, 226 aa, synthetic construct
KYGPPCPPCPAPEAAGGPSVFLFPPKPKDTLMISRTPEVTCVVVDVSQEDPEVQFNWYVDGVEVHNAKTKPREEQFNSTYRVVSVLTVLHQDWLNGKEYKCKVSNKGLPSSIEKTISKAKGQPREPQVYTLPPSQEEMTKNQVSLWCLVKGFYPSDIAVEWESNGQPENNYKTTPPVLDSDGSFFLYSRLTVDKSRWQEGNVFSCSVMHEALHNHYTQKSLSLSLG

SEQ ID NO: 177 - protein, 227 aa, synthetic construct
KYGPPCPPCPAPEFLGGPSVFLFPPKPKDTLYITREPEVTCVVVDVSQEDPEVQFNWYVDGVEVHNAKTKPREEQFNSTYRVVSVLTVLHQDWLNGKEYKCKVSNKGLPSSIEKTISKAKGQPREPQVYTLPPSQEEMTKNQVSLWCLVKGFYPSDIAVEWESNGQPENNYKTTPPVLDSDGSFFLYSRLTVDKSRWQEGNVFSCSVMHEALHNHYTQKSLSLSLGK

SEQ ID NO: 178 - protein, 226 aa, synthetic construct
KYGPPCPPCPAPEFLGGPSVFLFPPKPKDTLYITREPEVTCVVVDVSQEDPEVQFNWYVDGVEVHNAKTKPREEQFNSTYRVVSVLTVLHQDWLNGKEYKCKVSNKGLPSSIEKTISKAKGQPREPQVYTLPPSQEEMTKNQVSLWCLVKGFYPSDIAVEWESNGQPENNYKTTPPVLDSDGSFFLYSRLTVDKSRWQEGNVFSCSVMHEALHNHYTQKSLSLSLG

SEQ ID NO: 179 - protein, 227 aa, synthetic construct
KYGPPCPPCPAPESTRGPSVFLFPPKPKDTLYITREPEVTCVVVDVSQEDPEVQFNWYVDGVEVHNAKTKPREEQFNSTYRVVSVLTVLHQDWLNGKEYKCKVSNKGLPSSIEKTISKAKGQPREPQVYTLPPSQEEMTKNQVSLWCLVKGFYPSDIAVEWESNGQPENNYKTTPPVLDSDGSFFLYSRLTVDKSRWQEGNVFSCSVMHEALHNHYTQKSLSLSLGK

SEQ ID NO: 180 - protein, 226 aa, synthetic construct
KYGPPCPPCPAPESTRGPSVFLFPPKPKDTLYITREPEVTCVVVDVSQEDPEVQFNWYVDGVEVHNAKTKPREEQFNSTYRVVSVLTVLHQDWLNGKEYKCKVSNKGLPSSIEKTISKAKGQPREPQVYTLPPSQEEMTKNQVSLWCLVKGFYPSDIAVEWESNGQPENNYKTTPPVLDSDGSFFLYSRLTVDKSRWQEGNVFSCSVMHEALHNHYTQKSLSLSLG

SEQ ID NO: 181 - protein, 227 aa, synthetic construct
KYGPPCPPCPAPEAAGGPSVFLFPPKPKDTLYITREPEVTCVVVDVSQEDPEVQFNWYVDGVEVHNAKTKPREEQFNSTYRVVSVLTVLHQDWLNGKEYKCKVSNKGLPSSIEKTISKAKGQPREPQVYTLPPSQEEMTKNQVSLWCLVKGFYPSDIAVEWESNGQPENNYKTTPPVLDSDGSFFLYSRLTVDKSRWQEGNVFSCSVMHEALHNHYTQKSLSLSLGK

SEQ ID NO: 182 - protein, 226 aa, synthetic construct
KYGPPCPPCPAPEAAGGPSVFLFPPKPKDTLYITREPEVTCVVVDVSQEDPEVQFNWYVDGVEVHNAKTKPREEQFNSTYRVVSVLTVLHQDWLNGKEYKCKVSNKGLPSSIEKTISKAKGQPREPQVYTLPPSQEEMTKNQVSLWCLVKGFYPSDIAVEWESNGQPENNYKTTPPVLDSDGSFFLYSRLTVDKSRWQEGNVFSCSVMHEALHNHYTQKSLSLSLG

SEQ ID NO: 183 - protein, 227 aa, synthetic construct
KYGPPCPPCPAPEFLGGPSVFLFPPKPKDTLMISRTPEVTCVVVDVSQEDPEVQFNWYVDGVEVHNAKTKPREEQFNSTYRVVSVLTVLHRDWLNGKEYKCKVSNKGLPSSIEKTISKAKGQPREPQVYTLPPSQEEMTKNQVSLWCLVKGFYPSDIAVEWESNGQPENNYKTTPPVLDSDGSFFLYSRLTVDKSRWQEGNVFSCSVEHEALHWHYTQKSLSLSLGK

SEQ ID NO: 184 - protein, 226 aa, synthetic construct
KYGPPCPPCPAPEFLGGPSVFLFPPKPKDTLMISRTPEVTCVVVDVSQEDPEVQFNWYVDGVEVHNAKTKPREEQFNSTYRVVSVLTVLHRDWLNGKEYKCKVSNKGLPSSIEKTISKAKGQPREPQVYTLPPSQEEMTKNQVSLWCLVKGFYPSDIAVEWESNGQPENNYKTTPPVLDSDGSFFLYSRLTVDKSRWQEGNVFSCSVEHEALHWHYTQKSLSLSLG

SEQ ID NO: 185 - protein, 227 aa, synthetic construct
KYGPPCPPCPAPESTRGPSVFLFPPKPKDTLMISRTPEVTCVVVDVSQEDPEVQFNWYVDGVEVHNAKTKPREEQFNSTYRVVSVLTVLHRDWLNGKEYKCKVSNKGLPSSIEKTISKAKGQPREPQVYTLPPSQEEMTKNQVSLWCLVKGFYPSDIAVEWESNGQPENNYKTTPPVLDSDGSFFLYSRLTVDKSRWQEGNVFSCSVEHEALHWHYTQKSLSLSLGK

SEQ ID NO: 186 - protein, 226 aa, synthetic construct
KYGPPCPPCPAPESTRGPSVFLFPPKPKDTLMISRTPEVTCVVVDVSQEDPEVQFNWYVDGVEVHNAKTKPREEQFNSTYRVVSVLTVLHRDWLNGKEYKCKVSNKGLPSSIEKTISKAKGQPREPQVYTLPPSQEEMTKNQVSLWCLVKGFYPSDIAVEWESNGQPENNYKTTPPVLDSDGSFFLYSRLTVDKSRWQEGNVFSCSVEHEALHWHYTQKSLSLSLG

SEQ ID NO: 187 - protein, 227 aa, synthetic construct
KYGPPCPPCPAPEAAGGPSVFLFPPKPKDTLMISRTPEVTCVVVDVSQEDPEVQFNWYVDGVEVHNAKTKPREEQFNSTYRVVSVLTVLHRDWLNGKEYKCKVSNKGLPSSIEKTISKAKGQPREPQVYTLPPSQEEMTKNQVSLWCLVKGFYPSDIAVEWESNGQPENNYKTTPPVLDSDGSFFLYSRLTVDKSRWQEGNVFSCSVEHEALHWHYTQKSLSLSLGK

SEQ ID NO: 188 - protein, 226 aa, synthetic construct
KYGPPCPPCPAPEAAGGPSVFLFPPKPKDTLMISRTPEVTCVVVDVSQEDPEVQFNWYVDGVEVHNAKTKPREEQFNSTYRVVSVLTVLHRDWLNGKEYKCKVSNKGLPSSIEKTISKAKGQPREPQVYTLPPSQEEMTKNQVSLWCLVKGFYPSDIAVEWESNGQPENNYKTTPPVLDSDGSFFLYSRLTVDKSRWQEGNVFSCSVEHEALHWHYTQKSLSLSLG

SEQ ID NO: 189 - protein, 227 aa, synthetic construct
KYGPPCPPCPAPEFLGGPSVFLFPPKPKDTLMISRTPEVTCVVVDVSQEDPEVQFNWYVDGVEVHNAKTKPREEQFNSTYRVVSVLTVLHQDWLNGKEYKCKVSNKGLPSSIEKTISKAKGQPREPQVYTLPPSQEEMTKNQVSLWCLVKGFYPSDIAVEWESNGQPENNYKTTPPVLDSDGSFFLYSRLTVDKSRWQEGNVFSCSVLHEALHSHYTQKSLSLSLGK

SEQ ID NO: 190 - protein, 226 aa, synthetic construct
KYGPPCPPCPAPEFLGGPSVFLFPPKPKDTLMISRTPEVTCVVVDVSQEDPEVQFNWYVDGVEVHNAKTKPREEQFNSTYRVVSVLTVLHQDWLNGKEYKCKVSNKGLPSSIEKTISKAKGQPREPQVYTLPPSQEEMTKNQVSLWCLVKGFYPSDIAVEWESNGQPENNYKTTPPVLDSDGSFFLYSRLTVDKSRWQEGNVFSCSVLHEALHSHYTQKSLSLSLG

SEQ ID NO: 191 - protein, 227 aa, synthetic construct
KYGPPCPPCPAPESTRGPSVFLFPPKPKDTLMISRTPEVTCVVVDVSQEDPEVQFNWYVDGVEVHNAKTKPREEQFNSTYRVVSVLTVLHQDWLNGKEYKCKVSNKGLPSSIEKTISKAKGQPREPQVYTLPPSQEEMTKNQVSLWCLVKGFYPSDIAVEWESNGQPENNYKTTPPVLDSDGSFFLYSRLTVDKSRWQEGNVFSCSVLHEALHSHYTQKSLSLSLGK

SEQ ID NO: 192 - protein, 226 aa, synthetic construct
KYGPPCPPCPAPESTRGPSVFLFPPKPKDTLMISRTPEVTCVVVDVSQEDPEVQFNWYVDGVEVHNAKTKPREEQFNSTYRVVSVLTVLHQDWLNGKEYKCKVSNKGLPSSIEKTISKAKGQPREPQVYTLPPSQEEMTKNQVSLWCLVKGFYPSDIAVEWESNGQPENNYKTTPPVLDSDGSFFLYSRLTVDKSRWQEGNVFSCSVLHEALHSHYTQKSLSLSLG

SEQ ID NO: 193 - protein, 227 aa, synthetic construct
KYGPPCPPCPAPEAAGGPSVFLFPPKPKDTLMISRTPEVTCVVVDVSQEDPEVQFNWYVDGVEVHNAKTKPREEQFNSTYRVVSVLTVLHQDWLNGKEYKCKVSNKGLPSSIEKTISKAKGQPREPQVYTLPPSQEEMTKNQVSLWCLVKGFYPSDIAVEWESNGQPENNYKTTPPVLDSDGSFFLYSRLTVDKSRWQEGNVFSCSVLHEALHSHYTQKSLSLSLGK

SEQ ID NO: 194 - protein, 226 aa, synthetic construct
KYGPPCPPCPAPEAAGGPSVFLFPPKPKDTLMISRTPEVTCVVVDVSQEDPEVQFNWYVDGVEVHNAKTKPREEQFNSTYRVVSVLTVLHQDWLNGKEYKCKVSNKGLPSSIEKTISKAKGQPREPQVYTLPPSQEEMTKNQVSLWCLVKGFYPSDIAVEWESNGQPENNYKTTPPVLDSDGSFFLYSRLTVDKSRWQEGNVFSCSVLHEALHSHYTQKSLSLSLG

SEQ ID NO: 195 - protein, 227 aa, synthetic construct
KYGPPCPPCPAPEFLGGPSVFLFPPKPKDQLMISRTPEVTCVVVDVSQEDPEVQFNWYVDGVEVHNAKTKPREEQFNSTYRVVSVLTVLHQDWLNGKEYKCKVSNKGLPSSIEKTISKAKGQPREPQVYTLPPSQEEMTKNQVSLWCLVKGFYPSDIAVEWESNGQPENNYKTTPPVLDSDGSFFLYSRLTVDKSRWQEGNVFSCSVLHEALHNHYTQKSLSLSLGK

SEQ ID NO: 196 - protein, 226 aa, synthetic construct
KYGPPCPPCPAPEFLGGPSVFLFPPKPKDQLMISRTPEVTCVVVDVSQEDPEVQFNWYVDGVEVHNAKTKPREEQFNSTYRVVSVLTVLHQDWLNGKEYKCKVSNKGLPSSIEKTISKAKGQPREPQVYTLPPSQEEMTKNQVSLWCLVKGFYPSDIAVEWESNGQPENNYKTTPPVLDSDGSFFLYSRLTVDKSRWQEGNVFSCSVLHEALHNHYTQKSLSLSLG

SEQ ID NO: 197 - protein, 227 aa, synthetic construct
KYGPPCPPCPAPESTRGPSVFLFPPKPKDQLMISRTPEVTCVVVDVSQEDPEVQFNWYVDGVEVHNAKTKPREEQFNSTYRVVSVLTVLHQDWLNGKEYKCKVSNKGLPSSIEKTISKAKGQPREPQVYTLPPSQEEMTKNQVSLWCLVKGFYPSDIAVEWESNGQPENNYKTTPPVLDSDGSFFLYSRLTVDKSRWQEGNVFSCSVLHEALHNHYTQKSLSLSLGK

SEQ ID NO: 198 - protein, 226 aa, synthetic construct
KYGPPCPPCPAPESTRGPSVFLFPPKPKDQLMISRTPEVTCVVVDVSQEDPEVQFNWYVDGVEVHNAKTKPREEQFNSTYRVVSVLTVLHQDWLNGKEYKCKVSNKGLPSSIEKTISKAKGQPREPQVYTLPPSQEEMTKNQVSLWCLVKGFYPSDIAVEWESNGQPENNYKTTPPVLDSDGSFFLYSRLTVDKSRWQEGNVFSCSVLHEALHNHYTQKSLSLSLG

SEQ ID NO: 199 - protein, 227 aa, synthetic construct
KYGPPCPPCPAPEAAGGPSVFLFPPKPKDQLMISRTPEVTCVVVDVSQEDPEVQFNWYVDGVEVHNAKTKPREEQFNSTYRVVSVLTVLHQDWLNGKEYKCKVSNKGLPSSIEKTISKAKGQPREPQVYTLPPSQEEMTKNQVSLWCLVKGFYPSDIAVEWESNGQPENNYKTTPPVLDSDGSFFLYSRLTVDKSRWQEGNVFSCSVLHEALHNHYTQKSLSLSLGK

SEQ ID NO: 200 - protein, 226 aa, synthetic construct
KYGPPCPPCPAPEAAGGPSVFLFPPKPKDQLMISRTPEVTCVVVDVSQEDPEVQFNWYVDGVEVHNAKTKPREEQFNSTYRVVSVLTVLHQDWLNGKEYKCKVSNKGLPSSIEKTISKAKGQPREPQVYTLPPSQEEMTKNQVSLWCLVKGFYPSDIAVEWESNGQPENNYKTTPPVLDSDGSFFLYSRLTVDKSRWQEGNVFSCSVLHEALHNHYTQKSLSLSLG

SEQ ID NO: 201 - protein, 227 aa, synthetic construct
KYGPPCPPCPAPEFLGGPSVFLFPPKPKDTLMISRTPEVTCVVVDVSQEDPEVQFNWYVDGVEVHNAKTKPREEQFNSTYRVVSVLTVDHHDWLNGKEYKCKVSNKGLPSSIEKTISKAKGQPREPQVYTLPPSQEEMTKNQVSLWCLVKGFYPSDIAVEWESNGQPENNYKTTPPVLDSDGSFFLYSRLTVDKSRWQEGNVFSCSVMHEALHSHYTQKSLSLSLGK

SEQ ID NO: 202 - protein, 226 aa, synthetic construct
KYGPPCPPCPAPEFLGGPSVFLFPPKPKDTLMISRTPEVTCVVVDVSQEDPEVQFNWYVDGVEVHNAKTKPREEQFNSTYRVVSVLTVDHHDWLNGKEYKCKVSNKGLPSSIEKTISKAKGQPREPQVYTLPPSQEEMTKNQVSLWCLVKGFYPSDIAVEWESNGQPENNYKTTPPVLDSDGSFFLYSRLTVDKSRWQEGNVFSCSVMHEALHSHYTQKSLSLSLG

SEQ ID NO: 203 - protein, 227 aa, synthetic construct
KYGPPCPPCPAPESTRGPSVFLFPPKPKDTLMISRTPEVTCVVVDVSQEDPEVQFNWYVDGVEVHNAKTKPREEQFNSTYRVVSVLTVDHHDWLNGKEYKCKVSNKGLPSSIEKTISKAKGQPREPQVYTLPPSQEEMTKNQVSLWCLVKGFYPSDIAVEWESNGQPENNYKTTPPVLDSDGSFFLYSRLTVDKSRWQEGNVFSCSVMHEALHSHYTQKSLSLSLGK

SEQ ID NO: 204 - protein, 226 aa, synthetic construct
KYGPPCPPCPAPESTRGPSVFLFPPKPKDTLMISRTPEVTCVVVDVSQEDPEVQFNWYVDGVEVHNAKTKPREEQFNSTYRVVSVLTVDHHDWLNGKEYKCKVSNKGLPSSIEKTISKAKGQPREPQVYTLPPSQEEMTKNQVSLWCLVKGFYPSDIAVEWESNGQPENNYKTTPPVLDSDGSFFLYSRLTVDKSRWQEGNVFSCSVMHEALHSHYTQKSLSLSLG

SEQ ID NO: 205 - protein, 227 aa, synthetic construct
KYGPPCPPCPAPEAAGGPSVFLFPPKPKDTLMISRTPEVTCVVVDVSQEDPEVQFNWYVDGVEVHNAKTKPREEQFNSTYRVVSVLTVDHHDWLNGKEYKCKVSNKGLPSSIEKTISKAKGQPREPQVYTLPPSQEEMTKNQVSLWCLVKGFYPSDIAVEWESNGQPENNYKTTPPVLDSDGSFFLYSRLTVDKSRWQEGNVFSCSVMHEALHSHYTQKSLSLSLGK

SEQ ID NO: 206 - protein, 226 aa, synthetic construct
KYGPPCPPCPAPEAAGGPSVFLFPPKPKDTLMISRTPEVTCVVVDVSQEDPEVQFNWYVDGVEVHNAKTKPREEQFNSTYRVVSVLTVDHHDWLNGKEYKCKVSNKGLPSSIEKTISKAKGQPREPQVYTLPPSQEEMTKNQVSLWCLVKGFYPSDIAVEWESNGQPENNYKTTPPVLDSDGSFFLYSRLTVDKSRWQEGNVFSCSVMHEALHSHYTQKSLSLSLG

SEQ ID NO: 207 - protein, 227 aa, synthetic construct
KYGPPCPSCPAPEFLGGPSVFLFPPKPKDTLMISRTPEVTCVVVDVSQEDPEVQFNWYVDGVEVHNAKTKPREEQFNSTYRVVSVLTVLHQDWLNGKEYKCKVSNKGLPSSIEKTISKAKGQPREPQVYTLPPSQEEMTKNQVSLWCLVKGFYPSDIAVEWESNGQPENNYKTTPPVLDSDGSFFLYSRLTVDKSRWQEGNVFSCSVMHEALHNHYTQKSLSLSLGK

SEQ ID NO: 208 - protein, 226 aa, synthetic construct
KYGPPCPSCPAPEFLGGPSVFLFPPKPKDTLMISRTPEVTCVVVDVSQEDPEVQFNWYVDGVEVHNAKTKPREEQFNSTYRVVSVLTVLHQDWLNGKEYKCKVSNKGLPSSIEKTISKAKGQPREPQVYTLPPSQEEMTKNQVSLWCLVKGFYPSDIAVEWESNGQPENNYKTTPPVLDSDGSFFLYSRLTVDKSRWQEGNVFSCSVMHEALHNHYTQKSLSLSLG

SEQ ID NO: 209 - protein, 227 aa, synthetic construct
KYGPPCPSCPAPESTRGPSVFLFPPKPKDTLMISRTPEVTCVVVDVSQEDPEVQFNWYVDGVEVHNAKTKPREEQFNSTYRVVSVLTVLHQDWLNGKEYKCKVSNKGLPSSIEKTISKAKGQPREPQVYTLPPSQEEMTKNQVSLWCLVKGFYPSDIAVEWESNGQPENNYKTTPPVLDSDGSFFLYSRLTVDKSRWQEGNVFSCSVMHEALHNHYTQKSLSLSLGK

SEQ ID NO: 210 - protein, 226 aa, synthetic construct
KYGPPCPSCPAPESTRGPSVFLFPPKPKDTLMISRTPEVTCVVVDVSQEDPEVQFNWYVDGVEVHNAKTKPREEQFNSTYRVVSVLTVLHQDWLNGKEYKCKVSNKGLPSSIEKTISKAKGQPREPQVYTLPPSQEEMTKNQVSLWCLVKGFYPSDIAVEWESNGQPENNYKTTPPVLDSDGSFFLYSRLTVDKSRWQEGNVFSCSVMHEALHNHYTQKSLSLSLG

SEQ ID NO: 211 - protein, 227 aa, synthetic construct
KYGPPCPSCPAPEAAGGPSVFLFPPKPKDTLMISRTPEVTCVVVDVSQEDPEVQFNWYVDGVEVHNAKTKPREEQFNSTYRVVSVLTVLHQDWLNGKEYKCKVSNKGLPSSIEKTISKAKGQPREPQVYTLPPSQEEMTKNQVSLWCLVKGFYPSDIAVEWESNGQPENNYKTTPPVLDSDGSFFLYSRLTVDKSRWQEGNVFSCSVMHEALHNHYTQKSLSLSLGK

SEQ ID NO: 212 - protein, 226 aa, synthetic construct
KYGPPCPSCPAPEAAGGPSVFLFPPKPKDTLMISRTPEVTCVVVDVSQEDPEVQFNWYVDGVEVHNAKTKPREEQFNSTYRVVSVLTVLHQDWLNGKEYKCKVSNKGLPSSIEKTISKAKGQPREPQVYTLPPSQEEMTKNQVSLWCLVKGFYPSDIAVEWESNGQPENNYKTTPPVLDSDGSFFLYSRLTVDKSRWQEGNVFSCSVMHEALHNHYTQKSLSLSLG

SEQ ID NO: 213 - protein, 227 aa, synthetic construct
KYGPPCPSCPAPEFLGGPSVFLFPPKPKDTLYITREPEVTCVVVDVSQEDPEVQFNWYVDGVEVHNAKTKPREEQFNSTYRVVSVLTVLHQDWLNGKEYKCKVSNKGLPSSIEKTISKAKGQPREPQVYTLPPSQEEMTKNQVSLWCLVKGFYPSDIAVEWESNGQPENNYKTTPPVLDSDGSFFLYSRLTVDKSRWQEGNVFSCSVMHEALHNHYTQKSLSLSLGK

SEQ ID NO: 214 - protein, 226 aa, synthetic construct
KYGPPCPSCPAPEFLGGPSVFLFPPKPKDTLYITREPEVTCVVVDVSQEDPEVQFNWYVDGVEVHNAKTKPREEQFNSTYRVVSVLTVLHQDWLNGKEYKCKVSNKGLPSSIEKTISKAKGQPREPQVYTLPPSQEEMTKNQVSLWCLVKGFYPSDIAVEWESNGQPENNYKTTPPVLDSDGSFFLYSRLTVDKSRWQEGNVFSCSVMHEALHNHYTQKSLSLSLG

SEQ ID NO: 215 - protein, 227 aa, synthetic construct
KYGPPCPSCPAPESTRGPSVFLFPPKPKDTLYITREPEVTCVVVDVSQEDPEVQFNWYVDGVEVHNAKTKPREEQFNSTYRVVSVLTVLHQDWLNGKEYKCKVSNKGLPSSIEKTISKAKGQPREPQVYTLPPSQEEMTKNQVSLWCLVKGFYPSDIAVEWESNGQPENNYKTTPPVLDSDGSFFLYSRLTVDKSRWQEGNVFSCSVMHEALHNHYTQKSLSLSLGK

SEQ ID NO: 216 - protein, 226 aa, synthetic construct
KYGPPCPSCPAPESTRGPSVFLFPPKPKDTLYITREPEVTCVVVDVSQEDPEVQFNWYVDGVEVHNAKTKPREEQFNSTYRVVSVLTVLHQDWLNGKEYKCKVSNKGLPSSIEKTISKAKGQPREPQVYTLPPSQEEMTKNQVSLWCLVKGFYPSDIAVEWESNGQPENNYKTTPPVLDSDGSFFLYSRLTVDKSRWQEGNVFSCSVMHEALHNHYTQKSLSLSLG

SEQ ID NO: 217 - protein, 227 aa, synthetic construct
KYGPPCPSCPAPEAAGGPSVFLFPPKPKDTLYITREPEVTCVVVDVSQEDPEVQFNWYVDGVEVHNAKTKPREEQFNSTYRVVSVLTVLHQDWLNGKEYKCKVSNKGLPSSIEKTISKAKGQPREPQVYTLPPSQEEMTKNQVSLWCLVKGFYPSDIAVEWESNGQPENNYKTTPPVLDSDGSFFLYSRLTVDKSRWQEGNVFSCSVMHEALHNHYTQKSLSLSLGK

SEQ ID NO: 218 - protein, 226 aa, synthetic construct
KYGPPCPSCPAPEAAGGPSVFLFPPKPKDTLYITREPEVTCVVVDVSQEDPEVQFNWYVDGVEVHNAKTKPREEQFNSTYRVVSVLTVLHQDWLNGKEYKCKVSNKGLPSSIEKTISKAKGQPREPQVYTLPPSQEEMTKNQVSLWCLVKGFYPSDIAVEWESNGQPENNYKTTPPVLDSDGSFFLYSRLTVDKSRWQEGNVFSCSVMHEALHNHYTQKSLSLSLG

SEQ ID NO: 219 - protein, 227 aa, synthetic construct
KYGPPCPSCPAPEFLGGPSVFLFPPKPKDTLMISRTPEVTCVVVDVSQEDPEVQFNWYVDGVEVHNAKTKPREEQFNSTYRVVSVLTVLHRDWLNGKEYKCKVSNKGLPSSIEKTISKAKGQPREPQVYTLPPSQEEMTKNQVSLWCLVKGFYPSDIAVEWESNGQPENNYKTTPPVLDSDGSFFLYSRLTVDKSRWQEGNVFSCSVEHEALHWHYTQKSLSLSLGK

SEQ ID NO: 220 - protein, 226 aa, synthetic construct
KYGPPCPSCPAPEFLGGPSVFLFPPKPKDTLMISRTPEVTCVVVDVSQEDPEVQFNWYVDGVEVHNAKTKPREEQFNSTYRVVSVLTVLHRDWLNGKEYKCKVSNKGLPSSIEKTISKAKGQPREPQVYTLPPSQEEMTKNQVSLWCLVKGFYPSDIAVEWESNGQPENNYKTTPPVLDSDGSFFLYSRLTVDKSRWQEGNVFSCSVEHEALHWHYTQKSLSLSLG

SEQ ID NO: 221 - protein, 227 aa, synthetic construct
KYGPPCPSCPAPESTRGPSVFLFPPKPKDTLMISRTPEVTCVVVDVSQEDPEVQFNWYVDGVEVHNAKTKPREEQFNSTYRVVSVLTVLHRDWLNGKEYKCKVSNKGLPSSIEKTISKAKGQPREPQVYTLPPSQEEMTKNQVSLWCLVKGFYPSDIAVEWESNGQPENNYKTTPPVLDSDGSFFLYSRLTVDKSRWQEGNVFSCSVEHEALHWHYTQKSLSLSLGK

SEQ ID NO: 222 - protein, 226 aa, synthetic construct
KYGPPCPSCPAPESTRGPSVFLFPPKPKDTLMISRTPEVTCVVVDVSQEDPEVQFNWYVDGVEVHNAKTKPREEQFNSTYRVVSVLTVLHRDWLNGKEYKCKVSNKGLPSSIEKTISKAKGQPREPQVYTLPPSQEEMTKNQVSLWCLVKGFYPSDIAVEWESNGQPENNYKTTPPVLDSDGSFFLYSRLTVDKSRWQEGNVFSCSVEHEALHWHYTQKSLSLSLG

SEQ ID NO: 223 - protein, 227 aa, synthetic construct
KYGPPCPSCPAPEAAGGPSVFLFPPKPKDTLMISRTPEVTCVVVDVSQEDPEVQFNWYVDGVEVHNAKTKPREEQFNSTYRVVSVLTVLHRDWLNGKEYKCKVSNKGLPSSIEKTISKAKGQPREPQVYTLPPSQEEMTKNQVSLWCLVKGFYPSDIAVEWESNGQPENNYKTTPPVLDSDGSFFLYSRLTVDKSRWQEGNVFSCSVEHEALHWHYTQKSLSLSLGK

SEQ ID NO: 224 - protein, 226 aa, synthetic construct
KYGPPCPSCPAPEAAGGPSVFLFPPKPKDTLMISRTPEVTCVVVDVSQEDPEVQFNWYVDGVEVHNAKTKPREEQFNSTYRVVSVLTVLHRDWLNGKEYKCKVSNKGLPSSIEKTISKAKGQPREPQVYTLPPSQEEMTKNQVSLWCLVKGFYPSDIAVEWESNGQPENNYKTTPPVLDSDGSFFLYSRLTVDKSRWQEGNVFSCSVEHEALHWHYTQKSLSLSLG

SEQ ID NO: 225 - protein, 227 aa, synthetic construct
KYGPPCPSCPAPEFLGGPSVFLFPPKPKDTLMISRTPEVTCVVVDVSQEDPEVQFNWYVDGVEVHNAKTKPREEQFNSTYRVVSVLTVLHQDWLNGKEYKCKVSNKGLPSSIEKTISKAKGQPREPQVYTLPPSQEEMTKNQVSLWCLVKGFYPSDIAVEWESNGQPENNYKTTPPVLDSDGSFFLYSRLTVDKSRWQEGNVFSCSVLHEALHSHYTQKSLSLSLGK

SEQ ID NO: 226 - protein, 226 aa, synthetic construct
KYGPPCPSCPAPEFLGGPSVFLFPPKPKDTLMISRTPEVTCVVVDVSQEDPEVQFNWYVDGVEVHNAKTKPREEQFNSTYRVVSVLTVLHQDWLNGKEYKCKVSNKGLPSSIEKTISKAKGQPREPQVYTLPPSQEEMTKNQVSLWCLVKGFYPSDIAVEWESNGQPENNYKTTPPVLDSDGSFFLYSRLTVDKSRWQEGNVFSCSVLHEALHSHYTQKSLSLSLG

SEQ ID NO: 227 - protein, 227 aa, synthetic construct
KYGPPCPSCPAPESTRGPSVFLFPPKPKDTLMISRTPEVTCVVVDVSQEDPEVQFNWYVDGVEVHNAKTKPREEQFNSTYRVVSVLTVLHQDWLNGKEYKCKVSNKGLPSSIEKTISKAKGQPREPQVYTLPPSQEEMTKNQVSLWCLVKGFYPSDIAVEWESNGQPENNYKTTPPVLDSDGSFFLYSRLTVDKSRWQEGNVFSCSVLHEALHSHYTQKSLSLSLGK

SEQ ID NO: 228 - protein, 226 aa, synthetic construct
KYGPPCPSCPAPESTRGPSVFLFPPKPKDTLMISRTPEVTCVVVDVSQEDPEVQFNWYVDGVEVHNAKTKPREEQFNSTYRVVSVLTVLHQDWLNGKEYKCKVSNKGLPSSIEKTISKAKGQPREPQVYTLPPSQEEMTKNQVSLWCLVKGFYPSDIAVEWESNGQPENNYKTTPPVLDSDGSFFLYSRLTVDKSRWQEGNVFSCSVLHEALHSHYTQKSLSLSLG

SEQ ID NO: 229 - protein, 227 aa, synthetic construct
KYGPPCPSCPAPEAAGGPSVFLFPPKPKDTLMISRTPEVTCVVVDVSQEDPEVQFNWYVDGVEVHNAKTKPREEQFNSTYRVVSVLTVLHQDWLNGKEYKCKVSNKGLPSSIEKTISKAKGQPREPQVYTLPPSQEEMTKNQVSLWCLVKGFYPSDIAVEWESNGQPENNYKTTPPVLDSDGSFFLYSRLTVDKSRWQEGNVFSCSVLHEALHSHYTQKSLSLSLGK

SEQ ID NO: 230 - protein, 226 aa, synthetic construct
KYGPPCPSCPAPEAAGGPSVFLFPPKPKDTLMISRTPEVTCVVVDVSQEDPEVQFNWYVDGVEVHNAKTKPREEQFNSTYRVVSVLTVLHQDWLNGKEYKCKVSNKGLPSSIEKTISKAKGQPREPQVYTLPPSQEEMTKNQVSLWCLVKGFYPSDIAVEWESNGQPENNYKTTPPVLDSDGSFFLYSRLTVDKSRWQEGNVFSCSVLHEALHSHYTQKSLSLSLG

SEQ ID NO: 231 - protein, 227 aa, synthetic construct
KYGPPCPSCPAPEFLGGPSVFLFPPKPKDQLMISRTPEVTCVVVDVSQEDPEVQFNWYVDGVEVHNAKTKPREEQFNSTYRVVSVLTVLHQDWLNGKEYKCKVSNKGLPSSIEKTISKAKGQPREPQVYTLPPSQEEMTKNQVSLWCLVKGFYPSDIAVEWESNGQPENNYKTTPPVLDSDGSFFLYSRLTVDKSRWQEGNVFSCSVLHEALHNHYTQKSLSLSLGK

SEQ ID NO: 232 - protein, 226 aa, synthetic construct
KYGPPCPSCPAPEFLGGPSVFLFPPKPKDQLMISRTPEVTCVVVDVSQEDPEVQFNWYVDGVEVHNAKTKPREEQFNSTYRVVSVLTVLHQDWLNGKEYKCKVSNKGLPSSIEKTISKAKGQPREPQVYTLPPSQEEMTKNQVSLWCLVKGFYPSDIAVEWESNGQPENNYKTTPPVLDSDGSFFLYSRLTVDKSRWQEGNVFSCSVLHEALHNHYTQKSLSLSLG

SEQ ID NO: 233 - protein, 227 aa, synthetic construct
KYGPPCPSCPAPESTRGPSVFLFPPKPKDQLMISRTPEVTCVVVDVSQEDPEVQFNWYVDGVEVHNAKTKPREEQFNSTYRVVSVLTVLHQDWLNGKEYKCKVSNKGLPSSIEKTISKAKGQPREPQVYTLPPSQEEMTKNQVSLWCLVKGFYPSDIAVEWESNGQPENNYKTTPPVLDSDGSFFLYSRLTVDKSRWQEGNVFSCSVLHEALHNHYTQKSLSLSLGK

SEQ ID NO: 234 - protein, 226 aa, synthetic construct
KYGPPCPSCPAPESTRGPSVFLFPPKPKDQLMISRTPEVTCVVVDVSQEDPEVQFNWYVDGVEVHNAKTKPREEQFNSTYRVVSVLTVLHQDWLNGKEYKCKVSNKGLPSSIEKTISKAKGQPREPQVYTLPPSQEEMTKNQVSLWCLVKGFYPSDIAVEWESNGQPENNYKTTPPVLDSDGSFFLYSRLTVDKSRWQEGNVFSCSVLHEALHNHYTQKSLSLSLG

SEQ ID NO: 235 - protein, 227 aa, synthetic construct
KYGPPCPSCPAPEAAGGPSVFLFPPKPKDQLMISRTPEVTCVVVDVSQEDPEVQFNWYVDGVEVHNAKTKPREEQFNSTYRVVSVLTVLHQDWLNGKEYKCKVSNKGLPSSIEKTISKAKGQPREPQVYTLPPSQEEMTKNQVSLWCLVKGFYPSDIAVEWESNGQPENNYKTTPPVLDSDGSFFLYSRLTVDKSRWQEGNVFSCSVLHEALHNHYTQKSLSLSLGK

SEQ ID NO: 236 - protein, 226 aa, synthetic construct
KYGPPCPSCPAPEAAGGPSVFLFPPKPKDQLMISRTPEVTCVVVDVSQEDPEVQFNWYVDGVEVHNAKTKPREEQFNSTYRVVSVLTVLHQDWLNGKEYKCKVSNKGLPSSIEKTISKAKGQPREPQVYTLPPSQEEMTKNQVSLWCLVKGFYPSDIAVEWESNGQPENNYKTTPPVLDSDGSFFLYSRLTVDKSRWQEGNVFSCSVLHEALHNHYTQKSLSLSLG

SEQ ID NO: 237 - protein, 227 aa, synthetic construct
KYGPPCPSCPAPEFLGGPSVFLFPPKPKDTLMISRTPEVTCVVVDVSQEDPEVQFNWYVDGVEVHNAKTKPREEQFNSTYRVVSVLTVDHHDWLNGKEYKCKVSNKGLPSSIEKTISKAKGQPREPQVYTLPPSQEEMTKNQVSLWCLVKGFYPSDIAVEWESNGQPENNYKTTPPVLDSDGSFFLYSRLTVDKSRWQEGNVFSCSVMHEALHSHYTQKSLSLSLGK

SEQ ID NO: 238 - protein, 226 aa, synthetic construct
KYGPPCPSCPAPEFLGGPSVFLFPPKPKDTLMISRTPEVTCVVVDVSQEDPEVQFNWYVDGVEVHNAKTKPREEQFNSTYRVVSVLTVDHHDWLNGKEYKCKVSNKGLPSSIEKTISKAKGQPREPQVYTLPPSQEEMTKNQVSLWCLVKGFYPSDIAVEWESNGQPENNYKTTPPVLDSDGSFFLYSRLTVDKSRWQEGNVFSCSVMHEALHSHYTQKSLSLSLG

SEQ ID NO: 239 - protein, 227 aa, synthetic construct
KYGPPCPSCPAPESTRGPSVFLFPPKPKDTLMISRTPEVTCVVVDVSQEDPEVQFNWYVDGVEVHNAKTKPREEQFNSTYRVVSVLTVDHHDWLNGKEYKCKVSNKGLPSSIEKTISKAKGQPREPQVYTLPPSQEEMTKNQVSLWCLVKGFYPSDIAVEWESNGQPENNYKTTPPVLDSDGSFFLYSRLTVDKSRWQEGNVFSCSVMHEALHSHYTQKSLSLSLGK

SEQ ID NO: 240 - protein, 226 aa, synthetic construct
KYGPPCPSCPAPESTRGPSVFLFPPKPKDTLMISRTPEVTCVVVDVSQEDPEVQFNWYVDGVEVHNAKTKPREEQFNSTYRVVSVLTVDHHDWLNGKEYKCKVSNKGLPSSIEKTISKAKGQPREPQVYTLPPSQEEMTKNQVSLWCLVKGFYPSDIAVEWESNGQPENNYKTTPPVLDSDGSFFLYSRLTVDKSRWQEGNVFSCSVMHEALHSHYTQKSLSLSLG

SEQ ID NO: 241 - protein, 227 aa, synthetic construct
KYGPPCPSCPAPEAAGGPSVFLFPPKPKDTLMISRTPEVTCVVVDVSQEDPEVQFNWYVDGVEVHNAKTKPREEQFNSTYRVVSVLTVDHHDWLNGKEYKCKVSNKGLPSSIEKTISKAKGQPREPQVYTLPPSQEEMTKNQVSLWCLVKGFYPSDIAVEWESNGQPENNYKTTPPVLDSDGSFFLYSRLTVDKSRWQEGNVFSCSVMHEALHSHYTQKSLSLSLGK

SEQ ID NO: 242 - protein, 226 aa, synthetic construct
KYGPPCPSCPAPEAAGGPSVFLFPPKPKDTLMISRTPEVTCVVVDVSQEDPEVQFNWYVDGVEVHNAKTKPREEQFNSTYRVVSVLTVDHHDWLNGKEYKCKVSNKGLPSSIEKTISKAKGQPREPQVYTLPPSQEEMTKNQVSLWCLVKGFYPSDIAVEWESNGQPENNYKTTPPVLDSDGSFFLYSRLTVDKSRWQEGNVFSCSVMHEALHSHYTQKSLSLSLG

SEQ ID NO: 243 - protein, 330 aa, synthetic construct
ASTKGPSVFPLAPSSKSTSGGTAALGCLVKDYFPEPVTVSWNSGALTSGVHTFPAVLQSSGLYSLSSVVTVPSSSLGTQTYICNVNHKPSNTKVDKKVEPKSCDKTHTCPPCPAPELLGGPSVFLFPPKPKDTLMISRTPEVTCVVVDVSHEDPEVKFNWYVDGVEVHNAKTKPREEQYNSTYRVVSVLTVLHQDWLNGKEYKCKVSNKALPAPIEKTISKAKGQPREPQVYTLPPSREEMTKNQVSLSCAVKGFYPSDIAVEWESNGQPENNYKTTPPVLDSDGSFFLVSKLTVDKSRWQQGNVFSCSVMHEALHNHYTQKSLSLSPGK

SEQ ID NO: 244 - protein, 329 aa, synthetic construct
ASTKGPSVFPLAPSSKSTSGGTAALGCLVKDYFPEPVTVSWNSGALTSGVHTFPAVLQSSGLYSLSSVVTVPSSSLGTQTYICNVNHKPSNTKVDKKVEPKSCDKTHTCPPCPAPELLGGPSVFLFPPKPKDTLMISRTPEVTCVVVDVSHEDPEVKFNWYVDGVEVHNAKTKPREEQYNSTYRVVSVLTVLHQDWLNGKEYKCKVSNKALPAPIEKTISKAKGQPREPQVYTLPPSREEMTKNQVSLSCAVKGFYPSDIAVEWESNGQPENNYKTTPPVLDSDGSFFLVSKLTVDKSRWQQGNVFSCSVMHEALHNHYTQKSLSLSPG

SEQ ID NO: 245 - protein, 330 aa, synthetic construct
ASTKGPSVFPLAPSSKSTSGGTAALGCLVKDYFPEPVTVSWNSGALTSGVHTFPAVLQSSGLYSLSSVVTVPSSSLGTQTYICNVNHKPSNTKVDKKVEPKSCDKTHTCPPCPAPESTRGPSVFLFPPKPKDTLMISRTPEVTCVVVDVSHEDPEVKFNWYVDGVEVHNAKTKPREEQYNSTYRVVSVLTVLHQDWLNGKEYKCKVSNKALPAPIEKTISKAKGQPREPQVYTLPPSREEMTKNQVSLSCAVKGFYPSDIAVEWESNGQPENNYKTTPPVLDSDGSFFLVSKLTVDKSRWQQGNVFSCSVMHEALHNHYTQKSLSLSPGK

SEQ ID NO: 246 - protein, 329 aa, synthetic construct
ASTKGPSVFPLAPSSKSTSGGTAALGCLVKDYFPEPVTVSWNSGALTSGVHTFPAVLQSSGLYSLSSVVTVPSSSLGTQTYICNVNHKPSNTKVDKKVEPKSCDKTHTCPPCPAPESTRGPSVFLFPPKPKDTLMISRTPEVTCVVVDVSHEDPEVKFNWYVDGVEVHNAKTKPREEQYNSTYRVVSVLTVLHQDWLNGKEYKCKVSNKALPAPIEKTISKAKGQPREPQVYTLPPSREEMTKNQVSLSCAVKGFYPSDIAVEWESNGQPENNYKTTPPVLDSDGSFFLVSKLTVDKSRWQQGNVFSCSVMHEALHNHYTQKSLSLSPG

SEQ ID NO: 247 - protein, 330 aa, synthetic construct
ASTKGPSVFPLAPSSKSTSGGTAALGCLVKDYFPEPVTVSWNSGALTSGVHTFPAVLQSSGLYSLSSVVTVPSSSLGTQTYICNVNHKPSNTKVDKKVEPKSCDKTHTCPPCPAPEAAGGPSVFLFPPKPKDTLMISRTPEVTCVVVDVSHEDPEVKFNWYVDGVEVHNAKTKPREEQYNSTYRVVSVLTVLHQDWLNGKEYKCKVSNKALPAPIEKTISKAKGQPREPQVYTLPPSREEMTKNQVSLSCAVKGFYPSDIAVEWESNGQPENNYKTTPPVLDSDGSFFLVSKLTVDKSRWQQGNVFSCSVMHEALHNHYTQKSLSLSPGK

SEQ ID NO: 248 - protein, 329 aa, synthetic construct
ASTKGPSVFPLAPSSKSTSGGTAALGCLVKDYFPEPVTVSWNSGALTSGVHTFPAVLQSSGLYSLSSVVTVPSSSLGTQTYICNVNHKPSNTKVDKKVEPKSCDKTHTCPPCPAPEAAGGPSVFLFPPKPKDTLMISRTPEVTCVVVDVSHEDPEVKFNWYVDGVEVHNAKTKPREEQYNSTYRVVSVLTVLHQDWLNGKEYKCKVSNKALPAPIEKTISKAKGQPREPQVYTLPPSREEMTKNQVSLSCAVKGFYPSDIAVEWESNGQPENNYKTTPPVLDSDGSFFLVSKLTVDKSRWQQGNVFSCSVMHEALHNHYTQKSLSLSPG

SEQ ID NO: 249 - protein, 330 aa, synthetic construct
ASTKGPSVFPLAPSSKSTSGGTAALGCLVKDYFPEPVTVSWNSGALTSGVHTFPAVLQSSGLYSLSSVVTVPSSSLGTQTYICNVNHKPSNTKVDKKVEPKSCDKTHTCPPCPAPELLGGPSVFLFPPKPKDTLYITREPEVTCVVVDVSHEDPEVKFNWYVDGVEVHNAKTKPREEQYNSTYRVVSVLTVLHQDWLNGKEYKCKVSNKALPAPIEKTISKAKGQPREPQVYTLPPSREEMTKNQVSLSCAVKGFYPSDIAVEWESNGQPENNYKTTPPVLDSDGSFFLVSKLTVDKSRWQQGNVFSCSVMHEALHNHYTQKSLSLSPGK

SEQ ID NO: 250 - protein, 329 aa, synthetic construct
ASTKGPSVFPLAPSSKSTSGGTAALGCLVKDYFPEPVTVSWNSGALTSGVHTFPAVLQSSGLYSLSSVVTVPSSSLGTQTYICNVNHKPSNTKVDKKVEPKSCDKTHTCPPCPAPELLGGPSVFLFPPKPKDTLYITREPEVTCVVVDVSHEDPEVKFNWYVDGVEVHNAKTKPREEQYNSTYRVVSVLTVLHQDWLNGKEYKCKVSNKALPAPIEKTISKAKGQPREPQVYTLPPSREEMTKNQVSLSCAVKGFYPSDIAVEWESNGQPENNYKTTPPVLDSDGSFFLVSKLTVDKSRWQQGNVFSCSVMHEALHNHYTQKSLSLSPG

SEQ ID NO: 251 - protein, 330 aa, synthetic construct
ASTKGPSVFPLAPSSKSTSGGTAALGCLVKDYFPEPVTVSWNSGALTSGVHTFPAVLQSSGLYSLSSVVTVPSSSLGTQTYICNVNHKPSNTKVDKKVEPKSCDKTHTCPPCPAPESTRGPSVFLFPPKPKDTLYITREPEVTCVVVDVSHEDPEVKFNWYVDGVEVHNAKTKPREEQYNSTYRVVSVLTVLHQDWLNGKEYKCKVSNKALPAPIEKTISKAKGQPREPQVYTLPPSREEMTKNQVSLSCAVKGFYPSDIAVEWESNGQPENNYKTTPPVLDSDGSFFLVSKLTVDKSRWQQGNVFSCSVMHEALHNHYTQKSLSLSPGK

SEQ ID NO: 252 - protein, 329 aa, synthetic construct
ASTKGPSVFPLAPSSKSTSGGTAALGCLVKDYFPEPVTVSWNSGALTSGVHTFPAVLQSSGLYSLSSVVTVPSSSLGTQTYICNVNHKPSNTKVDKKVEPKSCDKTHTCPPCPAPESTRGPSVFLFPPKPKDTLYITREPEVTCVVVDVSHEDPEVKFNWYVDGVEVHNAKTKPREEQYNSTYRVVSVLTVLHQDWLNGKEYKCKVSNKALPAPIEKTISKAKGQPREPQVYTLPPSREEMTKNQVSLSCAVKGFYPSDIAVEWESNGQPENNYKTTPPVLDSDGSFFLVSKLTVDKSRWQQGNVFSCSVMHEALHNHYTQKSLSLSPG

SEQ ID NO: 253 - protein, 330 aa, synthetic construct
ASTKGPSVFPLAPSSKSTSGGTAALGCLVKDYFPEPVTVSWNSGALTSGVHTFPAVLQSSGLYSLSSVVTVPSSSLGTQTYICNVNHKPSNTKVDKKVEPKSCDKTHTCPPCPAPEAAGGPSVFLFPPKPKDTLYITREPEVTCVVVDVSHEDPEVKFNWYVDGVEVHNAKTKPREEQYNSTYRVVSVLTVLHQDWLNGKEYKCKVSNKALPAPIEKTISKAKGQPREPQVYTLPPSREEMTKNQVSLSCAVKGFYPSDIAVEWESNGQPENNYKTTPPVLDSDGSFFLVSKLTVDKSRWQQGNVFSCSVMHEALHNHYTQKSLSLSPGK

SEQ ID NO: 254 - protein, 329 aa, synthetic construct
ASTKGPSVFPLAPSSKSTSGGTAALGCLVKDYFPEPVTVSWNSGALTSGVHTFPAVLQSSGLYSLSSVVTVPSSSLGTQTYICNVNHKPSNTKVDKKVEPKSCDKTHTCPPCPAPEAAGGPSVFLFPPKPKDTLYITREPEVTCVVVDVSHEDPEVKFNWYVDGVEVHNAKTKPREEQYNSTYRVVSVLTVLHQDWLNGKEYKCKVSNKALPAPIEKTISKAKGQPREPQVYTLPPSREEMTKNQVSLSCAVKGFYPSDIAVEWESNGQPENNYKTTPPVLDSDGSFFLVSKLTVDKSRWQQGNVFSCSVMHEALHNHYTQKSLSLSPG

SEQ ID NO: 255 - protein, 330 aa, synthetic construct
ASTKGPSVFPLAPSSKSTSGGTAALGCLVKDYFPEPVTVSWNSGALTSGVHTFPAVLQSSGLYSLSSVVTVPSSSLGTQTYICNVNHKPSNTKVDKKVEPKSCDKTHTCPPCPAPELLGGPSVFLFPPKPKDTLMISRTPEVTCVVVDVSHEDPEVKFNWYVDGVEVHNAKTKPREEQYNSTYRVVSVLTVLHRDWLNGKEYKCKVSNKALPAPIEKTISKAKGQPREPQVYTLPPSREEMTKNQVSLSCAVKGFYPSDIAVEWESNGQPENNYKTTPPVLDSDGSFFLVSKLTVDKSRWQQGNVFSCSVEHEALHWHYTQKSLSLSPGK

SEQ ID NO: 256 - protein, 329 aa, synthetic construct
ASTKGPSVFPLAPSSKSTSGGTAALGCLVKDYFPEPVTVSWNSGALTSGVHTFPAVLQSSGLYSLSSVVTVPSSSLGTQTYICNVNHKPSNTKVDKKVEPKSCDKTHTCPPCPAPELLGGPSVFLFPPKPKDTLMISRTPEVTCVVVDVSHEDPEVKFNWYVDGVEVHNAKTKPREEQYNSTYRVVSVLTVLHRDWLNGKEYKCKVSNKALPAPIEKTISKAKGQPREPQVYTLPPSREEMTKNQVSLSCAVKGFYPSDIAVEWESNGQPENNYKTTPPVLDSDGSFFLVSKLTVDKSRWQQGNVFSCSVEHEALHWHYTQKSLSLSPG

SEQ ID NO: 257 - protein, 330 aa, synthetic construct
ASTKGPSVFPLAPSSKSTSGGTAALGCLVKDYFPEPVTVSWNSGALTSGVHTFPAVLQSSGLYSLSSVVTVPSSSLGTQTYICNVNHKPSNTKVDKKVEPKSCDKTHTCPPCPAPESTRGPSVFLFPPKPKDTLMISRTPEVTCVVVDVSHEDPEVKFNWYVDGVEVHNAKTKPREEQYNSTYRVVSVLTVLHRDWLNGKEYKCKVSNKALPAPIEKTISKAKGQPREPQVYTLPPSREEMTKNQVSLSCAVKGFYPSDIAVEWESNGQPENNYKTTPPVLDSDGSFFLVSKLTVDKSRWQQGNVFSCSVEHEALHWHYTQKSLSLSPGK

SEQ ID NO: 258 - protein, 329 aa, synthetic construct
ASTKGPSVFPLAPSSKSTSGGTAALGCLVKDYFPEPVTVSWNSGALTSGVHTFPAVLQSSGLYSLSSVVTVPSSSLGTQTYICNVNHKPSNTKVDKKVEPKSCDKTHTCPPCPAPESTRGPSVFLFPPKPKDTLMISRTPEVTCVVVDVSHEDPEVKFNWYVDGVEVHNAKTKPREEQYNSTYRVVSVLTVLHRDWLNGKEYKCKVSNKALPAPIEKTISKAKGQPREPQVYTLPPSREEMTKNQVSLSCAVKGFYPSDIAVEWESNGQPENNYKTTPPVLDSDGSFFLVSKLTVDKSRWQQGNVFSCSVEHEALHWHYTQKSLSLSPG

SEQ ID NO: 259 - protein, 330 aa, synthetic construct
ASTKGPSVFPLAPSSKSTSGGTAALGCLVKDYFPEPVTVSWNSGALTSGVHTFPAVLQSSGLYSLSSVVTVPSSSLGTQTYICNVNHKPSNTKVDKKVEPKSCDKTHTCPPCPAPEAAGGPSVFLFPPKPKDTLMISRTPEVTCVVVDVSHEDPEVKFNWYVDGVEVHNAKTKPREEQYNSTYRVVSVLTVLHRDWLNGKEYKCKVSNKALPAPIEKTISKAKGQPREPQVYTLPPSREEMTKNQVSLSCAVKGFYPSDIAVEWESNGQPENNYKTTPPVLDSDGSFFLVSKLTVDKSRWQQGNVFSCSVEHEALHWHYTQKSLSLSPGK

SEQ ID NO: 260 - protein, 329 aa, synthetic construct
ASTKGPSVFPLAPSSKSTSGGTAALGCLVKDYFPEPVTVSWNSGALTSGVHTFPAVLQSSGLYSLSSVVTVPSSSLGTQTYICNVNHKPSNTKVDKKVEPKSCDKTHTCPPCPAPEAAGGPSVFLFPPKPKDTLMISRTPEVTCVVVDVSHEDPEVKFNWYVDGVEVHNAKTKPREEQYNSTYRVVSVLTVLHRDWLNGKEYKCKVSNKALPAPIEKTISKAKGQPREPQVYTLPPSREEMTKNQVSLSCAVKGFYPSDIAVEWESNGQPENNYKTTPPVLDSDGSFFLVSKLTVDKSRWQQGNVFSCSVEHEALHWHYTQKSLSLSPG

SEQ ID NO: 261 - protein, 330 aa, synthetic construct
ASTKGPSVFPLAPSSKSTSGGTAALGCLVKDYFPEPVTVSWNSGALTSGVHTFPAVLQSSGLYSLSSVVTVPSSSLGTQTYICNVNHKPSNTKVDKKVEPKSCDKTHTCPPCPAPELLGGPSVFLFPPKPKDTLMISRTPEVTCVVVDVSHEDPEVKFNWYVDGVEVHNAKTKPREEQYNSTYRVVSVLTVLHQDWLNGKEYKCKVSNKALPAPIEKTISKAKGQPREPQVYTLPPSREEMTKNQVSLSCAVKGFYPSDIAVEWESNGQPENNYKTTPPVLDSDGSFFLVSKLTVDKSRWQQGNVFSCSVLHEALHSHYTQKSLSLSPGK

SEQ ID NO: 262 - protein, 329 aa, synthetic construct
ASTKGPSVFPLAPSSKSTSGGTAALGCLVKDYFPEPVTVSWNSGALTSGVHTFPAVLQSSGLYSLSSVVTVPSSSLGTQTYICNVNHKPSNTKVDKKVEPKSCDKTHTCPPCPAPELLGGPSVFLFPPKPKDTLMISRTPEVTCVVVDVSHEDPEVKFNWYVDGVEVHNAKTKPREEQYNSTYRVVSVLTVLHQDWLNGKEYKCKVSNKALPAPIEKTISKAKGQPREPQVYTLPPSREEMTKNQVSLSCAVKGFYPSDIAVEWESNGQPENNYKTTPPVLDSDGSFFLVSKLTVDKSRWQQGNVFSCSVLHEALHSHYTQKSLSLSPG

SEQ ID NO: 263 - protein, 330 aa, synthetic construct
ASTKGPSVFPLAPSSKSTSGGTAALGCLVKDYFPEPVTVSWNSGALTSGVHTFPAVLQSSGLYSLSSVVTVPSSSLGTQTYICNVNHKPSNTKVDKKVEPKSCDKTHTCPPCPAPESTRGPSVFLFPPKPKDTLMISRTPEVTCVVVDVSHEDPEVKFNWYVDGVEVHNAKTKPREEQYNSTYRVVSVLTVLHQDWLNGKEYKCKVSNKALPAPIEKTISKAKGQPREPQVYTLPPSREEMTKNQVSLSCAVKGFYPSDIAVEWESNGQPENNYKTTPPVLDSDGSFFLVSKLTVDKSRWQQGNVFSCSVLHEALHSHYTQKSLSLSPGK

SEQ ID NO: 264 - protein, 329 aa, synthetic construct
ASTKGPSVFPLAPSSKSTSGGTAALGCLVKDYFPEPVTVSWNSGALTSGVHTFPAVLQSSGLYSLSSVVTVPSSSLGTQTYICNVNHKPSNTKVDKKVEPKSCDKTHTCPPCPAPESTRGPSVFLFPPKPKDTLMISRTPEVTCVVVDVSHEDPEVKFNWYVDGVEVHNAKTKPREEQYNSTYRVVSVLTVLHQDWLNGKEYKCKVSNKALPAPIEKTISKAKGQPREPQVYTLPPSREEMTKNQVSLSCAVKGFYPSDIAVEWESNGQPENNYKTTPPVLDSDGSFFLVSKLTVDKSRWQQGNVFSCSVLHEALHSHYTQKSLSLSPG

SEQ ID NO: 265 - protein, 330 aa, synthetic construct
ASTKGPSVFPLAPSSKSTSGGTAALGCLVKDYFPEPVTVSWNSGALTSGVHTFPAVLQSSGLYSLSSVVTVPSSSLGTQTYICNVNHKPSNTKVDKKVEPKSCDKTHTCPPCPAPEAAGGPSVFLFPPKPKDTLMISRTPEVTCVVVDVSHEDPEVKFNWYVDGVEVHNAKTKPREEQYNSTYRVVSVLTVLHQDWLNGKEYKCKVSNKALPAPIEKTISKAKGQPREPQVYTLPPSREEMTKNQVSLSCAVKGFYPSDIAVEWESNGQPENNYKTTPPVLDSDGSFFLVSKLTVDKSRWQQGNVFSCSVLHEALHSHYTQKSLSLSPGK

SEQ ID NO: 266 - protein, 329 aa, synthetic construct
ASTKGPSVFPLAPSSKSTSGGTAALGCLVKDYFPEPVTVSWNSGALTSGVHTFPAVLQSSGLYSLSSVVTVPSSSLGTQTYICNVNHKPSNTKVDKKVEPKSCDKTHTCPPCPAPEAAGGPSVFLFPPKPKDTLMISRTPEVTCVVVDVSHEDPEVKFNWYVDGVEVHNAKTKPREEQYNSTYRVVSVLTVLHQDWLNGKEYKCKVSNKALPAPIEKTISKAKGQPREPQVYTLPPSREEMTKNQVSLSCAVKGFYPSDIAVEWESNGQPENNYKTTPPVLDSDGSFFLVSKLTVDKSRWQQGNVFSCSVLHEALHSHYTQKSLSLSPG

SEQ ID NO: 267 - protein, 330 aa, synthetic construct
ASTKGPSVFPLAPSSKSTSGGTAALGCLVKDYFPEPVTVSWNSGALTSGVHTFPAVLQSSGLYSLSSVVTVPSSSLGTQTYICNVNHKPSNTKVDKKVEPKSCDKTHTCPPCPAPELLGGPSVFLFPPKPKDQLMISRTPEVTCVVVDVSHEDPEVKFNWYVDGVEVHNAKTKPREEQYNSTYRVVSVLTVLHQDWLNGKEYKCKVSNKALPAPIEKTISKAKGQPREPQVYTLPPSREEMTKNQVSLSCAVKGFYPSDIAVEWESNGQPENNYKTTPPVLDSDGSFFLVSKLTVDKSRWQQGNVFSCSVLHEALHNHYTQKSLSLSPGK

SEQ ID NO: 268 - protein, 329 aa, synthetic construct
ASTKGPSVFPLAPSSKSTSGGTAALGCLVKDYFPEPVTVSWNSGALTSGVHTFPAVLQSSGLYSLSSVVTVPSSSLGTQTYICNVNHKPSNTKVDKKVEPKSCDKTHTCPPCPAPELLGGPSVFLFPPKPKDQLMISRTPEVTCVVVDVSHEDPEVKFNWYVDGVEVHNAKTKPREEQYNSTYRVVSVLTVLHQDWLNGKEYKCKVSNKALPAPIEKTISKAKGQPREPQVYTLPPSREEMTKNQVSLSCAVKGFYPSDIAVEWESNGQPENNYKTTPPVLDSDGSFFLVSKLTVDKSRWQQGNVFSCSVLHEALHNHYTQKSLSLSPG

SEQ ID NO: 269 - protein, 330 aa, synthetic construct
ASTKGPSVFPLAPSSKSTSGGTAALGCLVKDYFPEPVTVSWNSGALTSGVHTFPAVLQSSGLYSLSSVVTVPSSSLGTQTYICNVNHKPSNTKVDKKVEPKSCDKTHTCPPCPAPESTRGPSVFLFPPKPKDQLMISRTPEVTCVVVDVSHEDPEVKFNWYVDGVEVHNAKTKPREEQYNSTYRVVSVLTVLHQDWLNGKEYKCKVSNKALPAPIEKTISKAKGQPREPQVYTLPPSREEMTKNQVSLSCAVKGFYPSDIAVEWESNGQPENNYKTTPPVLDSDGSFFLVSKLTVDKSRWQQGNVFSCSVLHEALHNHYTQKSLSLSPGK

SEQ ID NO: 270 - protein, 329 aa, synthetic construct
ASTKGPSVFPLAPSSKSTSGGTAALGCLVKDYFPEPVTVSWNSGALTSGVHTFPAVLQSSGLYSLSSVVTVPSSSLGTQTYICNVNHKPSNTKVDKKVEPKSCDKTHTCPPCPAPESTRGPSVFLFPPKPKDQLMISRTPEVTCVVVDVSHEDPEVKFNWYVDGVEVHNAKTKPREEQYNSTYRVVSVLTVLHQDWLNGKEYKCKVSNKALPAPIEKTISKAKGQPREPQVYTLPPSREEMTKNQVSLSCAVKGFYPSDIAVEWESNGQPENNYKTTPPVLDSDGSFFLVSKLTVDKSRWQQGNVFSCSVLHEALHNHYTQKSLSLSPG

SEQ ID NO: 271 - protein, 330 aa, synthetic construct
ASTKGPSVFPLAPSSKSTSGGTAALGCLVKDYFPEPVTVSWNSGALTSGVHTFPAVLQSSGLYSLSSVVTVPSSSLGTQTYICNVNHKPSNTKVDKKVEPKSCDKTHTCPPCPAPEAAGGPSVFLFPPKPKDQLMISRTPEVTCVVVDVSHEDPEVKFNWYVDGVEVHNAKTKPREEQYNSTYRVVSVLTVLHQDWLNGKEYKCKVSNKALPAPIEKTISKAKGQPREPQVYTLPPSREEMTKNQVSLSCAVKGFYPSDIAVEWESNGQPENNYKTTPPVLDSDGSFFLVSKLTVDKSRWQQGNVFSCSVLHEALHNHYTQKSLSLSPGK

SEQ ID NO: 272 - protein, 329 aa, synthetic construct
ASTKGPSVFPLAPSSKSTSGGTAALGCLVKDYFPEPVTVSWNSGALTSGVHTFPAVLQSSGLYSLSSVVTVPSSSLGTQTYICNVNHKPSNTKVDKKVEPKSCDKTHTCPPCPAPEAAGGPSVFLFPPKPKDQLMISRTPEVTCVVVDVSHEDPEVKFNWYVDGVEVHNAKTKPREEQYNSTYRVVSVLTVLHQDWLNGKEYKCKVSNKALPAPIEKTISKAKGQPREPQVYTLPPSREEMTKNQVSLSCAVKGFYPSDIAVEWESNGQPENNYKTTPPVLDSDGSFFLVSKLTVDKSRWQQGNVFSCSVLHEALHNHYTQKSLSLSPG

SEQ ID NO: 273 - protein, 330 aa, synthetic construct
ASTKGPSVFPLAPSSKSTSGGTAALGCLVKDYFPEPVTVSWNSGALTSGVHTFPAVLQSSGLYSLSSVVTVPSSSLGTQTYICNVNHKPSNTKVDKKVEPKSCDKTHTCPPCPAPELLGGPSVFLFPPKPKDTLMISRTPEVTCVVVDVSHEDPEVKFNWYVDGVEVHNAKTKPREEQYNSTYRVVSVLTVDHHDWLNGKEYKCKVSNKALPAPIEKTISKAKGQPREPQVYTLPPSREEMTKNQVSLSCAVKGFYPSDIAVEWESNGQPENNYKTTPPVLDSDGSFFLVSKLTVDKSRWQQGNVFSCSVMHEALHSHYTQKSLSLSPGK

SEQ ID NO: 274 - protein, 329 aa, synthetic construct
ASTKGPSVFPLAPSSKSTSGGTAALGCLVKDYFPEPVTVSWNSGALTSGVHTFPAVLQSSGLYSLSSVVTVPSSSLGTQTYICNVNHKPSNTKVDKKVEPKSCDKTHTCPPCPAPELLGGPSVFLFPPKPKDTLMISRTPEVTCVVVDVSHEDPEVKFNWYVDGVEVHNAKTKPREEQYNSTYRVVSVLTVDHHDWLNGKEYKCKVSNKALPAPIEKTISKAKGQPREPQVYTLPPSREEMTKNQVSLSCAVKGFYPSDIAVEWESNGQPENNYKTTPPVLDSDGSFFLVSKLTVDKSRWQQGNVFSCSVMHEALHSHYTQKSLSLSPG

SEQ ID NO: 275 - protein, 330 aa, synthetic construct
ASTKGPSVFPLAPSSKSTSGGTAALGCLVKDYFPEPVTVSWNSGALTSGVHTFPAVLQSSGLYSLSSVVTVPSSSLGTQTYICNVNHKPSNTKVDKKVEPKSCDKTHTCPPCPAPESTRGPSVFLFPPKPKDTLMISRTPEVTCVVVDVSHEDPEVKFNWYVDGVEVHNAKTKPREEQYNSTYRVVSVLTVDHHDWLNGKEYKCKVSNKALPAPIEKTISKAKGQPREPQVYTLPPSREEMTKNQVSLSCAVKGFYPSDIAVEWESNGQPENNYKTTPPVLDSDGSFFLVSKLTVDKSRWQQGNVFSCSVMHEALHSHYTQKSLSLSPGK

SEQ ID NO: 276 - protein, 329 aa, synthetic construct
ASTKGPSVFPLAPSSKSTSGGTAALGCLVKDYFPEPVTVSWNSGALTSGVHTFPAVLQSSGLYSLSSVVTVPSSSLGTQTYICNVNHKPSNTKVDKKVEPKSCDKTHTCPPCPAPESTRGPSVFLFPPKPKDTLMISRTPEVTCVVVDVSHEDPEVKFNWYVDGVEVHNAKTKPREEQYNSTYRVVSVLTVDHHDWLNGKEYKCKVSNKALPAPIEKTISKAKGQPREPQVYTLPPSREEMTKNQVSLSCAVKGFYPSDIAVEWESNGQPENNYKTTPPVLDSDGSFFLVSKLTVDKSRWQQGNVFSCSVMHEALHSHYTQKSLSLSPG

SEQ ID NO: 277 - protein, 330 aa, synthetic construct
ASTKGPSVFPLAPSSKSTSGGTAALGCLVKDYFPEPVTVSWNSGALTSGVHTFPAVLQSSGLYSLSSVVTVPSSSLGTQTYICNVNHKPSNTKVDKKVEPKSCDKTHTCPPCPAPEAAGGPSVFLFPPKPKDTLMISRTPEVTCVVVDVSHEDPEVKFNWYVDGVEVHNAKTKPREEQYNSTYRVVSVLTVDHHDWLNGKEYKCKVSNKALPAPIEKTISKAKGQPREPQVYTLPPSREEMTKNQVSLSCAVKGFYPSDIAVEWESNGQPENNYKTTPPVLDSDGSFFLVSKLTVDKSRWQQGNVFSCSVMHEALHSHYTQKSLSLSPGK

SEQ ID NO: 278 - protein, 329 aa, synthetic construct
ASTKGPSVFPLAPSSKSTSGGTAALGCLVKDYFPEPVTVSWNSGALTSGVHTFPAVLQSSGLYSLSSVVTVPSSSLGTQTYICNVNHKPSNTKVDKKVEPKSCDKTHTCPPCPAPEAAGGPSVFLFPPKPKDTLMISRTPEVTCVVVDVSHEDPEVKFNWYVDGVEVHNAKTKPREEQYNSTYRVVSVLTVDHHDWLNGKEYKCKVSNKALPAPIEKTISKAKGQPREPQVYTLPPSREEMTKNQVSLSCAVKGFYPSDIAVEWESNGQPENNYKTTPPVLDSDGSFFLVSKLTVDKSRWQQGNVFSCSVMHEALHSHYTQKSLSLSPG

SEQ ID NO: 279 - protein, 327 aa, synthetic construct
ASTKGPSVFPLAPCSRSTSESTAALGCLVKDYFPEPVTVSWNSGALTSGVHTFPAVLQSSGLYSLSSVVTVPSSSLGTKTYTCNVDHKPSNTKVDKRVESKYGPPCPPCPAPEFLGGPSVFLFPPKPKDTLMISRTPEVTCVVVDVSQEDPEVQFNWYVDGVEVHNAKTKPREEQFNSTYRVVSVLTVLHQDWLNGKEYKCKVSNKGLPSSIEKTISKAKGQPREPQVYTLPPSQEEMTKNQVSLSCAVKGFYPSDIAVEWESNGQPENNYKTTPPVLDSDGSFFLVSRLTVDKSRWQEGNVFSCSVMHEALHNHYTQKSLSLSLGK

SEQ ID NO: 280 - protein, 326 aa, synthetic construct
ASTKGPSVFPLAPCSRSTSESTAALGCLVKDYFPEPVTVSWNSGALTSGVHTFPAVLQSSGLYSLSSVVTVPSSSLGTKTYTCNVDHKPSNTKVDKRVESKYGPPCPPCPAPEFLGGPSVFLFPPKPKDTLMISRTPEVTCVVVDVSQEDPEVQFNWYVDGVEVHNAKTKPREEQFNSTYRVVSVLTVLHQDWLNGKEYKCKVSNKGLPSSIEKTISKAKGQPREPQVYTLPPSQEEMTKNQVSLSCAVKGFYPSDIAVEWESNGQPENNYKTTPPVLDSDGSFFLVSRLTVDKSRWQEGNVFSCSVMHEALHNHYTQKSLSLSLG

SEQ ID NO: 281 - protein, 327 aa, synthetic construct
ASTKGPSVFPLAPCSRSTSESTAALGCLVKDYFPEPVTVSWNSGALTSGVHTFPAVLQSSGLYSLSSVVTVPSSSLGTKTYTCNVDHKPSNTKVDKRVESKYGPPCPPCPAPESTRGPSVFLFPPKPKDTLMISRTPEVTCVVVDVSQEDPEVQFNWYVDGVEVHNAKTKPREEQFNSTYRVVSVLTVLHQDWLNGKEYKCKVSNKGLPSSIEKTISKAKGQPREPQVYTLPPSQEEMTKNQVSLSCAVKGFYPSDIAVEWESNGQPENNYKTTPPVLDSDGSFFLVSRLTVDKSRWQEGNVFSCSVMHEALHNHYTQKSLSLSLGK

SEQ ID NO: 282 - protein, 326 aa, synthetic construct
ASTKGPSVFPLAPCSRSTSESTAALGCLVKDYFPEPVTVSWNSGALTSGVHTFPAVLQSSGLYSLSSVVTVPSSSLGTKTYTCNVDHKPSNTKVDKRVESKYGPPCPPCPAPESTRGPSVFLFPPKPKDTLMISRTPEVTCVVVDVSQEDPEVQFNWYVDGVEVHNAKTKPREEQFNSTYRVVSVLTVLHQDWLNGKEYKCKVSNKGLPSSIEKTISKAKGQPREPQVYTLPPSQEEMTKNQVSLSCAVKGFYPSDIAVEWESNGQPENNYKTTPPVLDSDGSFFLVSRLTVDKSRWQEGNVFSCSVMHEALHNHYTQKSLSLSLG

SEQ ID NO: 283 - protein, 327 aa, synthetic construct
ASTKGPSVFPLAPCSRSTSESTAALGCLVKDYFPEPVTVSWNSGALTSGVHTFPAVLQSSGLYSLSSVVTVPSSSLGTKTYTCNVDHKPSNTKVDKRVESKYGPPCPPCPAPEAAGGPSVFLFPPKPKDTLMISRTPEVTCVVVDVSQEDPEVQFNWYVDGVEVHNAKTKPREEQFNSTYRVVSVLTVLHQDWLNGKEYKCKVSNKGLPSSIEKTISKAKGQPREPQVYTLPPSQEEMTKNQVSLSCAVKGFYPSDIAVEWESNGQPENNYKTTPPVLDSDGSFFLVSRLTVDKSRWQEGNVFSCSVMHEALHNHYTQKSLSLSLGK

SEQ ID NO: 284 - protein, 326 aa, synthetic construct
ASTKGPSVFPLAPCSRSTSESTAALGCLVKDYFPEPVTVSWNSGALTSGVHTFPAVLQSSGLYSLSSVVTVPSSSLGTKTYTCNVDHKPSNTKVDKRVESKYGPPCPPCPAPEAAGGPSVFLFPPKPKDTLMISRTPEVTCVVVDVSQEDPEVQFNWYVDGVEVHNAKTKPREEQFNSTYRVVSVLTVLHQDWLNGKEYKCKVSNKGLPSSIEKTISKAKGQPREPQVYTLPPSQEEMTKNQVSLSCAVKGFYPSDIAVEWESNGQPENNYKTTPPVLDSDGSFFLVSRLTVDKSRWQEGNVFSCSVMHEALHNHYTQKSLSLSLG

SEQ ID NO: 285 - protein, 327 aa, synthetic construct
ASTKGPSVFPLAPCSRSTSESTAALGCLVKDYFPEPVTVSWNSGALTSGVHTFPAVLQSSGLYSLSSVVTVPSSSLGTKTYTCNVDHKPSNTKVDKRVESKYGPPCPPCPAPEFLGGPSVFLFPPKPKDTLYITREPEVTCVVVDVSQEDPEVQFNWYVDGVEVHNAKTKPREEQFNSTYRVVSVLTVLHQDWLNGKEYKCKVSNKGLPSSIEKTISKAKGQPREPQVYTLPPSQEEMTKNQVSLSCAVKGFYPSDIAVEWESNGQPENNYKTTPPVLDSDGSFFLVSRLTVDKSRWQEGNVFSCSVMHEALHNHYTQKSLSLSLGK

SEQ ID NO: 286 - protein, 326 aa, synthetic construct
ASTKGPSVFPLAPCSRSTSESTAALGCLVKDYFPEPVTVSWNSGALTSGVHTFPAVLQSSGLYSLSSVVTVPSSSLGTKTYTCNVDHKPSNTKVDKRVESKYGPPCPPCPAPEFLGGPSVFLFPPKPKDTLYITREPEVTCVVVDVSQEDPEVQFNWYVDGVEVHNAKTKPREEQFNSTYRVVSVLTVLHQDWLNGKEYKCKVSNKGLPSSIEKTISKAKGQPREPQVYTLPPSQEEMTKNQVSLSCAVKGFYPSDIAVEWESNGQPENNYKTTPPVLDSDGSFFLVSRLTVDKSRWQEGNVFSCSVMHEALHNHYTQKSLSLSLG

SEQ ID NO: 287 - protein, 327 aa, synthetic construct
ASTKGPSVFPLAPCSRSTSESTAALGCLVKDYFPEPVTVSWNSGALTSGVHTFPAVLQSSGLYSLSSVVTVPSSSLGTKTYTCNVDHKPSNTKVDKRVESKYGPPCPPCPAPESTRGPSVFLFPPKPKDTLYITREPEVTCVVVDVSQEDPEVQFNWYVDGVEVHNAKTKPREEQFNSTYRVVSVLTVLHQDWLNGKEYKCKVSNKGLPSSIEKTISKAKGQPREPQVYTLPPSQEEMTKNQVSLSCAVKGFYPSDIAVEWESNGQPENNYKTTPPVLDSDGSFFLVSRLTVDKSRWQEGNVFSCSVMHEALHNHYTQKSLSLSLGK

SEQ ID NO: 288 - protein, 326 aa, synthetic construct
ASTKGPSVFPLAPCSRSTSESTAALGCLVKDYFPEPVTVSWNSGALTSGVHTFPAVLQSSGLYSLSSVVTVPSSSLGTKTYTCNVDHKPSNTKVDKRVESKYGPPCPPCPAPESTRGPSVFLFPPKPKDTLYITREPEVTCVVVDVSQEDPEVQFNWYVDGVEVHNAKTKPREEQFNSTYRVVSVLTVLHQDWLNGKEYKCKVSNKGLPSSIEKTISKAKGQPREPQVYTLPPSQEEMTKNQVSLSCAVKGFYPSDIAVEWESNGQPENNYKTTPPVLDSDGSFFLVSRLTVDKSRWQEGNVFSCSVMHEALHNHYTQKSLSLSLG

SEQ ID NO: 289 - protein, 327 aa, synthetic construct
ASTKGPSVFPLAPCSRSTSESTAALGCLVKDYFPEPVTVSWNSGALTSGVHTFPAVLQSSGLYSLSSVVTVPSSSLGTKTYTCNVDHKPSNTKVDKRVESKYGPPCPPCPAPEAAGGPSVFLFPPKPKDTLYITREPEVTCVVVDVSQEDPEVQFNWYVDGVEVHNAKTKPREEQFNSTYRVVSVLTVLHQDWLNGKEYKCKVSNKGLPSSIEKTISKAKGQPREPQVYTLPPSQEEMTKNQVSLSCAVKGFYPSDIAVEWESNGQPENNYKTTPPVLDSDGSFFLVSRLTVDKSRWQEGNVFSCSVMHEALHNHYTQKSLSLSLGK

SEQ ID NO: 290 - protein, 326 aa, synthetic construct
ASTKGPSVFPLAPCSRSTSESTAALGCLVKDYFPEPVTVSWNSGALTSGVHTFPAVLQSSGLYSLSSVVTVPSSSLGTKTYTCNVDHKPSNTKVDKRVESKYGPPCPPCPAPEAAGGPSVFLFPPKPKDTLYITREPEVTCVVVDVSQEDPEVQFNWYVDGVEVHNAKTKPREEQFNSTYRVVSVLTVLHQDWLNGKEYKCKVSNKGLPSSIEKTISKAKGQPREPQVYTLPPSQEEMTKNQVSLSCAVKGFYPSDIAVEWESNGQPENNYKTTPPVLDSDGSFFLVSRLTVDKSRWQEGNVFSCSVMHEALHNHYTQKSLSLSLG

SEQ ID NO: 291 - protein, 327 aa, synthetic construct
ASTKGPSVFPLAPCSRSTSESTAALGCLVKDYFPEPVTVSWNSGALTSGVHTFPAVLQSSGLYSLSSVVTVPSSSLGTKTYTCNVDHKPSNTKVDKRVESKYGPPCPPCPAPEFLGGPSVFLFPPKPKDTLMISRTPEVTCVVVDVSQEDPEVQFNWYVDGVEVHNAKTKPREEQFNSTYRVVSVLTVLHRDWLNGKEYKCKVSNKGLPSSIEKTISKAKGQPREPQVYTLPPSQEEMTKNQVSLSCAVKGFYPSDIAVEWESNGQPENNYKTTPPVLDSDGSFFLVSRLTVDKSRWQEGNVFSCSVEHEALHWHYTQKSLSLSLGK

SEQ ID NO: 292 - protein, 326 aa, synthetic construct
ASTKGPSVFPLAPCSRSTSESTAALGCLVKDYFPEPVTVSWNSGALTSGVHTFPAVLQSSGLYSLSSVVTVPSSSLGTKTYTCNVDHKPSNTKVDKRVESKYGPPCPPCPAPEFLGGPSVFLFPPKPKDTLMISRTPEVTCVVVDVSQEDPEVQFNWYVDGVEVHNAKTKPREEQFNSTYRVVSVLTVLHRDWLNGKEYKCKVSNKGLPSSIEKTISKAKGQPREPQVYTLPPSQEEMTKNQVSLSCAVKGFYPSDIAVEWESNGQPENNYKTTPPVLDSDGSFFLVSRLTVDKSRWQEGNVFSCSVEHEALHWHYTQKSLSLSLG

SEQ ID NO: 293 - protein, 327 aa, synthetic construct
ASTKGPSVFPLAPCSRSTSESTAALGCLVKDYFPEPVTVSWNSGALTSGVHTFPAVLQSSGLYSLSSVVTVPSSSLGTKTYTCNVDHKPSNTKVDKRVESKYGPPCPPCPAPESTRGPSVFLFPPKPKDTLMISRTPEVTCVVVDVSQEDPEVQFNWYVDGVEVHNAKTKPREEQFNSTYRVVSVLTVLHRDWLNGKEYKCKVSNKGLPSSIEKTISKAKGQPREPQVYTLPPSQEEMTKNQVSLSCAVKGFYPSDIAVEWESNGQPENNYKTTPPVLDSDGSFFLVSRLTVDKSRWQEGNVFSCSVEHEALHWHYTQKSLSLSLGK

SEQ ID NO: 294 - protein, 326 aa, synthetic construct
ASTKGPSVFPLAPCSRSTSESTAALGCLVKDYFPEPVTVSWNSGALTSGVHTFPAVLQSSGLYSLSSVVTVPSSSLGTKTYTCNVDHKPSNTKVDKRVESKYGPPCPPCPAPESTRGPSVFLFPPKPKDTLMISRTPEVTCVVVDVSQEDPEVQFNWYVDGVEVHNAKTKPREEQFNSTYRVVSVLTVLHRDWLNGKEYKCKVSNKGLPSSIEKTISKAKGQPREPQVYTLPPSQEEMTKNQVSLSCAVKGFYPSDIAVEWESNGQPENNYKTTPPVLDSDGSFFLVSRLTVDKSRWQEGNVFSCSVEHEALHWHYTQKSLSLSLG

SEQ ID NO: 295 - protein, 327 aa, synthetic construct
ASTKGPSVFPLAPCSRSTSESTAALGCLVKDYFPEPVTVSWNSGALTSGVHTFPAVLQSSGLYSLSSVVTVPSSSLGTKTYTCNVDHKPSNTKVDKRVESKYGPPCPPCPAPEAAGGPSVFLFPPKPKDTLMISRTPEVTCVVVDVSQEDPEVQFNWYVDGVEVHNAKTKPREEQFNSTYRVVSVLTVLHRDWLNGKEYKCKVSNKGLPSSIEKTISKAKGQPREPQVYTLPPSQEEMTKNQVSLSCAVKGFYPSDIAVEWESNGQPENNYKTTPPVLDSDGSFFLVSRLTVDKSRWQEGNVFSCSVEHEALHWHYTQKSLSLSLGK

SEQ ID NO: 296 - protein, 326 aa, synthetic construct
ASTKGPSVFPLAPCSRSTSESTAALGCLVKDYFPEPVTVSWNSGALTSGVHTFPAVLQSSGLYSLSSVVTVPSSSLGTKTYTCNVDHKPSNTKVDKRVESKYGPPCPPCPAPEAAGGPSVFLFPPKPKDTLMISRTPEVTCVVVDVSQEDPEVQFNWYVDGVEVHNAKTKPREEQFNSTYRVVSVLTVLHRDWLNGKEYKCKVSNKGLPSSIEKTISKAKGQPREPQVYTLPPSQEEMTKNQVSLSCAVKGFYPSDIAVEWESNGQPENNYKTTPPVLDSDGSFFLVSRLTVDKSRWQEGNVFSCSVEHEALHWHYTQKSLSLSLG

SEQ ID NO: 297 - protein, 327 aa, synthetic construct
ASTKGPSVFPLAPCSRSTSESTAALGCLVKDYFPEPVTVSWNSGALTSGVHTFPAVLQSSGLYSLSSVVTVPSSSLGTKTYTCNVDHKPSNTKVDKRVESKYGPPCPPCPAPEFLGGPSVFLFPPKPKDTLMISRTPEVTCVVVDVSQEDPEVQFNWYVDGVEVHNAKTKPREEQFNSTYRVVSVLTVLHQDWLNGKEYKCKVSNKGLPSSIEKTISKAKGQPREPQVYTLPPSQEEMTKNQVSLSCAVKGFYPSDIAVEWESNGQPENNYKTTPPVLDSDGSFFLVSRLTVDKSRWQEGNVFSCSVLHEALHSHYTQKSLSLSLGK

SEQ ID NO: 298 - protein, 326 aa, synthetic construct
ASTKGPSVFPLAPCSRSTSESTAALGCLVKDYFPEPVTVSWNSGALTSGVHTFPAVLQSSGLYSLSSVVTVPSSSLGTKTYTCNVDHKPSNTKVDKRVESKYGPPCPPCPAPEFLGGPSVFLFPPKPKDTLMISRTPEVTCVVVDVSQEDPEVQFNWYVDGVEVHNAKTKPREEQFNSTYRVVSVLTVLHQDWLNGKEYKCKVSNKGLPSSIEKTISKAKGQPREPQVYTLPPSQEEMTKNQVSLSCAVKGFYPSDIAVEWESNGQPENNYKTTPPVLDSDGSFFLVSRLTVDKSRWQEGNVFSCSVLHEALHSHYTQKSLSLSLG

SEQ ID NO: 299 - protein, 327 aa, synthetic construct
ASTKGPSVFPLAPCSRSTSESTAALGCLVKDYFPEPVTVSWNSGALTSGVHTFPAVLQSSGLYSLSSVVTVPSSSLGTKTYTCNVDHKPSNTKVDKRVESKYGPPCPPCPAPESTRGPSVFLFPPKPKDTLMISRTPEVTCVVVDVSQEDPEVQFNWYVDGVEVHNAKTKPREEQFNSTYRVVSVLTVLHQDWLNGKEYKCKVSNKGLPSSIEKTISKAKGQPREPQVYTLPPSQEEMTKNQVSLSCAVKGFYPSDIAVEWESNGQPENNYKTTPPVLDSDGSFFLVSRLTVDKSRWQEGNVFSCSVLHEALHSHYTQKSLSLSLGK

SEQ ID NO: 300 - protein, 326 aa, synthetic construct
ASTKGPSVFPLAPCSRSTSESTAALGCLVKDYFPEPVTVSWNSGALTSGVHTFPAVLQSSGLYSLSSVVTVPSSSLGTKTYTCNVDHKPSNTKVDKRVESKYGPPCPPCPAPESTRGPSVFLFPPKPKDTLMISRTPEVTCVVVDVSQEDPEVQFNWYVDGVEVHNAKTKPREEQFNSTYRVVSVLTVLHQDWLNGKEYKCKVSNKGLPSSIEKTISKAKGQPREPQVYTLPPSQEEMTKNQVSLSCAVKGFYPSDIAVEWESNGQPENNYKTTPPVLDSDGSFFLVSRLTVDKSRWQEGNVFSCSVLHEALHSHYTQKSLSLSLG

SEQ ID NO: 301 - protein, 327 aa, synthetic construct
ASTKGPSVFPLAPCSRSTSESTAALGCLVKDYFPEPVTVSWNSGALTSGVHTFPAVLQSSGLYSLSSVVTVPSSSLGTKTYTCNVDHKPSNTKVDKRVESKYGPPCPPCPAPEAAGGPSVFLFPPKPKDTLMISRTPEVTCVVVDVSQEDPEVQFNWYVDGVEVHNAKTKPREEQFNSTYRVVSVLTVLHQDWLNGKEYKCKVSNKGLPSSIEKTISKAKGQPREPQVYTLPPSQEEMTKNQVSLSCAVKGFYPSDIAVEWESNGQPENNYKTTPPVLDSDGSFFLVSRLTVDKSRWQEGNVFSCSVLHEALHSHYTQKSLSLSLGK

SEQ ID NO: 302 - protein, 326 aa, synthetic construct
ASTKGPSVFPLAPCSRSTSESTAALGCLVKDYFPEPVTVSWNSGALTSGVHTFPAVLQSSGLYSLSSVVTVPSSSLGTKTYTCNVDHKPSNTKVDKRVESKYGPPCPPCPAPEAAGGPSVFLFPPKPKDTLMISRTPEVTCVVVDVSQEDPEVQFNWYVDGVEVHNAKTKPREEQFNSTYRVVSVLTVLHQDWLNGKEYKCKVSNKGLPSSIEKTISKAKGQPREPQVYTLPPSQEEMTKNQVSLSCAVKGFYPSDIAVEWESNGQPENNYKTTPPVLDSDGSFFLVSRLTVDKSRWQEGNVFSCSVLHEALHSHYTQKSLSLSLG

SEQ ID NO: 303 - protein, 327 aa, synthetic construct
ASTKGPSVFPLAPCSRSTSESTAALGCLVKDYFPEPVTVSWNSGALTSGVHTFPAVLQSSGLYSLSSVVTVPSSSLGTKTYTCNVDHKPSNTKVDKRVESKYGPPCPPCPAPEFLGGPSVFLFPPKPKDQLMISRTPEVTCVVVDVSQEDPEVQFNWYVDGVEVHNAKTKPREEQFNSTYRVVSVLTVLHQDWLNGKEYKCKVSNKGLPSSIEKTISKAKGQPREPQVYTLPPSQEEMTKNQVSLSCAVKGFYPSDIAVEWESNGQPENNYKTTPPVLDSDGSFFLVSRLTVDKSRWQEGNVFSCSVLHEALHNHYTQKSLSLSLGK

SEQ ID NO: 304 - protein, 326 aa, synthetic construct
ASTKGPSVFPLAPCSRSTSESTAALGCLVKDYFPEPVTVSWNSGALTSGVHTFPAVLQSSGLYSLSSVVTVPSSSLGTKTYTCNVDHKPSNTKVDKRVESKYGPPCPPCPAPEFLGGPSVFLFPPKPKDQLMISRTPEVTCVVVDVSQEDPEVQFNWYVDGVEVHNAKTKPREEQFNSTYRVVSVLTVLHQDWLNGKEYKCKVSNKGLPSSIEKTISKAKGQPREPQVYTLPPSQEEMTKNQVSLSCAVKGFYPSDIAVEWESNGQPENNYKTTPPVLDSDGSFFLVSRLTVDKSRWQEGNVFSCSVLHEALHNHYTQKSLSLSLG

SEQ ID NO: 305 - protein, 327 aa, synthetic construct
ASTKGPSVFPLAPCSRSTSESTAALGCLVKDYFPEPVTVSWNSGALTSGVHTFPAVLQSSGLYSLSSVVTVPSSSLGTKTYTCNVDHKPSNTKVDKRVESKYGPPCPPCPAPESTRGPSVFLFPPKPKDQLMISRTPEVTCVVVDVSQEDPEVQFNWYVDGVEVHNAKTKPREEQFNSTYRVVSVLTVLHQDWLNGKEYKCKVSNKGLPSSIEKTISKAKGQPREPQVYTLPPSQEEMTKNQVSLSCAVKGFYPSDIAVEWESNGQPENNYKTTPPVLDSDGSFFLVSRLTVDKSRWQEGNVFSCSVLHEALHNHYTQKSLSLSLGK

SEQ ID NO: 306 - protein, 326 aa, synthetic construct
ASTKGPSVFPLAPCSRSTSESTAALGCLVKDYFPEPVTVSWNSGALTSGVHTFPAVLQSSGLYSLSSVVTVPSSSLGTKTYTCNVDHKPSNTKVDKRVESKYGPPCPPCPAPESTRGPSVFLFPPKPKDQLMISRTPEVTCVVVDVSQEDPEVQFNWYVDGVEVHNAKTKPREEQFNSTYRVVSVLTVLHQDWLNGKEYKCKVSNKGLPSSIEKTISKAKGQPREPQVYTLPPSQEEMTKNQVSLSCAVKGFYPSDIAVEWESNGQPENNYKTTPPVLDSDGSFFLVSRLTVDKSRWQEGNVFSCSVLHEALHNHYTQKSLSLSLG

SEQ ID NO: 307 - protein, 327 aa, synthetic construct
ASTKGPSVFPLAPCSRSTSESTAALGCLVKDYFPEPVTVSWNSGALTSGVHTFPAVLQSSGLYSLSSVVTVPSSSLGTKTYTCNVDHKPSNTKVDKRVESKYGPPCPPCPAPEAAGGPSVFLFPPKPKDQLMISRTPEVTCVVVDVSQEDPEVQFNWYVDGVEVHNAKTKPREEQFNSTYRVVSVLTVLHQDWLNGKEYKCKVSNKGLPSSIEKTISKAKGQPREPQVYTLPPSQEEMTKNQVSLSCAVKGFYPSDIAVEWESNGQPENNYKTTPPVLDSDGSFFLVSRLTVDKSRWQEGNVFSCSVLHEALHNHYTQKSLSLSLGK

SEQ ID NO: 308 - protein, 326 aa, synthetic construct
ASTKGPSVFPLAPCSRSTSESTAALGCLVKDYFPEPVTVSWNSGALTSGVHTFPAVLQSSGLYSLSSVVTVPSSSLGTKTYTCNVDHKPSNTKVDKRVESKYGPPCPPCPAPEAAGGPSVFLFPPKPKDQLMISRTPEVTCVVVDVSQEDPEVQFNWYVDGVEVHNAKTKPREEQFNSTYRVVSVLTVLHQDWLNGKEYKCKVSNKGLPSSIEKTISKAKGQPREPQVYTLPPSQEEMTKNQVSLSCAVKGFYPSDIAVEWESNGQPENNYKTTPPVLDSDGSFFLVSRLTVDKSRWQEGNVFSCSVLHEALHNHYTQKSLSLSLG

SEQ ID NO: 309 - protein, 327 aa, synthetic construct
ASTKGPSVFPLAPCSRSTSESTAALGCLVKDYFPEPVTVSWNSGALTSGVHTFPAVLQSSGLYSLSSVVTVPSSSLGTKTYTCNVDHKPSNTKVDKRVESKYGPPCPPCPAPEFLGGPSVFLFPPKPKDTLMISRTPEVTCVVVDVSQEDPEVQFNWYVDGVEVHNAKTKPREEQFNSTYRVVSVLTVDHHDWLNGKEYKCKVSNKGLPSSIEKTISKAKGQPREPQVYTLPPSQEEMTKNQVSLSCAVKGFYPSDIAVEWESNGQPENNYKTTPPVLDSDGSFFLVSRLTVDKSRWQEGNVFSCSVMHEALHSHYTQKSLSLSLGK

SEQ ID NO: 310 - protein, 326 aa, synthetic construct
ASTKGPSVFPLAPCSRSTSESTAALGCLVKDYFPEPVTVSWNSGALTSGVHTFPAVLQSSGLYSLSSVVTVPSSSLGTKTYTCNVDHKPSNTKVDKRVESKYGPPCPPCPAPEFLGGPSVFLFPPKPKDTLMISRTPEVTCVVVDVSQEDPEVQFNWYVDGVEVHNAKTKPREEQFNSTYRVVSVLTVDHHDWLNGKEYKCKVSNKGLPSSIEKTISKAKGQPREPQVYTLPPSQEEMTKNQVSLSCAVKGFYPSDIAVEWESNGQPENNYKTTPPVLDSDGSFFLVSRLTVDKSRWQEGNVFSCSVMHEALHSHYTQKSLSLSLG

SEQ ID NO: 311 - protein, 327 aa, synthetic construct
ASTKGPSVFPLAPCSRSTSESTAALGCLVKDYFPEPVTVSWNSGALTSGVHTFPAVLQSSGLYSLSSVVTVPSSSLGTKTYTCNVDHKPSNTKVDKRVESKYGPPCPPCPAPESTRGPSVFLFPPKPKDTLMISRTPEVTCVVVDVSQEDPEVQFNWYVDGVEVHNAKTKPREEQFNSTYRVVSVLTVDHHDWLNGKEYKCKVSNKGLPSSIEKTISKAKGQPREPQVYTLPPSQEEMTKNQVSLSCAVKGFYPSDIAVEWESNGQPENNYKTTPPVLDSDGSFFLVSRLTVDKSRWQEGNVFSCSVMHEALHSHYTQKSLSLSLGK

SEQ ID NO: 312 - protein, 326 aa, synthetic construct
ASTKGPSVFPLAPCSRSTSESTAALGCLVKDYFPEPVTVSWNSGALTSGVHTFPAVLQSSGLYSLSSVVTVPSSSLGTKTYTCNVDHKPSNTKVDKRVESKYGPPCPPCPAPESTRGPSVFLFPPKPKDTLMISRTPEVTCVVVDVSQEDPEVQFNWYVDGVEVHNAKTKPREEQFNSTYRVVSVLTVDHHDWLNGKEYKCKVSNKGLPSSIEKTISKAKGQPREPQVYTLPPSQEEMTKNQVSLSCAVKGFYPSDIAVEWESNGQPENNYKTTPPVLDSDGSFFLVSRLTVDKSRWQEGNVFSCSVMHEALHSHYTQKSLSLSLG

SEQ ID NO: 313 - protein, 327 aa, synthetic construct
ASTKGPSVFPLAPCSRSTSESTAALGCLVKDYFPEPVTVSWNSGALTSGVHTFPAVLQSSGLYSLSSVVTVPSSSLGTKTYTCNVDHKPSNTKVDKRVESKYGPPCPPCPAPEAAGGPSVFLFPPKPKDTLMISRTPEVTCVVVDVSQEDPEVQFNWYVDGVEVHNAKTKPREEQFNSTYRVVSVLTVDHHDWLNGKEYKCKVSNKGLPSSIEKTISKAKGQPREPQVYTLPPSQEEMTKNQVSLSCAVKGFYPSDIAVEWESNGQPENNYKTTPPVLDSDGSFFLVSRLTVDKSRWQEGNVFSCSVMHEALHSHYTQKSLSLSLGK

SEQ ID NO: 314 - protein, 326 aa, synthetic construct
ASTKGPSVFPLAPCSRSTSESTAALGCLVKDYFPEPVTVSWNSGALTSGVHTFPAVLQSSGLYSLSSVVTVPSSSLGTKTYTCNVDHKPSNTKVDKRVESKYGPPCPPCPAPEAAGGPSVFLFPPKPKDTLMISRTPEVTCVVVDVSQEDPEVQFNWYVDGVEVHNAKTKPREEQFNSTYRVVSVLTVDHHDWLNGKEYKCKVSNKGLPSSIEKTISKAKGQPREPQVYTLPPSQEEMTKNQVSLSCAVKGFYPSDIAVEWESNGQPENNYKTTPPVLDSDGSFFLVSRLTVDKSRWQEGNVFSCSVMHEALHSHYTQKSLSLSLG

SEQ ID NO: 315 - protein, 327 aa, synthetic construct
ASTKGPSVFPLAPCSRSTSESTAALGCLVKDYFPEPVTVSWNSGALTSGVHTFPAVLQSSGLYSLSSVVTVPSSSLGTKTYTCNVDHKPSNTKVDKRVESKYGPPCPSCPAPEFLGGPSVFLFPPKPKDTLMISRTPEVTCVVVDVSQEDPEVQFNWYVDGVEVHNAKTKPREEQFNSTYRVVSVLTVLHQDWLNGKEYKCKVSNKGLPSSIEKTISKAKGQPREPQVYTLPPSQEEMTKNQVSLSCAVKGFYPSDIAVEWESNGQPENNYKTTPPVLDSDGSFFLVSRLTVDKSRWQEGNVFSCSVMHEALHNHYTQKSLSLSLGK

SEQ ID NO: 316 - protein, 326 aa, synthetic construct
ASTKGPSVFPLAPCSRSTSESTAALGCLVKDYFPEPVTVSWNSGALTSGVHTFPAVLQSSGLYSLSSVVTVPSSSLGTKTYTCNVDHKPSNTKVDKRVESKYGPPCPSCPAPEFLGGPSVFLFPPKPKDTLMISRTPEVTCVVVDVSQEDPEVQFNWYVDGVEVHNAKTKPREEQFNSTYRVVSVLTVLHQDWLNGKEYKCKVSNKGLPSSIEKTISKAKGQPREPQVYTLPPSQEEMTKNQVSLSCAVKGFYPSDIAVEWESNGQPENNYKTTPPVLDSDGSFFLVSRLTVDKSRWQEGNVFSCSVMHEALHNHYTQKSLSLSLG

SEQ ID NO: 317 - protein, 327 aa, synthetic construct
ASTKGPSVFPLAPCSRSTSESTAALGCLVKDYFPEPVTVSWNSGALTSGVHTFPAVLQSSGLYSLSSVVTVPSSSLGTKTYTCNVDHKPSNTKVDKRVESKYGPPCPSCPAPESTRGPSVFLFPPKPKDTLMISRTPEVTCVVVDVSQEDPEVQFNWYVDGVEVHNAKTKPREEQFNSTYRVVSVLTVLHQDWLNGKEYKCKVSNKGLPSSIEKTISKAKGQPREPQVYTLPPSQEEMTKNQVSLSCAVKGFYPSDIAVEWESNGQPENNYKTTPPVLDSDGSFFLVSRLTVDKSRWQEGNVFSCSVMHEALHNHYTQKSLSLSLGK

SEQ ID NO: 318 - protein, 326 aa, synthetic construct
ASTKGPSVFPLAPCSRSTSESTAALGCLVKDYFPEPVTVSWNSGALTSGVHTFPAVLQSSGLYSLSSVVTVPSSSLGTKTYTCNVDHKPSNTKVDKRVESKYGPPCPSCPAPESTRGPSVFLFPPKPKDTLMISRTPEVTCVVVDVSQEDPEVQFNWYVDGVEVHNAKTKPREEQFNSTYRVVSVLTVLHQDWLNGKEYKCKVSNKGLPSSIEKTISKAKGQPREPQVYTLPPSQEEMTKNQVSLSCAVKGFYPSDIAVEWESNGQPENNYKTTPPVLDSDGSFFLVSRLTVDKSRWQEGNVFSCSVMHEALHNHYTQKSLSLSLG

SEQ ID NO: 319 - protein, 327 aa, synthetic construct
ASTKGPSVFPLAPCSRSTSESTAALGCLVKDYFPEPVTVSWNSGALTSGVHTFPAVLQSSGLYSLSSVVTVPSSSLGTKTYTCNVDHKPSNTKVDKRVESKYGPPCPSCPAPEAAGGPSVFLFPPKPKDTLMISRTPEVTCVVVDVSQEDPEVQFNWYVDGVEVHNAKTKPREEQFNSTYRVVSVLTVLHQDWLNGKEYKCKVSNKGLPSSIEKTISKAKGQPREPQVYTLPPSQEEMTKNQVSLSCAVKGFYPSDIAVEWESNGQPENNYKTTPPVLDSDGSFFLVSRLTVDKSRWQEGNVFSCSVMHEALHNHYTQKSLSLSLGK

SEQ ID NO: 320 - protein, 326 aa, synthetic construct
ASTKGPSVFPLAPCSRSTSESTAALGCLVKDYFPEPVTVSWNSGALTSGVHTFPAVLQSSGLYSLSSVVTVPSSSLGTKTYTCNVDHKPSNTKVDKRVESKYGPPCPSCPAPEAAGGPSVFLFPPKPKDTLMISRTPEVTCVVVDVSQEDPEVQFNWYVDGVEVHNAKTKPREEQFNSTYRVVSVLTVLHQDWLNGKEYKCKVSNKGLPSSIEKTISKAKGQPREPQVYTLPPSQEEMTKNQVSLSCAVKGFYPSDIAVEWESNGQPENNYKTTPPVLDSDGSFFLVSRLTVDKSRWQEGNVFSCSVMHEALHNHYTQKSLSLSLG

SEQ ID NO: 321 - protein, 327 aa, synthetic construct
ASTKGPSVFPLAPCSRSTSESTAALGCLVKDYFPEPVTVSWNSGALTSGVHTFPAVLQSSGLYSLSSVVTVPSSSLGTKTYTCNVDHKPSNTKVDKRVESKYGPPCPSCPAPEFLGGPSVFLFPPKPKDTLYITREPEVTCVVVDVSQEDPEVQFNWYVDGVEVHNAKTKPREEQFNSTYRVVSVLTVLHQDWLNGKEYKCKVSNKGLPSSIEKTISKAKGQPREPQVYTLPPSQEEMTKNQVSLSCAVKGFYPSDIAVEWESNGQPENNYKTTPPVLDSDGSFFLVSRLTVDKSRWQEGNVFSCSVMHEALHNHYTQKSLSLSLGK

SEQ ID NO: 322 - protein, 326 aa, synthetic construct
ASTKGPSVFPLAPCSRSTSESTAALGCLVKDYFPEPVTVSWNSGALTSGVHTFPAVLQSSGLYSLSSVVTVPSSSLGTKTYTCNVDHKPSNTKVDKRVESKYGPPCPSCPAPEFLGGPSVFLFPPKPKDTLYITREPEVTCVVVDVSQEDPEVQFNWYVDGVEVHNAKTKPREEQFNSTYRVVSVLTVLHQDWLNGKEYKCKVSNKGLPSSIEKTISKAKGQPREPQVYTLPPSQEEMTKNQVSLSCAVKGFYPSDIAVEWESNGQPENNYKTTPPVLDSDGSFFLVSRLTVDKSRWQEGNVFSCSVMHEALHNHYTQKSLSLSLG

SEQ ID NO: 323 - protein, 327 aa, synthetic construct
ASTKGPSVFPLAPCSRSTSESTAALGCLVKDYFPEPVTVSWNSGALTSGVHTFPAVLQSSGLYSLSSVVTVPSSSLGTKTYTCNVDHKPSNTKVDKRVESKYGPPCPSCPAPESTRGPSVFLFPPKPKDTLYITREPEVTCVVVDVSQEDPEVQFNWYVDGVEVHNAKTKPREEQFNSTYRVVSVLTVLHQDWLNGKEYKCKVSNKGLPSSIEKTISKAKGQPREPQVYTLPPSQEEMTKNQVSLSCAVKGFYPSDIAVEWESNGQPENNYKTTPPVLDSDGSFFLVSRLTVDKSRWQEGNVFSCSVMHEALHNHYTQKSLSLSLGK

SEQ ID NO: 324 - protein, 326 aa, synthetic construct
ASTKGPSVFPLAPCSRSTSESTAALGCLVKDYFPEPVTVSWNSGALTSGVHTFPAVLQSSGLYSLSSVVTVPSSSLGTKTYTCNVDHKPSNTKVDKRVESKYGPPCPSCPAPESTRGPSVFLFPPKPKDTLYITREPEVTCVVVDVSQEDPEVQFNWYVDGVEVHNAKTKPREEQFNSTYRVVSVLTVLHQDWLNGKEYKCKVSNKGLPSSIEKTISKAKGQPREPQVYTLPPSQEEMTKNQVSLSCAVKGFYPSDIAVEWESNGQPENNYKTTPPVLDSDGSFFLVSRLTVDKSRWQEGNVFSCSVMHEALHNHYTQKSLSLSLG

SEQ ID NO: 325 - protein, 327 aa, synthetic construct
ASTKGPSVFPLAPCSRSTSESTAALGCLVKDYFPEPVTVSWNSGALTSGVHTFPAVLQSSGLYSLSSVVTVPSSSLGTKTYTCNVDHKPSNTKVDKRVESKYGPPCPSCPAPEAAGGPSVFLFPPKPKDTLYITREPEVTCVVVDVSQEDPEVQFNWYVDGVEVHNAKTKPREEQFNSTYRVVSVLTVLHQDWLNGKEYKCKVSNKGLPSSIEKTISKAKGQPREPQVYTLPPSQEEMTKNQVSLSCAVKGFYPSDIAVEWESNGQPENNYKTTPPVLDSDGSFFLVSRLTVDKSRWQEGNVFSCSVMHEALHNHYTQKSLSLSLGK

SEQ ID NO: 326 - protein, 326 aa, synthetic construct
ASTKGPSVFPLAPCSRSTSESTAALGCLVKDYFPEPVTVSWNSGALTSGVHTFPAVLQSSGLYSLSSVVTVPSSSLGTKTYTCNVDHKPSNTKVDKRVESKYGPPCPSCPAPEAAGGPSVFLFPPKPKDTLYITREPEVTCVVVDVSQEDPEVQFNWYVDGVEVHNAKTKPREEQFNSTYRVVSVLTVLHQDWLNGKEYKCKVSNKGLPSSIEKTISKAKGQPREPQVYTLPPSQEEMTKNQVSLSCAVKGFYPSDIAVEWESNGQPENNYKTTPPVLDSDGSFFLVSRLTVDKSRWQEGNVFSCSVMHEALHNHYTQKSLSLSLG

SEQ ID NO: 327 - protein, 327 aa, synthetic construct
ASTKGPSVFPLAPCSRSTSESTAALGCLVKDYFPEPVTVSWNSGALTSGVHTFPAVLQSSGLYSLSSVVTVPSSSLGTKTYTCNVDHKPSNTKVDKRVESKYGPPCPSCPAPEFLGGPSVFLFPPKPKDTLMISRTPEVTCVVVDVSQEDPEVQFNWYVDGVEVHNAKTKPREEQFNSTYRVVSVLTVLHRDWLNGKEYKCKVSNKGLPSSIEKTISKAKGQPREPQVYTLPPSQEEMTKNQVSLSCAVKGFYPSDIAVEWESNGQPENNYKTTPPVLDSDGSFFLVSRLTVDKSRWQEGNVFSCSVEHEALHWHYTQKSLSLSLGK

SEQ ID NO: 328 - protein, 326 aa, synthetic construct
ASTKGPSVFPLAPCSRSTSESTAALGCLVKDYFPEPVTVSWNSGALTSGVHTFPAVLQSSGLYSLSSVVTVPSSSLGTKTYTCNVDHKPSNTKVDKRVESKYGPPCPSCPAPEFLGGPSVFLFPPKPKDTLMISRTPEVTCVVVDVSQEDPEVQFNWYVDGVEVHNAKTKPREEQFNSTYRVVSVLTVLHRDWLNGKEYKCKVSNKGLPSSIEKTISKAKGQPREPQVYTLPPSQEEMTKNQVSLSCAVKGFYPSDIAVEWESNGQPENNYKTTPPVLDSDGSFFLVSRLTVDKSRWQEGNVFSCSVEHEALHWHYTQKSLSLSLG

SEQ ID NO: 329 - protein, 327 aa, synthetic construct
ASTKGPSVFPLAPCSRSTSESTAALGCLVKDYFPEPVTVSWNSGALTSGVHTFPAVLQSSGLYSLSSVVTVPSSSLGTKTYTCNVDHKPSNTKVDKRVESKYGPPCPSCPAPESTRGPSVFLFPPKPKDTLMISRTPEVTCVVVDVSQEDPEVQFNWYVDGVEVHNAKTKPREEQFNSTYRVVSVLTVLHRDWLNGKEYKCKVSNKGLPSSIEKTISKAKGQPREPQVYTLPPSQEEMTKNQVSLSCAVKGFYPSDIAVEWESNGQPENNYKTTPPVLDSDGSFFLVSRLTVDKSRWQEGNVFSCSVEHEALHWHYTQKSLSLSLGK

SEQ ID NO: 330 - protein, 326 aa, synthetic construct
ASTKGPSVFPLAPCSRSTSESTAALGCLVKDYFPEPVTVSWNSGALTSGVHTFPAVLQSSGLYSLSSVVTVPSSSLGTKTYTCNVDHKPSNTKVDKRVESKYGPPCPSCPAPESTRGPSVFLFPPKPKDTLMISRTPEVTCVVVDVSQEDPEVQFNWYVDGVEVHNAKTKPREEQFNSTYRVVSVLTVLHRDWLNGKEYKCKVSNKGLPSSIEKTISKAKGQPREPQVYTLPPSQEEMTKNQVSLSCAVKGFYPSDIAVEWESNGQPENNYKTTPPVLDSDGSFFLVSRLTVDKSRWQEGNVFSCSVEHEALHWHYTQKSLSLSLG

SEQ ID NO: 331 - protein, 327 aa, synthetic construct
ASTKGPSVFPLAPCSRSTSESTAALGCLVKDYFPEPVTVSWNSGALTSGVHTFPAVLQSSGLYSLSSVVTVPSSSLGTKTYTCNVDHKPSNTKVDKRVESKYGPPCPSCPAPEAAGGPSVFLFPPKPKDTLMISRTPEVTCVVVDVSQEDPEVQFNWYVDGVEVHNAKTKPREEQFNSTYRVVSVLTVLHRDWLNGKEYKCKVSNKGLPSSIEKTISKAKGQPREPQVYTLPPSQEEMTKNQVSLSCAVKGFYPSDIAVEWESNGQPENNYKTTPPVLDSDGSFFLVSRLTVDKSRWQEGNVFSCSVEHEALHWHYTQKSLSLSLGK

SEQ ID NO: 332 - protein, 326 aa, synthetic construct
ASTKGPSVFPLAPCSRSTSESTAALGCLVKDYFPEPVTVSWNSGALTSGVHTFPAVLQSSGLYSLSSVVTVPSSSLGTKTYTCNVDHKPSNTKVDKRVESKYGPPCPSCPAPEAAGGPSVFLFPPKPKDTLMISRTPEVTCVVVDVSQEDPEVQFNWYVDGVEVHNAKTKPREEQFNSTYRVVSVLTVLHRDWLNGKEYKCKVSNKGLPSSIEKTISKAKGQPREPQVYTLPPSQEEMTKNQVSLSCAVKGFYPSDIAVEWESNGQPENNYKTTPPVLDSDGSFFLVSRLTVDKSRWQEGNVFSCSVEHEALHWHYTQKSLSLSLG

SEQ ID NO: 333 - protein, 327 aa, synthetic construct
ASTKGPSVFPLAPCSRSTSESTAALGCLVKDYFPEPVTVSWNSGALTSGVHTFPAVLQSSGLYSLSSVVTVPSSSLGTKTYTCNVDHKPSNTKVDKRVESKYGPPCPSCPAPEFLGGPSVFLFPPKPKDTLMISRTPEVTCVVVDVSQEDPEVQFNWYVDGVEVHNAKTKPREEQFNSTYRVVSVLTVLHQDWLNGKEYKCKVSNKGLPSSIEKTISKAKGQPREPQVYTLPPSQEEMTKNQVSLSCAVKGFYPSDIAVEWESNGQPENNYKTTPPVLDSDGSFFLVSRLTVDKSRWQEGNVFSCSVLHEALHSHYTQKSLSLSLGK

SEQ ID NO: 334 - protein, 326 aa, synthetic construct
ASTKGPSVFPLAPCSRSTSESTAALGCLVKDYFPEPVTVSWNSGALTSGVHTFPAVLQSSGLYSLSSVVTVPSSSLGTKTYTCNVDHKPSNTKVDKRVESKYGPPCPSCPAPEFLGGPSVFLFPPKPKDTLMISRTPEVTCVVVDVSQEDPEVQFNWYVDGVEVHNAKTKPREEQFNSTYRVVSVLTVLHQDWLNGKEYKCKVSNKGLPSSIEKTISKAKGQPREPQVYTLPPSQEEMTKNQVSLSCAVKGFYPSDIAVEWESNGQPENNYKTTPPVLDSDGSFFLVSRLTVDKSRWQEGNVFSCSVLHEALHSHYTQKSLSLSLG

SEQ ID NO: 335 - protein, 327 aa, synthetic construct
ASTKGPSVFPLAPCSRSTSESTAALGCLVKDYFPEPVTVSWNSGALTSGVHTFPAVLQSSGLYSLSSVVTVPSSSLGTKTYTCNVDHKPSNTKVDKRVESKYGPPCPSCPAPESTRGPSVFLFPPKPKDTLMISRTPEVTCVVVDVSQEDPEVQFNWYVDGVEVHNAKTKPREEQFNSTYRVVSVLTVLHQDWLNGKEYKCKVSNKGLPSSIEKTISKAKGQPREPQVYTLPPSQEEMTKNQVSLSCAVKGFYPSDIAVEWESNGQPENNYKTTPPVLDSDGSFFLVSRLTVDKSRWQEGNVFSCSVLHEALHSHYTQKSLSLSLGK

SEQ ID NO: 336 - protein, 326 aa, synthetic construct
ASTKGPSVFPLAPCSRSTSESTAALGCLVKDYFPEPVTVSWNSGALTSGVHTFPAVLQSSGLYSLSSVVTVPSSSLGTKTYTCNVDHKPSNTKVDKRVESKYGPPCPSCPAPESTRGPSVFLFPPKPKDTLMISRTPEVTCVVVDVSQEDPEVQFNWYVDGVEVHNAKTKPREEQFNSTYRVVSVLTVLHQDWLNGKEYKCKVSNKGLPSSIEKTISKAKGQPREPQVYTLPPSQEEMTKNQVSLSCAVKGFYPSDIAVEWESNGQPENNYKTTPPVLDSDGSFFLVSRLTVDKSRWQEGNVFSCSVLHEALHSHYTQKSLSLSLG

SEQ ID NO: 337 - protein, 327 aa, synthetic construct
ASTKGPSVFPLAPCSRSTSESTAALGCLVKDYFPEPVTVSWNSGALTSGVHTFPAVLQSSGLYSLSSVVTVPSSSLGTKTYTCNVDHKPSNTKVDKRVESKYGPPCPSCPAPEAAGGPSVFLFPPKPKDTLMISRTPEVTCVVVDVSQEDPEVQFNWYVDGVEVHNAKTKPREEQFNSTYRVVSVLTVLHQDWLNGKEYKCKVSNKGLPSSIEKTISKAKGQPREPQVYTLPPSQEEMTKNQVSLSCAVKGFYPSDIAVEWESNGQPENNYKTTPPVLDSDGSFFLVSRLTVDKSRWQEGNVFSCSVLHEALHSHYTQKSLSLSLGK

SEQ ID NO: 338 - protein, 326 aa, synthetic construct
ASTKGPSVFPLAPCSRSTSESTAALGCLVKDYFPEPVTVSWNSGALTSGVHTFPAVLQSSGLYSLSSVVTVPSSSLGTKTYTCNVDHKPSNTKVDKRVESKYGPPCPSCPAPEAAGGPSVFLFPPKPKDTLMISRTPEVTCVVVDVSQEDPEVQFNWYVDGVEVHNAKTKPREEQFNSTYRVVSVLTVLHQDWLNGKEYKCKVSNKGLPSSIEKTISKAKGQPREPQVYTLPPSQEEMTKNQVSLSCAVKGFYPSDIAVEWESNGQPENNYKTTPPVLDSDGSFFLVSRLTVDKSRWQEGNVFSCSVLHEALHSHYTQKSLSLSLG

SEQ ID NO: 339 - protein, 327 aa, synthetic construct
ASTKGPSVFPLAPCSRSTSESTAALGCLVKDYFPEPVTVSWNSGALTSGVHTFPAVLQSSGLYSLSSVVTVPSSSLGTKTYTCNVDHKPSNTKVDKRVESKYGPPCPSCPAPEFLGGPSVFLFPPKPKDQLMISRTPEVTCVVVDVSQEDPEVQFNWYVDGVEVHNAKTKPREEQFNSTYRVVSVLTVLHQDWLNGKEYKCKVSNKGLPSSIEKTISKAKGQPREPQVYTLPPSQEEMTKNQVSLSCAVKGFYPSDIAVEWESNGQPENNYKTTPPVLDSDGSFFLVSRLTVDKSRWQEGNVFSCSVLHEALHNHYTQKSLSLSLGK

SEQ ID NO: 340 - protein, 326 aa, synthetic construct
ASTKGPSVFPLAPCSRSTSESTAALGCLVKDYFPEPVTVSWNSGALTSGVHTFPAVLQSSGLYSLSSVVTVPSSSLGTKTYTCNVDHKPSNTKVDKRVESKYGPPCPSCPAPEFLGGPSVFLFPPKPKDQLMISRTPEVTCVVVDVSQEDPEVQFNWYVDGVEVHNAKTKPREEQFNSTYRVVSVLTVLHQDWLNGKEYKCKVSNKGLPSSIEKTISKAKGQPREPQVYTLPPSQEEMTKNQVSLSCAVKGFYPSDIAVEWESNGQPENNYKTTPPVLDSDGSFFLVSRLTVDKSRWQEGNVFSCSVLHEALHNHYTQKSLSLSLG

SEQ ID NO: 341 - protein, 327 aa, synthetic construct
ASTKGPSVFPLAPCSRSTSESTAALGCLVKDYFPEPVTVSWNSGALTSGVHTFPAVLQSSGLYSLSSVVTVPSSSLGTKTYTCNVDHKPSNTKVDKRVESKYGPPCPSCPAPESTRGPSVFLFPPKPKDQLMISRTPEVTCVVVDVSQEDPEVQFNWYVDGVEVHNAKTKPREEQFNSTYRVVSVLTVLHQDWLNGKEYKCKVSNKGLPSSIEKTISKAKGQPREPQVYTLPPSQEEMTKNQVSLSCAVKGFYPSDIAVEWESNGQPENNYKTTPPVLDSDGSFFLVSRLTVDKSRWQEGNVFSCSVLHEALHNHYTQKSLSLSLGK

SEQ ID NO: 342 - protein, 326 aa, synthetic construct
ASTKGPSVFPLAPCSRSTSESTAALGCLVKDYFPEPVTVSWNSGALTSGVHTFPAVLQSSGLYSLSSVVTVPSSSLGTKTYTCNVDHKPSNTKVDKRVESKYGPPCPSCPAPESTRGPSVFLFPPKPKDQLMISRTPEVTCVVVDVSQEDPEVQFNWYVDGVEVHNAKTKPREEQFNSTYRVVSVLTVLHQDWLNGKEYKCKVSNKGLPSSIEKTISKAKGQPREPQVYTLPPSQEEMTKNQVSLSCAVKGFYPSDIAVEWESNGQPENNYKTTPPVLDSDGSFFLVSRLTVDKSRWQEGNVFSCSVLHEALHNHYTQKSLSLSLG

SEQ ID NO: 343 - protein, 327 aa, synthetic construct
ASTKGPSVFPLAPCSRSTSESTAALGCLVKDYFPEPVTVSWNSGALTSGVHTFPAVLQSSGLYSLSSVVTVPSSSLGTKTYTCNVDHKPSNTKVDKRVESKYGPPCPSCPAPEAAGGPSVFLFPPKPKDQLMISRTPEVTCVVVDVSQEDPEVQFNWYVDGVEVHNAKTKPREEQFNSTYRVVSVLTVLHQDWLNGKEYKCKVSNKGLPSSIEKTISKAKGQPREPQVYTLPPSQEEMTKNQVSLSCAVKGFYPSDIAVEWESNGQPENNYKTTPPVLDSDGSFFLVSRLTVDKSRWQEGNVFSCSVLHEALHNHYTQKSLSLSLGK

SEQ ID NO: 344 - protein, 326 aa, synthetic construct
ASTKGPSVFPLAPCSRSTSESTAALGCLVKDYFPEPVTVSWNSGALTSGVHTFPAVLQSSGLYSLSSVVTVPSSSLGTKTYTCNVDHKPSNTKVDKRVESKYGPPCPSCPAPEAAGGPSVFLFPPKPKDQLMISRTPEVTCVVVDVSQEDPEVQFNWYVDGVEVHNAKTKPREEQFNSTYRVVSVLTVLHQDWLNGKEYKCKVSNKGLPSSIEKTISKAKGQPREPQVYTLPPSQEEMTKNQVSLSCAVKGFYPSDIAVEWESNGQPENNYKTTPPVLDSDGSFFLVSRLTVDKSRWQEGNVFSCSVLHEALHNHYTQKSLSLSLG

SEQ ID NO: 345 - protein, 327 aa, synthetic construct
ASTKGPSVFPLAPCSRSTSESTAALGCLVKDYFPEPVTVSWNSGALTSGVHTFPAVLQSSGLYSLSSVVTVPSSSLGTKTYTCNVDHKPSNTKVDKRVESKYGPPCPSCPAPEFLGGPSVFLFPPKPKDTLMISRTPEVTCVVVDVSQEDPEVQFNWYVDGVEVHNAKTKPREEQFNSTYRVVSVLTVDHHDWLNGKEYKCKVSNKGLPSSIEKTISKAKGQPREPQVYTLPPSQEEMTKNQVSLSCAVKGFYPSDIAVEWESNGQPENNYKTTPPVLDSDGSFFLVSRLTVDKSRWQEGNVFSCSVMHEALHSHYTQKSLSLSLGK

SEQ ID NO: 346 - protein, 326 aa, synthetic construct
ASTKGPSVFPLAPCSRSTSESTAALGCLVKDYFPEPVTVSWNSGALTSGVHTFPAVLQSSGLYSLSSVVTVPSSSLGTKTYTCNVDHKPSNTKVDKRVESKYGPPCPSCPAPEFLGGPSVFLFPPKPKDTLMISRTPEVTCVVVDVSQEDPEVQFNWYVDGVEVHNAKTKPREEQFNSTYRVVSVLTVDHHDWLNGKEYKCKVSNKGLPSSIEKTISKAKGQPREPQVYTLPPSQEEMTKNQVSLSCAVKGFYPSDIAVEWESNGQPENNYKTTPPVLDSDGSFFLVSRLTVDKSRWQEGNVFSCSVMHEALHSHYTQKSLSLSLG

SEQ ID NO: 347 - protein, 327 aa, synthetic construct
ASTKGPSVFPLAPCSRSTSESTAALGCLVKDYFPEPVTVSWNSGALTSGVHTFPAVLQSSGLYSLSSVVTVPSSSLGTKTYTCNVDHKPSNTKVDKRVESKYGPPCPSCPAPESTRGPSVFLFPPKPKDTLMISRTPEVTCVVVDVSQEDPEVQFNWYVDGVEVHNAKTKPREEQFNSTYRVVSVLTVDHHDWLNGKEYKCKVSNKGLPSSIEKTISKAKGQPREPQVYTLPPSQEEMTKNQVSLSCAVKGFYPSDIAVEWESNGQPENNYKTTPPVLDSDGSFFLVSRLTVDKSRWQEGNVFSCSVMHEALHSHYTQKSLSLSLGK

SEQ ID NO: 348 - protein, 326 aa, synthetic construct
ASTKGPSVFPLAPCSRSTSESTAALGCLVKDYFPEPVTVSWNSGALTSGVHTFPAVLQSSGLYSLSSVVTVPSSSLGTKTYTCNVDHKPSNTKVDKRVESKYGPPCPSCPAPESTRGPSVFLFPPKPKDTLMISRTPEVTCVVVDVSQEDPEVQFNWYVDGVEVHNAKTKPREEQFNSTYRVVSVLTVDHHDWLNGKEYKCKVSNKGLPSSIEKTISKAKGQPREPQVYTLPPSQEEMTKNQVSLSCAVKGFYPSDIAVEWESNGQPENNYKTTPPVLDSDGSFFLVSRLTVDKSRWQEGNVFSCSVMHEALHSHYTQKSLSLSLG

SEQ ID NO: 349 - protein, 327 aa, synthetic construct
ASTKGPSVFPLAPCSRSTSESTAALGCLVKDYFPEPVTVSWNSGALTSGVHTFPAVLQSSGLYSLSSVVTVPSSSLGTKTYTCNVDHKPSNTKVDKRVESKYGPPCPSCPAPEAAGGPSVFLFPPKPKDTLMISRTPEVTCVVVDVSQEDPEVQFNWYVDGVEVHNAKTKPREEQFNSTYRVVSVLTVDHHDWLNGKEYKCKVSNKGLPSSIEKTISKAKGQPREPQVYTLPPSQEEMTKNQVSLSCAVKGFYPSDIAVEWESNGQPENNYKTTPPVLDSDGSFFLVSRLTVDKSRWQEGNVFSCSVMHEALHSHYTQKSLSLSLGK

SEQ ID NO: 350 - protein, 326 aa, synthetic construct
ASTKGPSVFPLAPCSRSTSESTAALGCLVKDYFPEPVTVSWNSGALTSGVHTFPAVLQSSGLYSLSSVVTVPSSSLGTKTYTCNVDHKPSNTKVDKRVESKYGPPCPSCPAPEAAGGPSVFLFPPKPKDTLMISRTPEVTCVVVDVSQEDPEVQFNWYVDGVEVHNAKTKPREEQFNSTYRVVSVLTVDHHDWLNGKEYKCKVSNKGLPSSIEKTISKAKGQPREPQVYTLPPSQEEMTKNQVSLSCAVKGFYPSDIAVEWESNGQPENNYKTTPPVLDSDGSFFLVSRLTVDKSRWQEGNVFSCSVMHEALHSHYTQKSLSLSLG

SEQ ID NO: 351 - protein, 253 aa, synthetic construct
EIVLTQSPATLSVTPGDRVSLSCRASQNINNNLHWYQQKPGQSPRLLIKYVSQSVSGIPDRFSGSGSGTDFTLSISSVEPEDEGMYFCQQSNSWPHYTFGCGTKLEIKGGGGSGGGGSGGGGSGGGGSEVQLVQSGGGLVQPGGSRRLSCAASGFTFSSFGMHWVRQAPGKCLEWVAYISSGSSTISYADSVKGRFTISRDNSKKTLLLQMTSLRAEDTAMYYCAREAYGSSMEYWGQGTLVTVSSGSEPKSS

SEQ ID NO: 352 - protein, 20 aa, synthetic construct
GGGGSGGGGSGGGGSGGGGS